European Patent Application EP 4 389 893 A1, published June 26, 2024. Title: ヒトトランスフェリンレセプター結合ペプチド－薬物コンジュゲート. Applicant: 武田薬品工業株式会社. Application JP. The sequence listing filed with the application follows.

SEQUENCE LISTING (883 sequences)

SEQ ID NO: 1 - protein, 12 aa, synthetic construct
  REGION 1..12: note = Synthesized polypeptide
AVFVWNYYIISC

SEQ ID NO: 2 - protein, 15 aa, synthetic construct
  REGION 1..15: note = Synthesized polypeptide
  MOD_RES 14: note = METHYLATION
AVFVWNYYIIRRYYC

SEQ ID NO: 3 - protein, 17 aa, synthetic construct
  REGION 1..17: note = Synthesized polypeptide
AVFVWNYYIVDRFGTGC

SEQ ID NO: 4 - protein, 17 aa, synthetic construct
  REGION 1..17: note = Synthesized polypeptide
AVFVWNYYIVGRNVPNC

SEQ ID NO: 5 - protein, 17 aa, synthetic construct
  REGION 1..17: note = Synthesized polypeptide
  MOD_RES 16: note = METHYLATION
ANRIVFVWNYYIIPRHC

SEQ ID NO: 6 - protein, 14 aa, synthetic construct
  REGION 1..14: note = Synthesized polypeptide
AVWVWNYFIIPRHC

SEQ ID NO: 7 - protein, 17 aa, synthetic construct
  REGION 1..17: note = Synthesized polypeptide
  MOD_RES 16: note = METHYLATION
AVFVWNYYIIDRFRSYC

SEQ ID NO: 8 - protein, 17 aa, synthetic construct
  REGION 1..17: note = Synthesized polypeptide
  MOD_RES 16: note = METHYLATION
AVFVWNYYIIDRFRSHC

SEQ ID NO: 9 - protein, 15 aa, synthetic construct
  REGION 1..15: note = Synthesized polypeptide
AVFVWNYYIIDRFRC

SEQ ID NO: 10 - protein, 17 aa, synthetic construct
  REGION 1..17: note = Synthesized polypeptide
ASAVFVWNYYIINRWAC

SEQ ID NO: 11 - protein, 14 aa, synthetic construct
  REGION 1..14: note = Synthesized polypeptide
AVFVWNYYIVPREC

SEQ ID NO: 12 - protein, 14 aa, synthetic construct
  REGION 1..14: note = Synthesized polypeptide
AVFVWNYYIVPRNC

SEQ ID NO: 13 - protein, 17 aa, synthetic construct
  REGION 1..17: note = Synthesized polypeptide
ANSRTVWVWNYYIVTRC

SEQ ID NO: 14 - protein, 17 aa, synthetic construct
  REGION 1..17: note = Synthesized polypeptide
  MOD_RES 16: note = METHYLATION
ANRIVFVWNYYIIPRYC

SEQ ID NO: 15 - protein, 14 aa, synthetic construct
  REGION 1..14: note = Synthesized polypeptide
AVFVWNYYIVPRDC

SEQ ID NO: 16 - protein, 12 aa, synthetic construct
  REGION 1..12: note = Synthesized polypeptide
AVFVWNYYIVHC

SEQ ID NO: 17 - protein, 14 aa, synthetic construct
  REGION 1..14: note = Synthesized polypeptide
  MOD_RES 13: note = METHYLATION
AVFVWNYYIVPRWC

SEQ ID NO: 18 - protein, 12 aa, synthetic construct
  REGION 1..12: note = Synthesized polypeptide
AVFVWNYYIVSC

SEQ ID NO: 19 - protein, 12 aa, synthetic construct
  REGION 1..12: note = Synthesized polypeptide
AVFVWNYYIISC

SEQ ID NO: 20 - protein, 12 aa, synthetic construct
  REGION 1..12: note = Synthesized polypeptide
AVWVWNYYIINC

SEQ ID NO: 21 - protein, 15 aa, synthetic construct
  REGION 1..15: note = Synthesized polypeptide
  MOD_RES 14: note = METHYLATION
AVFVWNYYIIRRYYC

SEQ ID NO: 22 - protein, 15 aa, synthetic construct
  REGION 1..15: note = Synthesized polypeptide
  MOD_RES 3: note = METHYLATION
  MOD_RES 14: note = METHYLATION
AVFVWNYYIIRRYYC

SEQ ID NO: 23 - protein, 15 aa, synthetic construct
  REGION 1..15: note = Synthesized polypeptide
  MOD_RES 3: note = METHYLATION
  MOD_RES 14: note = METHYLATION
AVFVWNYYIIKRYYC

SEQ ID NO: 24 - protein, 15 aa, synthetic construct
  REGION 1..15: note = Synthesized polypeptide
  MOD_RES 3: note = METHYLATION
  MOD_RES 5: note = METHYLATION
  MOD_RES 14: note = METHYLATION
AVFVWNYYIIRRYYC

SEQ ID NO: 25 - protein, 15 aa, synthetic construct
  REGION 1..15: note = Synthesized polypeptide
  MOD_RES 3: note = METHYLATION
  MOD_RES 5: note = METHYLATION
  MOD_RES 14: note = METHYLATION
AVFVWNYYIIKRYYC

SEQ ID NO: 26 - protein, 15 aa, synthetic construct
  REGION 1..15: note = Synthesized polypeptide
  MOD_RES 3: note = METHYLATION
  MOD_RES 5: note = METHYLATION
  MOD_RES 14: note = METHYLATION
AVFVWNYYIIKKYYC

SEQ ID NO: 27 - protein, 15 aa, synthetic construct
  REGION 1..15: note = Synthesized polypeptide
  MOD_RES 14: note = METHYLATION
AVFVWNYYIIRRYYC

SEQ ID NO: 28 - protein, 15 aa, synthetic construct
  REGION 1..15: note = Synthesized polypeptide
  MOD_RES 3: note = METHYLATION
  MOD_RES 14: note = METHYLATION
AVFVWNYYIIRRYYC

SEQ ID NO: 29 - protein, 15 aa, synthetic construct
  REGION 1..15: note = Synthesized polypeptide
  MOD_RES 3: note = METHYLATION
  MOD_RES 14: note = METHYLATION
AVFVWNYYIIKRYYC

SEQ ID NO: 30 - protein, 15 aa, synthetic construct
  REGION 1..15: note = Synthesized polypeptide
  MOD_RES 3: note = METHYLATION
  MOD_RES 5: note = METHYLATION
  MOD_RES 14: note = METHYLATION
AVFVWNYYIIRRYYC

SEQ ID NO: 31 - protein, 15 aa, synthetic construct
  REGION 1..15: note = Synthesized polypeptide
  MOD_RES 3: note = METHYLATION
  MOD_RES 5: note = METHYLATION
  MOD_RES 14: note = METHYLATION
AVFVWNYYIIKRYYC

SEQ ID NO: 32 - protein, 15 aa, synthetic construct
  REGION 1..15: note = Synthesized polypeptide
  MOD_RES 3: note = METHYLATION
  MOD_RES 5: note = METHYLATION
  MOD_RES 14: note = METHYLATION
AVFVWNYYIIKKYYC

SEQ ID NO: 33 - protein, 15 aa, synthetic construct
  REGION 1..15: note = Synthesized polypeptide
  MOD_RES 3: note = METHYLATION
  MOD_RES 5: note = METHYLATION
  MOD_RES 14: note = METHYLATION
AVFVWNYYIIKRYYC

SEQ ID NO: 34 - protein, 15 aa, synthetic construct
  REGION 1..15: note = Synthesized polypeptide
  MOD_RES 14: note = METHYLATION
AVFVWNYYIIRRYYC

SEQ ID NO: 35 - protein, 15 aa, synthetic construct
  REGION 1..15: note = Synthesized polypeptide
  MOD_RES 3: note = METHYLATION
  MOD_RES 5: note = METHYLATION
  MOD_RES 14: note = METHYLATION
AVFVWNYYIVKRYYC

SEQ ID NO: 36 - protein, 15 aa, synthetic construct
  REGION 1..15: note = Synthesized polypeptide
  MOD_RES 3: note = METHYLATION
  MOD_RES 5: note = METHYLATION
  SITE 11: note = MISC_FEATURE - Xaa is aMeK
  MOD_RES 14: note = METHYLATION
AVFVWNYYIIXRYYC

SEQ ID NO: 37 - protein, 15 aa, synthetic construct
  REGION 1..15: note = Synthesized polypeptide
  MOD_RES 3: note = METHYLATION
  MOD_RES 5: note = METHYLATION
  SITE 14: note = MISC_FEATURE - Xaa is MeBph
AVFVWNYYIIKRYXC

SEQ ID NO: 38 - protein, 15 aa, synthetic construct
  REGION 1..15: note = Synthesized polypeptide
  MOD_RES 3: note = METHYLATION
  SITE 5: note = MISC_FEATURE - Xaa is W1Et
  MOD_RES 14: note = METHYLATION
AVFVXNYYIIKRYYC

SEQ ID NO: 39 - protein, 15 aa, synthetic construct
  REGION 1..15: note = Synthesized polypeptide
  MOD_RES 3: note = METHYLATION
  SITE 5: note = MISC_FEATURE - Xaa is W1iPr
  MOD_RES 14: note = METHYLATION
AVFVXNYYIIKRYYC

SEQ ID NO: 40 - protein, 15 aa, synthetic construct
  REGION 1..15: note = Synthesized polypeptide
  MOD_RES 3: note = METHYLATION
  MOD_RES 5: note = METHYLATION
  SITE 11: note = MISC_FEATURE - Xaa is Hly
  MOD_RES 14: note = METHYLATION
AVFVWNYYIIXRYYC

SEQ ID NO: 41 - protein, 15 aa, synthetic construct
  REGION 1..15: note = Synthesized polypeptide
  MOD_RES 3: note = METHYLATION
  MOD_RES 5: note = METHYLATION
  MOD_RES 14: note = METHYLATION
AVFVWNYYIIKRYYC

SEQ ID NO: 42 - protein, 15 aa, synthetic construct
  REGION 1..15: note = Synthesized polypeptide
  MOD_RES 3: note = METHYLATION
  MOD_RES 5: note = METHYLATION
  SITE 14: note = MISC_FEATURE - Xaa is MeNal2
AVFVWNYYIIKRYXC

SEQ ID NO: 43 - protein, 15 aa, synthetic construct
  REGION 1..15: note = Synthesized polypeptide
  MOD_RES 3: note = METHYLATION
  MOD_RES 5: note = METHYLATION
  MOD_RES 14: note = METHYLATION
AVFVWNYYIIKKYYC

SEQ ID NO: 44 - protein, 15 aa, synthetic construct
  REGION 1..15: note = Synthesized polypeptide
  MOD_RES 3: note = METHYLATION
  MOD_RES 5: note = METHYLATION
  SITE 12: note = MISC_FEATURE - Xaa is Orn
  MOD_RES 14: note = METHYLATION
AVFVWNYYIIKXYYC

SEQ ID NO: 45 - protein, 15 aa, synthetic construct
  REGION 1..15: note = Synthesized polypeptide
  MOD_RES 3: note = METHYLATION
  MOD_RES 5: note = METHYLATION
  MOD_RES 14: note = METHYLATION
AVFVWNYYILKRYYC

SEQ ID NO: 46 - protein, 15 aa, synthetic construct
  REGION 1..15: note = Synthesized polypeptide
  MOD_RES 3: note = METHYLATION
  MOD_RES 5: note = METHYLATION
  MOD_RES 14: note = METHYLATION
AVFVWNYYIIKRYFC

SEQ ID NO: 47 - protein, 15 aa, synthetic construct
  REGION 1..15: note = Synthesized polypeptide
  MOD_RES 3: note = METHYLATION
  MOD_RES 5: note = METHYLATION
  SITE 12: note = MISC_FEATURE - Xaa is Hly
  MOD_RES 14: note = METHYLATION
AVFVWNYYIIKXYYC

SEQ ID NO: 48 - protein, 15 aa, synthetic construct
  REGION 1..15: note = Synthesized polypeptide
  MOD_RES 3: note = METHYLATION
  MOD_RES 5: note = METHYLATION
  MOD_RES 14: note = METHYLATION
AVFVWNYYIIKRYWC

SEQ ID NO: 49 - protein, 15 aa, synthetic construct
  REGION 1..15: note = Synthesized polypeptide
  MOD_RES 3: note = METHYLATION
  MOD_RES 5: note = METHYLATION
  SITE 14: note = MISC_FEATURE - Xaa is MeoBph
AVFVWNYYIIKRYXC

SEQ ID NO: 50 - protein, 15 aa, synthetic construct
  REGION 1..15: note = Synthesized polypeptide
  SITE 3: note = MISC_FEATURE - Xaa is F2OMe
  MOD_RES 5: note = METHYLATION
  MOD_RES 14: note = METHYLATION
AVXVWNYYIIKRYYC

SEQ ID NO: 51 - protein, 15 aa, synthetic construct
  REGION 1..15: note = Synthesized polypeptide
  SITE 3: note = MISC_FEATURE - Xaa is Cha
  MOD_RES 5: note = METHYLATION
  MOD_RES 14: note = METHYLATION
AVXVWNYYIIKRYYC

SEQ ID NO: 52 - protein, 15 aa, synthetic construct
  REGION 1..15: note = Synthesized polypeptide
  MOD_RES 3: note = METHYLATION
  MOD_RES 5: note = METHYLATION
  SITE 14: note = MISC_FEATURE - Xaa is MeNal1
AVFVWNYYIIKRYXC

SEQ ID NO: 53 - protein, 15 aa, synthetic construct
  REGION 1..15: note = Synthesized polypeptide
  MOD_RES 3: note = METHYLATION
  MOD_RES 5: note = METHYLATION
  SITE 14: note = MISC_FEATURE - Xaa is MemBph
AVFVWNYYIIKRYXC

SEQ ID NO: 54 - protein, 15 aa, synthetic construct
  REGION 1..15: note = Synthesized polypeptide
  MOD_RES 3: note = METHYLATION
  SITE 5: note = MISC_FEATURE - Xaa is Nal2
  MOD_RES 14: note = METHYLATION
AVFVXNYYIIKKYYC

SEQ ID NO: 55 - protein, 15 aa, synthetic construct
  REGION 1..15: note = Synthesized polypeptide
  MOD_RES 3: note = METHYLATION
  MOD_RES 5: note = METHYLATION
  SITE 14: note = MISC_FEATURE - Xaa is pHPeG
AVFVWNYYIIKRYXC

SEQ ID NO: 56 - protein, 15 aa, synthetic construct
  REGION 1..15: note = Synthesized polypeptide
  MOD_RES 3: note = METHYLATION
  SITE 5: note = MISC_FEATURE - Xaa is W1Et7Cl
  MOD_RES 14: note = METHYLATION
AVFVXNYYIIKRYYC

SEQ ID NO: 57 - protein, 15 aa, synthetic construct
  REGION 1..15: note = Synthesized polypeptide
  SITE 3: note = MISC_FEATURE - Xaa is MeNal1
  MOD_RES 5: note = METHYLATION
  MOD_RES 14: note = METHYLATION
AVXVWNYYIIKKYYC

SEQ ID NO: 58 - protein, 15 aa, synthetic construct
  REGION 1..15: note = Synthesized polypeptide
  MOD_RES 3: note = METHYLATION
  MOD_RES 5: note = METHYLATION
  SITE 12: note = MISC_FEATURE - Xaa is Cit
  MOD_RES 14: note = METHYLATION
AVFVWNYYIIKXYYC

SEQ ID NO: 59 - protein, 15 aa, synthetic construct
  REGION 1..15: note = Synthesized polypeptide
  MOD_RES 3: note = METHYLATION
  MOD_RES 5: note = METHYLATION
  SITE 11: note = MISC_FEATURE - Xaa is Dap
  MOD_RES 14: note = METHYLATION
AVFVWNYYIIXRYYC

SEQ ID NO: 60 - protein, 15 aa, synthetic construct
  REGION 1..15: note = Synthesized polypeptide
  MOD_RES 3: note = METHYLATION
  SITE 5: note = MISC_FEATURE - Xaa is Nal2
  SITE 12: note = MISC_FEATURE - Xaa is F4G
  MOD_RES 14: note = METHYLATION
AVFVXNYYIIKXYYC

SEQ ID NO: 61 - protein, 15 aa, synthetic construct
  REGION 1..15: note = Synthesized polypeptide
  MOD_RES 3: note = METHYLATION
  SITE 5: note = MISC_FEATURE - Xaa is Yph
  MOD_RES 14: note = METHYLATION
AVFVXNYYIIKRYYC

SEQ ID NO: 62 - protein, 15 aa, synthetic construct
  REGION 1..15: note = Synthesized polypeptide
  MOD_RES 3: note = METHYLATION
  MOD_RES 5: note = METHYLATION
  SITE 12: note = MISC_FEATURE - Xaa is Dab
  MOD_RES 14: note = METHYLATION
AVFVWNYYIIKXYYC

SEQ ID NO: 63 - protein, 15 aa, synthetic construct
  REGION 1..15: note = Synthesized polypeptide
  MOD_RES 3: note = METHYLATION
  SITE 5: note = MISC_FEATURE - Xaa is MeNal2
  MOD_RES 14: note = METHYLATION
AVFVXNYYIIKRYYC

SEQ ID NO: 64 - protein, 15 aa, synthetic construct
  REGION 1..15: note = Synthesized polypeptide
  MOD_RES 3: note = METHYLATION
  SITE 5: note = MISC_FEATURE - Xaa is MemBph
  MOD_RES 14: note = METHYLATION
AVFVXNYYIIKRYYC

SEQ ID NO: 65 - protein, 15 aa, synthetic construct
  REGION 1..15: note = Synthesized polypeptide
  MOD_RES 3: note = METHYLATION
  MOD_RES 5: note = METHYLATION
  SITE 11: note = MISC_FEATURE - Xaa is F4G
  MOD_RES 14: note = METHYLATION
AVFVWNYYIIXRYYC

SEQ ID NO: 66 - protein, 15 aa, synthetic construct
  REGION 1..15: note = Synthesized polypeptide
  MOD_RES 3: note = METHYLATION
  MOD_RES 5: note = METHYLATION
  SITE 12: note = MISC_FEATURE - Xaa is F4G
  MOD_RES 14: note = METHYLATION
AVFVWNYYIIKXYYC

SEQ ID NO: 67 - protein, 15 aa, synthetic construct
  REGION 1..15: note = Synthesized polypeptide
  MOD_RES 3: note = METHYLATION
  SITE 5: note = MISC_FEATURE - Xaa is MeNal1
  MOD_RES 14: note = METHYLATION
AVFVXNYYIIKRYYC

SEQ ID NO: 68 - protein, 15 aa, synthetic construct
  REGION 1..15: note = Synthesized polypeptide
  SITE 3: note = MISC_FEATURE - Xaa is MeNal1
  MOD_RES 5: note = METHYLATION
  SITE 12: note = MISC_FEATURE - Xaa is F4G
  MOD_RES 14: note = METHYLATION
AVXVWNYYIIKXYYC

SEQ ID NO: 69 - protein, 15 aa, synthetic construct
  REGION 1..15: note = Synthesized polypeptide
  MOD_RES 3: note = METHYLATION
  MOD_RES 5: note = METHYLATION
  MOD_RES 14: note = METHYLATION
AVFVWNYYISKRYYC

SEQ ID NO: 70 - protein, 15 aa, synthetic construct
  REGION 1..15: note = Synthesized polypeptide
  MOD_RES 3: note = METHYLATION
  MOD_RES 5: note = METHYLATION
  MOD_RES 14: note = METHYLATION
  SITE 15: note = MISC_FEATURE - Xaa is aMeC
AVFVWNYYIIKRYYX

SEQ ID NO: 71 - protein, 15 aa, synthetic construct
  REGION 1..15: note = Synthesized polypeptide
  SITE 3: note = MISC_FEATURE - Xaa is F2C
  MOD_RES 5: note = METHYLATION
  MOD_RES 14: note = METHYLATION
AVXVWNYYIIKRYYC

SEQ ID NO: 72 - protein, 15 aa, synthetic construct
  REGION 1..15: note = Synthesized polypeptide
  MOD_RES 3: note = METHYLATION
  MOD_RES 5: note = METHYLATION
  SITE 11: note = MISC_FEATURE - Xaa is Orn
  MOD_RES 14: note = METHYLATION
AVFVWNYYIIXRYYC

SEQ ID NO: 73 - protein, 15 aa, synthetic construct
  REGION 1..15: note = Synthesized polypeptide
  MOD_RES 3: note = METHYLATION
  MOD_RES 5: note = METHYLATION
  SITE 14: note = MISC_FEATURE - Xaa is aMeTyr
AVFVWNYYIIKRYXC

SEQ ID NO: 74 - protein, 15 aa, synthetic construct
  REGION 1..15: note = Synthesized polypeptide
  MOD_RES 3: note = METHYLATION
  MOD_RES 5: note = METHYLATION
  SITE 12: note = MISC_FEATURE - Xaa is Dap
  MOD_RES 14: note = METHYLATION
AVFVWNYYIIKXYYC

SEQ ID NO: 75 - protein, 15 aa, synthetic construct
  REGION 1..15: note = Synthesized polypeptide
  MOD_RES 3: note = METHYLATION
  MOD_RES 5: note = METHYLATION
  SITE 13: note = MISC_FEATURE - Xaa is pHPeG
  MOD_RES 14: note = METHYLATION
AVFVWNYYIIKRXYC

SEQ ID NO: 76 - protein, 15 aa, synthetic construct
  REGION 1..15: note = Synthesized polypeptide
  MOD_RES 3: note = METHYLATION
  MOD_RES 5: note = METHYLATION
  SITE 11: note = MISC_FEATURE - Xaa is Dab
  MOD_RES 14: note = METHYLATION
AVFVWNYYIIXRYYC

SEQ ID NO: 77 - protein, 15 aa, synthetic construct
  REGION 1..15: note = Synthesized polypeptide
  SITE 1: note = MISC_FEATURE - Xaa is Alaib
  MOD_RES 3: note = METHYLATION
  MOD_RES 5: note = METHYLATION
  MOD_RES 14: note = METHYLATION
XVFVWNYYIIKRYYC

SEQ ID NO: 78 - protein, 15 aa, synthetic construct
  REGION 1..15: note = Synthesized polypeptide
  MOD_RES 3: note = METHYLATION
  MOD_RES 5: note = METHYLATION
  MOD_RES 14: note = METHYLATION
AVFVWNYYLIKRYYC

SEQ ID NO: 79 - protein, 15 aa, synthetic construct
  REGION 1..15: note = Synthesized polypeptide
  SITE 3: note = MISC_FEATURE - Xaa is MeNal1
  MOD_RES 5: note = METHYLATION
  SITE 11: note = MISC_FEATURE - Xaa is F4G
  MOD_RES 14: note = METHYLATION
AVXVWNYYIIXKYYC

SEQ ID NO: 80 - protein, 15 aa, synthetic construct
  REGION 1..15: note = Synthesized polypeptide
  MOD_RES 3: note = METHYLATION
  MOD_RES 5: note = METHYLATION
  MOD_RES 14: note = METHYLATION
AVFVWQYYIIKRYYC

SEQ ID NO: 81 - protein, 15 aa, synthetic construct
  REGION 1..15: note = Synthesized polypeptide
  MOD_RES 3: note = METHYLATION
  MOD_RES 5: note = METHYLATION
  SITE 7: note = MISC_FEATURE - Xaa is Nal1
  MOD_RES 14: note = METHYLATION
AVFVWNXYIIKRYYC

SEQ ID NO: 82 - protein, 15 aa, synthetic construct
  REGION 1..15: note = Synthesized polypeptide
  SITE 3: note = MISC_FEATURE - Xaa is MeNal1
  SITE 5: note = MISC_FEATURE - Xaa is MeNal2
  SITE 7: note = MISC_FEATURE - Xaa is Nal1
  SITE 8: note = MISC_FEATURE - Xaa is Nal1
  MOD_RES 14: note = METHYLATION
AVXVXNXXIIKKYYC

SEQ ID NO: 83 - protein, 15 aa, synthetic construct
  REGION 1..15: note = Synthesized polypeptide
  MOD_RES 3: note = METHYLATION
  MOD_RES 5: note = METHYLATION
  MOD_RES 14: note = METHYLATION
PVFVWNYYIIKRYYC

SEQ ID NO: 84 - protein, 15 aa, synthetic construct
  REGION 1..15: note = Synthesized polypeptide
  SITE 3: note = MISC_FEATURE - Xaa is F4C
  MOD_RES 5: note = METHYLATION
  MOD_RES 14: note = METHYLATION
AVXVWNYYIIKRYYC

SEQ ID NO: 85 - protein, 15 aa, synthetic construct
  REGION 1..15: note = Synthesized polypeptide
  MOD_RES 3: note = METHYLATION
  MOD_RES 5: note = METHYLATION
  MOD_RES 14: note = METHYLATION
AVFVWNYYIPKRYYC

SEQ ID NO: 86 - protein, 15 aa, synthetic construct
  REGION 1..15: note = Synthesized polypeptide
  MOD_RES 3: note = METHYLATION
  SITE 5: note = MISC_FEATURE - Xaa is aMeTrp
  MOD_RES 14: note = METHYLATION
AVFVXNYYIIKRYYC

SEQ ID NO: 87 - protein, 15 aa, synthetic construct
  REGION 1..15: note = Synthesized polypeptide
  MOD_RES 3: note = METHYLATION
  SITE 5: note = MISC_FEATURE - Xaa is MeoBph
  MOD_RES 14: note = METHYLATION
AVFVXNYYIIKRYYC

SEQ ID NO: 88 - protein, 15 aa, synthetic construct
  REGION 1..15: note = Synthesized polypeptide
  MOD_RES 3: note = METHYLATION
  MOD_RES 5: note = METHYLATION
  SITE 12: note = MISC_FEATURE - Xaa is Orn
  MOD_RES 14: note = METHYLATION
AVFVWNYYIIKXYYC

SEQ ID NO: 89 - protein, 15 aa, synthetic construct
  REGION 1..15: note = Synthesized polypeptide
  MOD_RES 3: note = METHYLATION
  MOD_RES 5: note = METHYLATION
  SITE 11: note = MISC_FEATURE - Xaa is Hly
  MOD_RES 14: note = METHYLATION
AVFVWNYYIIXRYYC

SEQ ID NO: 90 - protein, 15 aa, synthetic construct
  REGION 1..15: note = Synthesized polypeptide
  MOD_RES 3: note = METHYLATION
  MOD_RES 5: note = METHYLATION
  SITE 11: note = MISC_FEATURE - Xaa is Orn
  MOD_RES 14: note = METHYLATION
AVFVWNYYIIXRYYC

SEQ ID NO: 91 - protein, 15 aa, synthetic construct
  REGION 1..15: note = Synthesized polypeptide
  MOD_RES 3: note = METHYLATION
  MOD_RES 5: note = METHYLATION
  SITE 11: note = MISC_FEATURE - Xaa is Dap
  MOD_RES 14: note = METHYLATION
AVFVWNYYIIXRYYC

SEQ ID NO: 92 - protein, 15 aa, synthetic construct
  REGION 1..15: note = Synthesized polypeptide
  MOD_RES 3: note = METHYLATION
  MOD_RES 5: note = METHYLATION
  SITE 14: note = MISC_FEATURE - Xaa is MemBph
AVFVWNYYIIKRYXC

SEQ ID NO: 93 - protein, 15 aa, synthetic construct
  REGION 1..15: note = Synthetic Peptide
  MOD_RES 3: note = METHYLATION
  MOD_RES 5: note = METHYLATION
  SITE 7: note = MISC_FEATURE - Xaa is Nal1
  MOD_RES 14: note = METHYLATION
AVFVWNXYIIKRYYC

SEQ ID NO: 94 - protein, 15 aa, synthetic construct
  REGION 1..15: note = Synthesized polypeptide
  MOD_RES 3: note = METHYLATION
  MOD_RES 5: note = METHYLATION
  MOD_RES 14: note = METHYLATION
AVFVWNYYIPKRYYC

SEQ ID NO: 95 - protein, 15 aa, synthetic construct
  REGION 1..15: note = Synthesized polypeptide
  MOD_RES 3: note = METHYLATION
  SITE 5: note = MISC_FEATURE - Xaa is dp
  MOD_RES 14: note = METHYLATION
AVFVXNYYIIKRYYC

SEQ ID NO: 96 - protein, 15 aa, synthetic construct
  REGION 1..15: note = Synthesized polypeptide
  MOD_RES 3: note = METHYLATION
  MOD_RES 5: note = METHYLATION
  SITE 9: note = MISC_FEATURE - Xaa is Tbg
  MOD_RES 14: note = METHYLATION
AVFVWNYYXIKRYYC

SEQ ID NO: 97 - protein, 15 aa, synthetic construct
  REGION 1..15: note = Synthesized polypeptide
  MOD_RES 3: note = METHYLATION
  MOD_RES 5: note = METHYLATION
  SITE 10: note = MISC_FEATURE - Xaa is Tbg
  MOD_RES 14: note = METHYLATION
AVFVWNYYIXKRYYC

SEQ ID NO: 98 - protein, 15 aa, synthetic construct
  REGION 1..15: note = Synthesized polypeptide
  SITE 3: note = MISC_FEATURE - Xaa is MePhe4F
  MOD_RES 14: note = METHYLATION
AVXVWNYYIIRRYYC

SEQ ID NO: 99 - protein, 15 aa, synthetic construct
  REGION 1..15: note = Synthesized polypeptide
  SITE 3: note = MISC_FEATURE - Xaa is MePhe3C
  MOD_RES 14: note = METHYLATION
AVXVWNYYIIRRYYC

SEQ ID NO: 100 - protein, 15 aa, synthetic construct
  REGION 1..15: note = Synthesized polypeptide
  MOD_RES 3: note = METHYLATION
  SITE 8: note = MISC_FEATURE - Xaa is F4OMe
  MOD_RES 14: note = METHYLATION
AVFVWNYXIIRRYYC

SEQ ID NO: 101 - protein, 15 aa, synthetic construct
  REGION 1..15: note = Synthesized polypeptide
  SITE 3: note = MISC_FEATURE - Xaa is MePhe3F
  MOD_RES 14: note = METHYLATION
AVXVWNYYIIRRYYC

SEQ ID NO: 102 - protein, 15 aa, synthetic construct
  REGION 1..15: note = Synthesized polypeptide
  MOD_RES 3: note = METHYLATION
  MOD_RES 14: note = METHYLATION
AVFVWNYYIIRRFYC

SEQ ID NO: 103 - protein, 15 aa, synthetic construct
  REGION 1..15: note = Synthesized polypeptide
  MOD_RES 3: note = METHYLATION
  MOD_RES 14: note = METHYLATION
AVFVWNYYIIRRYYC

SEQ ID NO: 104 - protein, 15 aa, synthetic construct
  REGION 1..15: note = Synthesized polypeptide
  MOD_RES 3: note = METHYLATION
  MOD_RES 14: note = METHYLATION
AVFVWNYWIIRRYYC

SEQ ID NO: 105 - protein, 15 aa, synthetic construct
  REGION 1..15: note = Synthesized polypeptide
  SITE 3: note = MISC_FEATURE - Xaa is MePhe3OMe
  MOD_RES 14: note = METHYLATION
AVXVWNYYIIRRYYC

SEQ ID NO: 106 - protein, 15 aa, synthetic construct
  REGION 1..15: note = Synthesized polypeptide
  MOD_RES 3: note = METHYLATION
  MOD_RES 14: note = METHYLATION
AVFVWNYYIIRYYYC

SEQ ID NO: 107 - protein, 15 aa, synthetic construct
  REGION 1..15: note = Synthesized polypeptide
  MOD_RES 3: note = METHYLATION
  MOD_RES 14: note = METHYLATION
AVFVWNYFIIRRYYC

SEQ ID NO: 108 - protein, 15 aa, synthetic construct
  REGION 1..15: note = Synthesized polypeptide
  MOD_RES 1: note = METHYLATION
  MOD_RES 3: note = METHYLATION
  MOD_RES 14: note = METHYLATION
AVFVWNYYIIRRYYC

SEQ ID NO: 109 - protein, 15 aa, synthetic construct
  REGION 1..15: note = Synthesized polypeptide
  MOD_RES 3: note = METHYLATION
  SITE 5: note = MISC_FEATURE - Xaa is F3C
  MOD_RES 14: note = METHYLATION
AVFVXNYYIIRRYYC

SEQ ID NO: 110 - protein, 15 aa, synthetic construct
  REGION 1..15: note = Synthesized polypeptide
  MOD_RES 3: note = METHYLATION
  MOD_RES 14: note = METHYLATION
AAFVWNYYIIRRYYC

SEQ ID NO: 111 - protein, 15 aa, synthetic construct
  REGION 1..15: note = Synthesized polypeptide
  SITE 1: note = MISC_FEATURE - Xaa is Alabu
  MOD_RES 3: note = METHYLATION
  MOD_RES 14: note = METHYLATION
XVFVWNYYIIRRYYC

SEQ ID NO: 112 - protein, 15 aa, synthetic construct
  REGION 1..15: note = Synthesized polypeptide
  MOD_RES 3: note = METHYLATION
  SITE 11: note = MISC_FEATURE - Xaa is MeAlarg
  MOD_RES 14: note = METHYLATION
AVFVWNYYIIXRYYC

SEQ ID NO: 113 - protein, 15 aa, synthetic construct
  REGION 1..15: note = Synthesized polypeptide
  MOD_RES 3: note = METHYLATION
  SITE 5: note = MISC_FEATURE - Xaa is F3OMe
  MOD_RES 14: note = METHYLATION
AVFVXNYYIIRRYYC

SEQ ID NO: 114 - protein, 15 aa, synthetic construct
  REGION 1..15: note = Synthesized polypeptide
  MOD_RES 3: note = METHYLATION
  SITE 5: note = MISC_FEATURE - Xaa is F4C
  MOD_RES 14: note = METHYLATION
AVFVXNYYIIRRYYC

SEQ ID NO: 115 - protein, 15 aa, synthetic construct
  REGION 1..15: note = Synthesized polypeptide
  MOD_RES 3: note = METHYLATION
  MOD_RES 14: note = METHYLATION
AVFVWNYYIYRRYYC

SEQ ID NO: 116 - protein, 15 aa, synthetic construct
  REGION 1..15: note = Synthesized polypeptide
  MOD_RES 3: note = METHYLATION
  SITE 12: note = MISC_FEATURE - Xaa is dr
  MOD_RES 14: note = METHYLATION
AVFVWNYYIIRXYYC

SEQ ID NO: 117 - protein, 15 aa, synthetic construct
  REGION 1..15: note = Synthesized polypeptide
  MOD_RES 3: note = METHYLATION
AVFVWNYYIIRRYAC

SEQ ID NO: 118 - protein, 15 aa, synthetic construct
  REGION 1..15: note = Synthesized polypeptide
  MOD_RES 3: note = METHYLATION
  SITE 5: note = MISC_FEATURE - Xaa is F4OMe
  MOD_RES 14: note = METHYLATION
AVFVXNYYIIRRYYC

SEQ ID NO: 119 - protein, 15 aa, synthetic construct
  REGION 1..15: note = Synthesized polypeptide
  MOD_RES 3: note = METHYLATION
  SITE 5: note = MISC_FEATURE - Xaa is F4F
  MOD_RES 14: note = METHYLATION
AVFVXNYYIIRRYYC

SEQ ID NO: 120 - protein, 15 aa, synthetic construct
  REGION 1..15: note = Synthesized polypeptide
  MOD_RES 3: note = METHYLATION
  MOD_RES 8: note = METHYLATION
  MOD_RES 14: note = METHYLATION
AVFVWNYYIIRRYYC

SEQ ID NO: 121 - protein, 15 aa, synthetic construct
  REGION 1..15: note = Synthesized polypeptide
  MOD_RES 3: note = METHYLATION
  MOD_RES 14: note = METHYLATION
AVFVWNYYIIYRYYC

SEQ ID NO: 122 - protein, 15 aa, synthetic construct
  REGION 1..15: note = Synthesized polypeptide
  MOD_RES 3: note = METHYLATION
  SITE 5: note = MISC_FEATURE - Xaa is F3F
  MOD_RES 14: note = METHYLATION
AVFVXNYYIIRRYYC

SEQ ID NO: 123 - protein, 15 aa, synthetic construct
  REGION 1..15: note = Synthesized polypeptide
  MOD_RES 3: note = METHYLATION
  MOD_RES 14: note = METHYLATION
AVFVWNYYIIRRAYC

SEQ ID NO: 124 - protein, 15 aa, synthetic construct
  REGION 1..15: note = Synthesized polypeptide
  MOD_RES 3: note = METHYLATION
AVFVWNYYIIRRYEC

SEQ ID NO: 125 - protein, 15 aa, synthetic construct
  REGION 1..15: note = Synthesized polypeptide
  MOD_RES 3: note = METHYLATION
  MOD_RES 14: note = METHYLATION
AVFVWNWYIIRRYYC

SEQ ID NO: 126 - protein, 15 aa, synthetic construct
  REGION 1..15: note = Synthesized polypeptide
  MOD_RES 3: note = METHYLATION
  MOD_RES 14: note = METHYLATION
AVFGWNYYIIRRYYC

SEQ ID NO: 127 - protein, 15 aa, synthetic construct
  REGION 1..15: note = Synthesized polypeptide
  MOD_RES 3: note = METHYLATION
AVFVWNYYIIRRYRC

SEQ ID NO: 128 - protein, 15 aa, synthetic construct
  REGION 1..15: note = Synthesized polypeptide
  MOD_RES 3: note = METHYLATION
  SITE 5: note = MISC_FEATURE - Xaa is Hph
  MOD_RES 14: note = METHYLATION
AVFVXNYYIIRRYYC

SEQ ID NO: 129 - protein, 15 aa, synthetic construct
  REGION 1..15: note = Synthesized polypeptide
  MOD_RES 3: note = METHYLATION
  MOD_RES 14: note = METHYLATION
AVFVWNYYIARRYYC

SEQ ID NO: 130 - protein, 15 aa, synthetic construct
  REGION 1..15: note = Synthesized polypeptide
  SITE 2: note = MISC_FEATURE - Xaa is Alahp
  MOD_RES 3: note = METHYLATION
  MOD_RES 14: note = METHYLATION
AXFVWNYYIIRRYYC

SEQ ID NO: 131 - protein, 15 aa, synthetic construct
  REGION 1..15: note = Synthesized polypeptide
  MOD_RES 3: note = METHYLATION
  MOD_RES 14: note = METHYLATION
GVFVWNYYIIRRYYC

SEQ ID NO: 132 - protein, 15 aa, synthetic construct
  REGION 1..15: note = Synthesized polypeptide
  MOD_RES 3: note = METHYLATION
  MOD_RES 14: note = METHYLATION
SVFVWNYYIIRRYYC

SEQ ID NO: 133 - protein, 15 aa, synthetic construct
  REGION 1..15: note = Synthesized polypeptide
  MOD_RES 3: note = METHYLATION
  MOD_RES 14: note = METHYLATION
AFFVWNYYIIRRYYC

SEQ ID NO: 134 - protein, 15 aa, synthetic construct
  REGION 1..15: note = Synthesized polypeptide
  MOD_RES 3: note = METHYLATION
  MOD_RES 14: note = METHYLATION
AVFVWDYYIIRRYYC

SEQ ID NO: 135 - protein, 15 aa, synthetic construct
  REGION 1..15: note = Synthesized polypeptide
  MOD_RES 3: note = METHYLATION
  MOD_RES 14: note = METHYLATION
AVFVWNFYIIRRYYC

SEQ ID NO: 136 - protein, 15 aa, synthetic construct
  REGION 1..15: note = Synthesized polypeptide
  SITE 3: note = MISC_FEATURE - Xaa is MePhe4OMe
  MOD_RES 14: note = METHYLATION
AVXVWNYYIIRRYYC

SEQ ID NO: 137 - protein, 15 aa, synthetic construct
  REGION 1..15: note = Synthesized polypeptide
  MOD_RES 3: note = METHYLATION
  MOD_RES 14: note = METHYLATION
AVFVWAYYIIRRYYC

SEQ ID NO: 138 - protein, 15 aa, synthetic construct
  REGION 1..15: note = Synthesized polypeptide
  MOD_RES 3: note = METHYLATION
  MOD_RES 14: note = METHYLATION
FVFVWNYYIIRRYYC

SEQ ID NO: 139 - protein, 15 aa, synthetic construct
  REGION 1..15: note = Synthesized polypeptide
  MOD_RES 3: note = METHYLATION
  SITE 8: note = MISC_FEATURE - Xaa is Alahp
  MOD_RES 14: note = METHYLATION
AVFVWNYXIIRRYYC

SEQ ID NO: 140 - protein, 15 aa, synthetic construct
  REGION 1..15: note = Synthesized polypeptide
  MOD_RES 3: note = METHYLATION
  MOD_RES 14: note = METHYLATION
AVFVWNAYIIRRYYC

SEQ ID NO: 141 - protein, 15 aa, synthetic construct
  REGION 1..15: note = Synthesized polypeptide
  MOD_RES 3: note = METHYLATION
  MOD_RES 14: note = METHYLATION
AVFSWNYYIIRRYYC

SEQ ID NO: 142 - protein, 15 aa, synthetic construct
  REGION 1..15: note = Synthesized polypeptide
  MOD_RES 3: note = METHYLATION
  SITE 7: note = MISC_FEATURE - Xaa is F4C
  MOD_RES 14: note = METHYLATION
AVFVWNXYIIRRYYC

SEQ ID NO: 143 - protein, 15 aa, synthetic construct
  REGION 1..15: note = Synthesized polypeptide
  MOD_RES 3: note = METHYLATION
  SITE 7: note = MISC_FEATURE - Xaa is Alahp
  MOD_RES 14: note = METHYLATION
AVFVWNXYIIRRYYC

SEQ ID NO: 144 - protein, 15 aa, synthetic construct
  REGION 1..15: note = Synthesized polypeptide
  MOD_RES 3: note = METHYLATION
  MOD_RES 14: note = METHYLATION
AVFAWNYYIIRRYYC

SEQ ID NO: 145 - protein, 15 aa, synthetic construct
  REGION 1..15: note = Synthesized polypeptide
  MOD_RES 3: note = METHYLATION
  MOD_RES 14: note = METHYLATION
AVFVWNRYIIRRYYC

SEQ ID NO: 146 - protein, 15 aa, synthetic construct
  REGION 1..15: note = Synthesized polypeptide
  MOD_RES 14: note = METHYLATION
AVFVWNYYIIRRYYC

SEQ ID NO: 147 - protein, 15 aa, synthetic construct
  REGION 1..15: note = Synthesized polypeptide
  MOD_RES 14: note = METHYLATION
AVFVWNYYIIRRYYC

SEQ ID NO: 148 - protein, 15 aa, synthetic construct
  REGION 1..15: note = Synthesized polypeptide
AVFVWNYYIIDRFRC

SEQ ID NO: 149 - protein, 17 aa, synthetic construct
  REGION 1..17: note = Synthesized polypeptide
  MOD_RES 16: note = METHYLATION
AVFVWNYYIIDRFRSHC

SEQ ID NO: 150 - protein, 17 aa, synthetic construct
  REGION 1..17: note = Synthesized polypeptide
  MOD_RES 16: note = METHYLATION
AVFVWNYYIIDRFRSYC

SEQ ID NO: 151 - protein, 17 aa, synthetic construct
  REGION 1..17: note = Synthesized polypeptide
AVFVWNYYIVDRFGTGC

SEQ ID NO: 152 - protein, 17 aa, synthetic construct
  REGION 1..17: note = Synthesized polypeptide
AVFVWNYYIVGRNVPNC

SEQ ID NO: 153 - protein, 17 aa, synthetic construct
  REGION 1..17: note = Synthesized polypeptide
  MOD_RES 16: note = METHYLATION
ANRIVFVWNYYIIPRYC

SEQ ID NO: 154 - protein, 17 aa, synthetic construct
  REGION 1..17: note = Synthesized polypeptide
  MOD_RES 16: note = METHYLATION
ANRIVFVWNYYIIPRHC

SEQ ID NO: 155 - protein, 17 aa, synthetic construct
  REGION 1..17: note = Synthesized polypeptide
ASAVFVWNYYIINRWAC

SEQ ID NO: 156 - protein, 17 aa, synthetic construct
  REGION 1..17: note = Synthesized polypeptide
  SITE 11: note = MISC_FEATURE - Xaa is PeG
AVFVWNYYIVXNGSNSC

SEQ ID NO: 157 - protein, 17 aa, synthetic construct
  REGION 1..17: note = Synthesized polypeptide
ANSRTVWVWNYYIVTRC

SEQ ID NO: 158 - protein, 15 aa, synthetic construct
  REGION 1..15: note = Synthesized polypeptide
  MOD_RES 2: note = METHYLATION
AYYRRIIYYNWVFVC

SEQ ID NO: 159 - protein, 15 aa, synthetic construct
  REGION 1..15: note = Synthesized polypeptide
  MOD_RES 14: note = METHYLATION
AVFVWNYYIIRRYYC

SEQ ID NO: 160 - protein, 15 aa, synthetic construct
  REGION 1..15: note = Synthesized polypeptide
  MOD_RES 14: note = METHYLATION
  SITE 15: note = MISC_FEATURE - Xaa is dc
AVFVWNYYIIRRYYX

SEQ ID NO: 161 - protein, 15 aa, synthetic construct
  REGION 1..15: note = Synthesized polypeptide
  MOD_RES 1: note = METHYLATION
  MOD_RES 14: note = METHYLATION
AVFVWNYYIIRRYYC

SEQ ID NO: 162 - protein, 15 aa, synthetic construct
  REGION 1..15: note = Synthesized polypeptide
  MOD_RES 3: note = METHYLATION
  MOD_RES 14: note = METHYLATION
AVFVWNYYIIRRYYC

SEQ ID NO: 163 - protein, 15 aa, synthetic construct
  REGION 1..15: note = Synthesized polypeptide
  MOD_RES 5: note = METHYLATION
  MOD_RES 14: note = METHYLATION
AVFVWNYYIIRRYYC

SEQ ID NO: 164 - protein, 15 aa, synthetic construct
  REGION 1..15: note = Synthesized polypeptide
  MOD_RES 11: note = METHYLATION
  MOD_RES 14: note = METHYLATION
AVFVWNYYIIRRYYC

SEQ ID NO: 165 - protein, 15 aa, synthetic construct
  REGION 1..15: note = Synthesized polypeptide
  MOD_RES 14: note = METHYLATION
AVFVWNYYIIRRYYC

SEQ ID NO: 166 - protein, 15 aa, synthetic construct
  REGION 1..15: note = Synthesized polypeptide
  MOD_RES 3: note = METHYLATION
  MOD_RES 14: note = METHYLATION
AVFVWNYYIIRRYYC

SEQ ID NO: 167 - protein, 15 aa, synthetic construct
  REGION 1..15: note = Synthesized polypeptide
  MOD_RES 3: note = METHYLATION
  MOD_RES 14: note = METHYLATION
AVFVWNYYIIKRYYC

SEQ ID NO: 168 - protein, 15 aa, synthetic construct
  REGION 1..15: note = Synthesized polypeptide
  MOD_RES 3: note = METHYLATION
  MOD_RES 5: note = METHYLATION
  MOD_RES 14: note = METHYLATION
AVFVWNYYIIRRYYC

SEQ ID NO: 169 - protein, 15 aa, synthetic construct
  REGION 1..15: note = Synthesized polypeptide
  MOD_RES 3: note = METHYLATION
  MOD_RES 5: note = METHYLATION
  MOD_RES 14: note = METHYLATION
AVFVWNYYIIKRYYC

SEQ ID NO: 170 - protein, 15 aa, synthetic construct
  REGION 1..15: note = Synthesized polypeptide
  MOD_RES 3: note = METHYLATION
  MOD_RES 5: note = METHYLATION
  MOD_RES 14: note = METHYLATION
AVFVWNYYIIKRYYC

SEQ ID NO: 171 - protein, 15 aa, synthetic construct
  REGION 1..15: note = Synthesized polypeptide
  MOD_RES 5: note = METHYLATION
  MOD_RES 14: note = METHYLATION
AVFVWNYYIIRRYYC

SEQ ID NO: 172 - protein, 15 aa, synthetic construct
  REGION 1..15: note = Synthesized polypeptide
  MOD_RES 5: note = METHYLATION
  MOD_RES 14: note = METHYLATION
AVFVWNYYIIKRYYC

SEQ ID NO: 173 - protein, 15 aa, synthetic construct
  REGION 1..15: note = Synthesized polypeptide
  MOD_RES 5: note = METHYLATION
  MOD_RES 14: note = METHYLATION
AVFVWNYYIIKRYYC

SEQ ID NO: 174 - protein, 15 aa, synthetic construct
  REGION 1..15: note = Synthesized polypeptide
  MOD_RES 3: note = METHYLATION
  MOD_RES 5: note = METHYLATION
  SITE 12: note = MISC_FEATURE - Xaa is Orn
  MOD_RES 14: note = METHYLATION
AVFVWNYYIIKXYYC

SEQ ID NO: 175 - protein, 15 aa, synthetic construct
  REGION 1..15: note = Synthesized polypeptide
  MOD_RES 3: note = METHYLATION
  MOD_RES 5: note = METHYLATION
  SITE 11: note = MISC_FEATURE - Xaa is Hly
  MOD_RES 14: note = METHYLATION
AVFVWNYYIIXRYYC

SEQ ID NO: 176 - protein, 15 aa, synthetic construct
  REGION 1..15: note = Synthesized polypeptide
  MOD_RES 3: note = METHYLATION
  MOD_RES 5: note = METHYLATION
  SITE 11: note = MISC_FEATURE - Xaa is Orn
  MOD_RES 14: note = METHYLATION
AVFVWNYYIIXRYYC

SEQ ID NO: 177 - protein, 15 aa, synthetic construct
  REGION 1..15: note = Synthesized polypeptide
  MOD_RES 3: note = METHYLATION
  MOD_RES 5: note = METHYLATION
  SITE 11: note = MISC_FEATURE - Xaa is Dap
  MOD_RES 14: note = METHYLATION
AVFVWNYYIIXRYYC

SEQ ID NO: 178 - protein, 15 aa, synthetic construct
  REGION 1..15: note = Synthesized polypeptide
  MOD_RES 3: note = METHYLATION
  MOD_RES 5: note = METHYLATION
  SITE 14: note = MISC_FEATURE - Xaa is MemBph
AVFVWNYYIIKRYXC

SEQ ID NO: 179 - protein, 15 aa, synthetic construct
  REGION 1..15: note = Synthesized polypeptide
  MOD_RES 3: note = METHYLATION
  MOD_RES 5: note = METHYLATION
  SITE 7: note = MISC_FEATURE - Xaa is Nal1
  MOD_RES 14: note = METHYLATION
AVFVWNXYIIKRYYC

SEQ ID NO: 180 - protein, 15 aa, synthetic construct
  REGION 1..15: note = Synthesized polypeptide
  MOD_RES 3: note = METHYLATION
  MOD_RES 5: note = METHYLATION
  MOD_RES 14: note = METHYLATION
AVFVWNYYIPKRYYC

SEQ ID NO: 181 - protein, 15 aa, synthetic construct
  REGION 1..15: note = Synthesized polypeptide
  MOD_RES 3: note = METHYLATION
  MOD_RES 14: note = METHYLATION
AVFVWNYYIIRRYYC

SEQ ID NO: 182 - protein, 15 aa, synthetic construct
  REGION 1..15: note = Synthesized polypeptide
  MOD_RES 3: note = METHYLATION
  MOD_RES 14: note = METHYLATION
AVFVWNYYIIRRYYC

SEQ ID NO: 183 - protein, 15 aa, synthetic construct
  REGION 1..15: note = Synthesized polypeptide
  MOD_RES 3: note = METHYLATION
  MOD_RES 5: note = METHYLATION
  MOD_RES 14: note = METHYLATION
AVFVWNYYIIRRYYC

SEQ ID NO: 184 - protein, 15 aa, synthetic construct
  REGION 1..15: note = Synthesized polypeptide
  MOD_RES 3: note = METHYLATION
  MOD_RES 5: note = METHYLATION
  MOD_RES 14: note = METHYLATION
AVFVWNYYIIRRYYC

SEQ ID NO: 185 - protein, 15 aa, synthetic construct
  REGION 1..15: note = Synthesized polypeptide
  MOD_RES 3: note = METHYLATION
  MOD_RES 5: note = METHYLATION
  MOD_RES 14: note = METHYLATION
AVFVWNYYIIRRYYC

SEQ ID NO: 186 - protein, 15 aa, synthetic construct
  REGION 1..15: note = Synthesized polypeptide
  MOD_RES 3: note = METHYLATION
  MOD_RES 14: note = METHYLATION
AVFVWNYYIIRRYYC

SEQ ID NO: 187 - protein, 15 aa, synthetic construct
  REGION 1..15: note = Synthesized polypeptide
  MOD_RES 3: note = METHYLATION
  MOD_RES 14: note = METHYLATION
AVFVWNYYIIRRYYC

SEQ ID NO: 188 - protein, 15 aa, synthetic construct
  REGION 1..15: note = Synthesized polypeptide
  MOD_RES 3: note = METHYLATION
  MOD_RES 14: note = METHYLATION
AVFVWNYYIIRRYYC

SEQ ID NO: 189 - protein, 15 aa, synthetic construct
  REGION 1..15: note = Synthesized polypeptide
  MOD_RES 3: note = METHYLATION
  MOD_RES 14: note = METHYLATION
AVFVWNYYIIRRYYC

SEQ ID NO: 190 - protein, 15 aa, synthetic construct
  REGION 1..15: note = Synthesized polypeptide
  MOD_RES 3: note = METHYLATION
  MOD_RES 14: note = METHYLATION
AVFVWNYYIIRRYYC

SEQ ID NO: 191 - protein, 15 aa, synthetic construct
  REGION 1..15: note = Synthesized polypeptide
  MOD_RES 3: note = METHYLATION
  MOD_RES 14: note = METHYLATION
AVFVWNYYIIRRYYC

SEQ ID NO: 192 - protein, 15 aa, synthetic construct
  REGION 1..15: note = Synthesized polypeptide
  MOD_RES 3: note = METHYLATION
  MOD_RES 14: note = METHYLATION
AVFVWNYYIIRRYYC

SEQ ID NO: 193 - protein, 15 aa, synthetic construct
  REGION 1..15: note = Synthesized polypeptide
  MOD_RES 3: note = METHYLATION
  MOD_RES 14: note = METHYLATION
AVFVWNYYIIRRYYC

SEQ ID NO: 194 - protein, 15 aa, synthetic construct
  REGION 1..15: note = Synthesized polypeptide
  MOD_RES 3: note = METHYLATION
  MOD_RES 14: note = METHYLATION
AVFVWNYYIIRRYYC

SEQ ID NO: 195 - protein, 15 aa, synthetic construct
  REGION 1..15: note = Synthesized polypeptide
  MOD_RES 3: note = METHYLATION
  MOD_RES 14: note = METHYLATION
AVFVWNYYIIRRYYC

SEQ ID NO: 196 - protein, 15 aa, synthetic construct
  REGION 1..15: note = Synthesized polypeptide
  MOD_RES 3: note = METHYLATION
  MOD_RES 14: note = METHYLATION
AVFVWNYYIIRRYYC

SEQ ID NO: 197 - protein, 15 aa, synthetic construct
  REGION 1..15: note = Synthesized polypeptide
  MOD_RES 5: note = METHYLATION
  MOD_RES 14: note = METHYLATION
AVFVWNYYIIRRYYC

SEQ ID NO: 198 - protein, 15 aa, synthetic construct
  REGION 1..15: note = Synthesized polypeptide
  MOD_RES 3: note = METHYLATION
  MOD_RES 5: note = METHYLATION
  MOD_RES 14: note = METHYLATION
AVFVWNYYIIRRYYC

SEQ ID NO: 199 - protein, 15 aa, synthetic construct
  REGION 1..15: note = Synthesized polypeptide
  MOD_RES 3: note = METHYLATION
  MOD_RES 5: note = METHYLATION
  MOD_RES 14: note = METHYLATION
AVFVWNYYIIRRYYC

SEQ ID NO: 200 - protein, 15 aa, synthetic construct
  REGION 1..15: note = Synthesized polypeptide
  MOD_RES 3: note = METHYLATION
  MOD_RES 5: note = METHYLATION
  MOD_RES 14: note = METHYLATION
AVFVWNYYIIRRYYC

SEQ ID NO: 201-202 - skipped (2 entries)

SEQ ID NO: 203 - protein, 12 aa, synthetic construct
  REGION 1..12: note = Synthesized polypeptide
  SITE 3: note = MISC_FEATURE - Xaa is MeF3C
  MOD_RES 5: note = METHYLATION
  SITE 8: note = MISC_FEATURE - Xaa is F4OMe
AEXVWNYXIISC

SEQ ID NO: 204 - protein, 12 aa, synthetic construct
  REGION 1..12: note = Synthesized polypeptide
AVFVWNYYIVHC

SEQ ID NO: 205 - protein, 12 aa, synthetic construct
  REGION 1..12: note = Synthesized polypeptide
  SITE 12: note = MISC_FEATURE - Xaa is Hgl
AVFVWNYYIISX

SEQ ID NO: 206 - protein, 14 aa, synthetic construct
  REGION 1..14: note = Synthesized polypeptide
  SITE 3: note = MISC_FEATURE - Xaa is MeF3C
  MOD_RES 5: note = METHYLATION
  SITE 8: note = MISC_FEATURE - Xaa is F4OMe
AEXVWNYXIVPREC

SEQ ID NO: 207 - protein, 14 aa, synthetic construct
  REGION 1..14: note = Synthesized polypeptide
  SITE 3: note = MISC_FEATURE - Xaa is MeF3C
  MOD_RES 5: note = METHYLATION
  SITE 8: note = MISC_FEATURE - Xaa is F4OMe
AEXVWNYXIVPRNC

SEQ ID NO: 208 - protein, 14 aa, synthetic construct
  REGION 1..14: note = Synthesized polypeptide
AVWVWNYFIIPRHC

SEQ ID NO: 209 - protein, 14 aa, synthetic construct
  REGION 1..14: note = Synthesized polypeptide
AVFVWNYYIVPRDC

SEQ ID NO: 210 - protein, 14 aa, synthetic construct
  REGION 1..14: note = Synthesized polypeptide
  MOD_RES 13: note = METHYLATION
AVFVWNYYIVPRWC

SEQ ID NO: 211 - protein, 14 aa, synthetic construct
  REGION 1..14: note = Synthesized polypeptide
AVFVWNYYIVPREC

SEQ ID NO: 212 - protein, 14 aa, synthetic construct
  REGION 1..14: note = Synthesized polypeptide
AVFVWNYYIVPRNC

SEQ ID NO: 213 - protein, 15 aa, synthetic construct
  REGION 1..15: note = Synthesized polypeptide
  MOD_RES 1: note = METHYLATION
  SITE 3: note = MISC_FEATURE - Xaa is MeF3C
  MOD_RES 5: note = METHYLATION
  SITE 8: note = MISC_FEATURE - Xaa is F4OMe
  MOD_RES 14: note = METHYLATION
AVXVWNYXIIKRFYC

SEQ ID NO: 214 - protein, 15 aa, synthetic construct
  REGION 1..15: note = Synthesized polypeptide
  MOD_RES 1: note = METHYLATION
  SITE 3: note = MISC_FEATURE - Xaa is MeF3C
  MOD_RES 5: note = METHYLATION
  SITE 8: note = MISC_FEATURE - Xaa is F4OMe
  MOD_RES 14: note = METHYLATION
AVXVWNYXIIRRFYC

SEQ ID NO: 215 - protein, 15 aa, synthetic construct
  REGION 1..15: note = Synthesized polypeptide
  MOD_RES 1: note = METHYLATION
  SITE 3: note = MISC_FEATURE - Xaa is MeF3C
  MOD_RES 5: note = METHYLATION
  SITE 8: note = MISC_FEATURE - Xaa is F4OMe
  SITE 12: note = MISC_FEATURE - Xaa is dr
  MOD_RES 14: note = METHYLATION
AVXVWNYXIIRXFYC

SEQ ID NO: 216 - protein, 15 aa, synthetic construct
  REGION 1..15: note = Synthesized polypeptide
  MOD_RES 1: note = METHYLATION
  SITE 3: note = MISC_FEATURE - Xaa is MeF3C
  MOD_RES 5: note = METHYLATION
  SITE 8: note = MISC_FEATURE - Xaa is F4OMe
  SITE 12: note = MISC_FEATURE - Xaa is da
  MOD_RES 14: note = METHYLATION
AVXVWNYXIIRXFYC

SEQ ID NO: 217 - protein, 15 aa, synthetic construct
  REGION 1..15: note = Synthesized polypeptide
  SITE 3: note = MISC_FEATURE - Xaa is MeF3C
  MOD_RES 5: note = METHYLATION
  SITE 8: note = MISC_FEATURE - Xaa is F4OMe
  MOD_RES 14: note = METHYLATION
EVXVWNYXIIRRFYC

SEQ ID NO: 218 - protein, 15 aa, synthetic construct
  REGION 1..15: note = Synthesized polypeptide
  MOD_RES 14: note = METHYLATION
EVFVWNYYIIRRYYC

SEQ ID NO: 219 - protein, 15 aa, synthetic construct
  REGION 1..15: note = Synthesized polypeptide
  MOD_RES 14: note = METHYLATION
AEFVWNYYIIRRYYC

SEQ ID NO: 220 - protein, 15 aa, synthetic construct
  REGION 1..15: note = Synthesized polypeptide
  MOD_RES 3: note = METHYLATION
  SITE 13: note = MISC_FEATURE - Xaa is KCOpipzaa
  MOD_RES 14: note = METHYLATION
AEFVWNYYIIRRXYC

SEQ ID NO: 221 - protein, 15 aa, synthetic construct
  REGION 1..15: note = Synthesized polypeptide
  MOD_RES 3: note = METHYLATION
  SITE 10: note = MISC_FEATURE - Xaa is KCOpipzaa
  MOD_RES 14: note = METHYLATION
AEFVWNYYIXRRYYC

SEQ ID NO: 222 - protein, 15 aa, synthetic construct
  REGION 1..15: note = Synthesized polypeptide
  SITE 3: note = MISC_FEATURE - Xaa is MeF3C
  SITE 8: note = MISC_FEATURE - Xaa is F4OMe
  SITE 12: note = MISC_FEATURE - Xaa is dr
  MOD_RES 14: note = METHYLATION
AEXVWNYXIIRXFYC

SEQ ID NO: 223 - protein, 15 aa, synthetic construct
  REGION 1..15: note = Synthesized polypeptide
  SITE 3: note = MISC_FEATURE - Xaa is MeF3C
  MOD_RES 5: note = METHYLATION
  SITE 8: note = MISC_FEATURE - Xaa is F4OMe
  SITE 12: note = MISC_FEATURE - Xaa is dr
  MOD_RES 14: note = METHYLATION
AEXVWNYXIERXFYC

SEQ ID NO: 224 - protein, 15 aa, synthetic construct
  REGION 1..15: note = Synthesized polypeptide
  SITE 3: note = MISC_FEATURE - Xaa is MeF3C
  MOD_RES 5: note = METHYLATION
  SITE 8: note = MISC_FEATURE - Xaa is F4OMe
  SITE 12: note = MISC_FEATURE - Xaa is dr
  MOD_RES 14: note = METHYLATION
AEXVWNYXIERXFYC

SEQ ID NO: 225 - protein, 15 aa, synthetic construct
  REGION 1..15: note = Synthesized polypeptide
  SITE 3: note = MISC_FEATURE - Xaa is MeF3C
  MOD_RES 5: note = METHYLATION
  SITE 8: note = MISC_FEATURE - Xaa is F4OMe
  MOD_RES 14: note = METHYLATION
AEXVWNYXIIAKFYC

SEQ ID NO: 226 - protein, 15 aa, synthetic construct
  REGION 1..15: note = Synthesized polypeptide
  SITE 3: note = MISC_FEATURE - Xaa is MeF3C
  MOD_RES 5: note = METHYLATION
  SITE 8: note = MISC_FEATURE - Xaa is F4OMe
  SITE 12: note = MISC_FEATURE - Xaa is dr
  MOD_RES 14: note = METHYLATION
AEXVWNYXIIAXFYC

SEQ ID NO: 227 - protein, 15 aa, synthetic construct
  REGION 1..15: note = Synthesized polypeptide
  SITE 3: note = MISC_FEATURE - Xaa is MeF3C
  MOD_RES 5: note = METHYLATION
  SITE 8: note = MISC_FEATURE - Xaa is F4OMe
AEXVWNYXIIDRFRC

SEQ ID NO: 228 - protein, 15 aa, synthetic construct
  REGION 1..15: note = Synthesized polypeptide
  SITE 3: note = MISC_FEATURE - Xaa is MeF3C
  MOD_RES 5: note = METHYLATION
  SITE 8: note = MISC_FEATURE - Xaa is F4OMe
  SITE 12: note = MISC_FEATURE - Xaa is dr
  MOD_RES 14: note = METHYLATION
AEXVWNYXIIKXFYC

SEQ ID NO: 229 - protein, 15 aa, synthetic construct
  REGION 1..15: note = Synthesized polypeptide
  SITE 3: note = MISC_FEATURE - Xaa is MeF3C
  MOD_RES 5: note = METHYLATION
  SITE 8: note = MISC_FEATURE - Xaa is F4OMe
  SITE 12: note = MISC_FEATURE - Xaa is dr
  MOD_RES 14: note = METHYLATION
AEXVWNYXIIKXFYC

SEQ ID NO: 230 - protein, 15 aa, synthetic construct
  REGION 1..15: note = Synthesized polypeptide
  SITE 3: note = MISC_FEATURE - Xaa is MeF3C
  MOD_RES 5: note = METHYLATION
  SITE 8: note = MISC_FEATURE - Xaa is F4OMe
  SITE 12: note = MISC_FEATURE - Xaa is dr
  MOD_RES 14: note = METHYLATION
AEXVWNYXIIKXFYC

SEQ ID NO: 231 - protein, 15 aa, synthetic construct
  REGION 1..15: note = Synthesized polypeptide
  SITE 3: note = MISC_FEATURE - Xaa is MeF3C
  MOD_RES 5: note = METHYLATION
  SITE 8: note = MISC_FEATURE - Xaa is F4OMe
  MOD_RES 14: note = METHYLATION
AEXVWNYXIIREFYC

SEQ ID NO: 232 - protein, 15 aa, synthetic construct
  REGION 1..15: note = Synthesized polypeptide
  SITE 3: note = MISC_FEATURE - Xaa is MeF3C
  MOD_RES 5: note = METHYLATION
  SITE 8: note = MISC_FEATURE - Xaa is F4OMe
  MOD_RES 14: note = METHYLATION
AEXVWNYXIIREFYC

SEQ ID NO: 233 - protein, 15 aa, synthetic construct
  REGION 1..15: note = Synthesized polypeptide
  SITE 3: note = MISC_FEATURE - Xaa is MeF3C
  MOD_RES 5: note = METHYLATION
  SITE 8: note = MISC_FEATURE - Xaa is F4OMe
  MOD_RES 14: note = METHYLATION
AEXVWNYXIIRRFYC

SEQ ID NO: 234 - protein, 15 aa, synthetic construct
  REGION 1..15: note = Synthesized polypeptide
  SITE 3: note = MISC_FEATURE - Xaa is MeF3C
  MOD_RES 5: note = METHYLATION
  SITE 8: note = MISC_FEATURE - Xaa is F4OMe
  SITE 12: note = MISC_FEATURE - Xaa is dr
  MOD_RES 14: note = METHYLATION
AEXVWNYXIIRXFYC

SEQ ID NO: 235 - protein, 15 aa, synthetic construct
  REGION 1..15: note = Synthesized polypeptide
  SITE 3: note = MISC_FEATURE - Xaa is MeF3C
  MOD_RES 5: note = METHYLATION
  SITE 8: note = MISC_FEATURE - Xaa is F4OMe
  SITE 12: note = MISC_FEATURE - Xaa is dr
  MOD_RES 14: note = METHYLATION
AEXVWNYXIIRXFYC

SEQ ID NO: 236 - protein, 15 aa, synthetic construct
  REGION 1..15: note = Synthesized polypeptide
  SITE 3: note = MISC_FEATURE - Xaa is MeF3C
  MOD_RES 5: note = METHYLATION
  SITE 8: note = MISC_FEATURE - Xaa is F4OMe
  SITE 12: note = MISC_FEATURE - Xaa is dr
  MOD_RES 14: note = METHYLATION
ADXVWNYXIIRXFYC

SEQ ID NO: 237 - protein, 15 aa, synthetic construct
  REGION 1..15: note = Synthesized polypeptide
  MOD_RES 14: note = METHYLATION
ARFVWNYYIIRRYYC

SEQ ID NO: 238 - protein, 15 aa, synthetic construct
  REGION 1..15: note = Synthesized polypeptide
  MOD_RES 14: note = METHYLATION
AKFVWNYYIIRRYYC

SEQ ID NO: 239 - protein, 15 aa, synthetic construct
  REGION 1..15: note = Synthesized polypeptide
  SITE 2: note = MISC_FEATURE - Xaa is Dap
  SITE 3: note = MISC_FEATURE - Xaa is MeF3C
  MOD_RES 5: note = METHYLATION
  SITE 8: note = MISC_FEATURE - Xaa is F4OMe
  SITE 12: note = MISC_FEATURE - Xaa is dr
  MOD_RES 14: note = METHYLATION
AXXVWNYXIIRXFYC

SEQ ID NO: 240 - protein, 15 aa, synthetic construct
  REGION 1..15: note = Synthesized polypeptide
  SITE 2: note = MISC_FEATURE - Xaa is E(PEG8Me)
  SITE 3: note = MISC_FEATURE - Xaa is MeF3C
  MOD_RES 5: note = METHYLATION
  SITE 8: note = MISC_FEATURE - Xaa is F4OMe
  SITE 12: note = MISC_FEATURE - Xaa is dr
  MOD_RES 14: note = METHYLATION
AXXVWNYXIIRXFYC

SEQ ID NO: 241 - protein, 15 aa, synthetic construct
  REGION 1..15: note = Synthesized polypeptide
  SITE 2: note = MISC_FEATURE - Xaa is E(de)
  SITE 3: note = MISC_FEATURE - Xaa is MeF3C
  MOD_RES 5: note = METHYLATION
  SITE 8: note = MISC_FEATURE - Xaa is F4OMe
  SITE 12: note = MISC_FEATURE - Xaa is dr
  MOD_RES 14: note = METHYLATION
AXXVWNYXIIRXFYC

SEQ ID NO: 242 - protein, 15 aa, synthetic construct
  REGION 1..15: note = Synthesized polypeptide
  SITE 2: note = MISC_FEATURE - Xaa is Har
  SITE 3: note = MISC_FEATURE - Xaa is MeF3C
  MOD_RES 5: note = METHYLATION
  SITE 8: note = MISC_FEATURE - Xaa is F4OMe
  SITE 12: note = MISC_FEATURE - Xaa is dr
  MOD_RES 14: note = METHYLATION
AXXVWNYXIIRXFYC

SEQ ID NO: 243 - protein, 15 aa, synthetic construct
  REGION 1..15: note = Synthesized polypeptide
  SITE 2: note = MISC_FEATURE - Xaa is Abu
  SITE 3: note = MISC_FEATURE - Xaa is MeF3C
  MOD_RES 5: note = METHYLATION
  SITE 8: note = MISC_FEATURE - Xaa is F4OMe
  SITE 12: note = MISC_FEATURE - Xaa is dr
  MOD_RES 14: note = METHYLATION
AXXVWNYXIIRXFYC

SEQ ID NO: 244 - protein, 15 aa, synthetic construct
  REGION 1..15: note = Synthesized polypeptide
  SITE 2: note = MISC_FEATURE - Xaa is Nva
  SITE 3: note = MISC_FEATURE - Xaa is MeF3C
  MOD_RES 5: note = METHYLATION
  SITE 8: note = MISC_FEATURE - Xaa is F4OMe
  SITE 12: note = MISC_FEATURE - Xaa is dr
  MOD_RES 14: note = METHYLATION
AXXVWNYXIIRXFYC

SEQ ID NO: 245 - protein, 15 aa, synthetic construct
  REGION 1..15: note = Synthesized polypeptide
  SITE 2: note = MISC_FEATURE - Xaa is Acpr
  SITE 3: note = MISC_FEATURE - Xaa is MeF3C
  MOD_RES 5: note = METHYLATION
  SITE 8: note = MISC_FEATURE - Xaa is F4OMe
  SITE 12: note = MISC_FEATURE - Xaa is dr
  MOD_RES 14: note = METHYLATION
AXXVWNYXIIRXFYC

SEQ ID NO: 246 - protein, 15 aa, synthetic construct
  REGION 1..15: note = Synthesized polypeptide
  SITE 2: note = MISC_FEATURE - Xaa is Atb
  SITE 3: note = MISC_FEATURE - Xaa is MeF3C
  MOD_RES 5: note = METHYLATION
  SITE 8: note = MISC_FEATURE - Xaa is F4OMe
  SITE 12: note = MISC_FEATURE - Xaa is dr
  MOD_RES 14: note = METHYLATION
AXXVWNYXIIRXFYC

SEQ ID NO: 247 - protein, 15 aa, synthetic construct
  REGION 1..15: note = Synthesized polypeptide
  MOD_RES 14: note = METHYLATION
AVFVWNYYIERRYYC

SEQ ID NO: 248 - protein, 15 aa, synthetic construct
  REGION 1..15: note = Synthesized polypeptide
  MOD_RES 14: note = METHYLATION
AVFVWNYYIRRRYYC

SEQ ID NO: 249 - protein, 15 aa, synthetic construct
  REGION 1..15: note = Synthesized polypeptide
  MOD_RES 14: note = METHYLATION
AVFVWNYYIKRRYYC

SEQ ID NO: 250 - protein, 15 aa, synthetic construct
  REGION 1..15: note = Synthesized polypeptide
  SITE 10: note = MISC_FEATURE - Xaa is Ahp
  MOD_RES 14: note = METHYLATION
AVFVWNYYIXRRYYC

SEQ ID NO: 251 - protein, 15 aa, synthetic construct
  REGION 1..15: note = Synthesized polypeptide
  MOD_RES 14: note = METHYLATION
AVFVWNYYIIERYYC

SEQ ID NO: 252 - protein, 15 aa, synthetic construct
  REGION 1..15: note = Synthesized polypeptide
  MOD_RES 14: note = METHYLATION
AVFVWNYYIIEAYYC

SEQ ID NO: 253 - protein, 15 aa, synthetic construct
  REGION 1..15: note = Synthesized polypeptide
  MOD_RES 14: note = METHYLATION
AVFVWNYYIIARYYC

SEQ ID NO: 254 - protein, 15 aa, synthetic construct
  REGION 1..15: note = Synthesized polypeptide
  MOD_RES 11: note = METHYLATION
  MOD_RES 14: note = METHYLATION
AVFVWNYYIIKRYYC

SEQ ID NO: 255 - protein, 15 aa, synthetic construct
  REGION 1..15: note = Synthesized polypeptide
  MOD_RES 14: note = METHYLATION
AVFVWNYYIIKRYYC

SEQ ID NO: 256 - protein, 15 aa, synthetic construct
  REGION 1..15: note = Synthesized polypeptide
  MOD_RES 14: note = METHYLATION
AVFVWNYYIIRAYYC

SEQ ID NO: 257 - protein, 15 aa, synthetic construct
  REGION 1..15: note = Synthesized polypeptide
  MOD_RES 14: note = METHYLATION
AVFVWNYYIIREYYC

SEQ ID NO: 258 - protein, 15 aa, synthetic construct
  REGION 1..15: note = Synthesized polypeptide
  MOD_RES 14: note = METHYLATION
AVFVWNYYIIRKYYC

SEQ ID NO: 259 - protein, 15 aa, synthetic construct
  REGION 1..15: note = Synthesized polypeptide
  MOD_RES 14: note = METHYLATION
AVFVWNYYIIRREYC

SEQ ID NO: 260 - protein, 15 aa, synthetic construct
  REGION 1..15: note = Synthesized polypeptide
  MOD_RES 14: note = METHYLATION
AVFVWNYYIIRRRYC

SEQ ID NO: 261 - protein, 15 aa, synthetic construct
  REGION 1..15: note = Synthesized polypeptide
  MOD_RES 14: note = METHYLATION
AVFVWNYYIIRRKYC

SEQ ID NO: 262 - protein, 15 aa, synthetic construct
  REGION 1..15: note = Synthesized polypeptide
AVFVWNYYIIRRFYC

SEQ ID NO: 263 - protein, 15 aa, synthetic construct
  REGION 1..15: note = Synthesized polypeptide
  MOD_RES 5: note = METHYLATION
  MOD_RES 14: note = METHYLATION
AVFVWNYYIIRRYYC

SEQ ID NO: 264 - protein, 15 aa, synthetic construct
  REGION 1..15: note = Synthesized polypeptide
  MOD_RES 5: note = METHYLATION
  MOD_RES 14: note = METHYLATION
AVFVWNYYIIRRYYC

SEQ ID NO: 265 - protein, 15 aa, synthetic construct
  REGION 1..15: note = Synthesized polypeptide
  SITE 3: note = MISC_FEATURE - Xaa is F3C
  MOD_RES 5: note = METHYLATION
  SITE 8: note = MISC_FEATURE - Xaa is F4OMe
  SITE 11: note = MISC_FEATURE - Xaa is Aib
  SITE 12: note = MISC_FEATURE - Xaa is dr
  MOD_RES 14: note = METHYLATION
AVXVWNYXIIXXFYC

SEQ ID NO: 266 - protein, 15 aa, synthetic construct
  REGION 1..15: note = Synthesized polypeptide
  MOD_RES 3: note = METHYLATION
  SITE 4: note = MISC_FEATURE - Xaa is Chg
  SITE 9: note = MISC_FEATURE - Xaa is Chg
  MOD_RES 14: note = METHYLATION
AVFXWNYYXIRRYYC

SEQ ID NO: 267 - protein, 15 aa, synthetic construct
  REGION 1..15: note = Synthesized polypeptide
  MOD_RES 3: note = METHYLATION
  SITE 4: note = MISC_FEATURE - Xaa is Chg
  SITE 9: note = MISC_FEATURE - Xaa is Chg
  MOD_RES 14: note = METHYLATION
AVFXWNYYXIRRYYC

SEQ ID NO: 268 - protein, 15 aa, synthetic construct
  REGION 1..15: note = Synthesized polypeptide
  MOD_RES 3: note = METHYLATION
  SITE 5: note = MISC_FEATURE - Xaa is W5C
  MOD_RES 14: note = METHYLATION
AVFVXNYYIIRRYYC

SEQ ID NO: 269 - protein, 15 aa, synthetic construct
  REGION 1..15: note = Synthesized polypeptide
  MOD_RES 3: note = METHYLATION
  SITE 5: note = MISC_FEATURE - Xaa is W5F
  MOD_RES 14: note = METHYLATION
AVFVXNYYIIRRYYC

SEQ ID NO: 270 - protein, 15 aa, synthetic construct
  REGION 1..15: note = Synthesized polypeptide
  MOD_RES 3: note = METHYLATION
  SITE 5: note = MISC_FEATURE - Xaa is W6F
  MOD_RES 14: note = METHYLATION
AVFVXNYYIIRRYYC

SEQ ID NO: 271 - protein, 15 aa, synthetic construct
  REGION 1..15: note = Synthesized polypeptide
  MOD_RES 3: note = METHYLATION
  SITE 5: note = MISC_FEATURE - Xaa is W1EtOH
  MOD_RES 14: note = METHYLATION
AVFVXNYYIIRRYYC

SEQ ID NO: 272 - protein, 15 aa, synthetic construct
  REGION 1..15: note = Synthesized polypeptide
  MOD_RES 3: note = METHYLATION
  SITE 5: note = MISC_FEATURE - Xaa is W5C
  SITE 12: note = MISC_FEATURE - Xaa is KCOpipzaa
  SITE 13: note = MISC_FEATURE - Xaa is KCOpipzaa
  MOD_RES 14: note = METHYLATION
AVFVXNYYIIRXXYC

SEQ ID NO: 273 - protein, 15 aa, synthetic construct
  REGION 1..15: note = Synthesized polypeptide
  MOD_RES 3: note = METHYLATION
  SITE 5: note = MISC_FEATURE - Xaa is W5C
  SITE 11: note = MISC_FEATURE - Xaa is E(PEG8Me)
  SITE 12: note = MISC_FEATURE - Xaa is KCOpipzaa
  SITE 13: note = MISC_FEATURE - Xaa is KCOpipzaa
  MOD_RES 14: note = METHYLATION
AVFVXNYYIIXXXYC

SEQ ID NO: 274 - protein, 15 aa, synthetic construct
  REGION 1..15: note = Synthesized polypeptide
  MOD_RES 3: note = METHYLATION
  MOD_RES 14: note = METHYLATION
AVFVWHYYIIRRYYC

SEQ ID NO: 275 - protein, 15 aa, synthetic construct
  REGION 1..15: note = Synthesized polypeptide
  MOD_RES 3: note = METHYLATION
  SITE 6: note = MISC_FEATURE - Xaa is Ndm
  MOD_RES 14: note = METHYLATION
AVFVWXYYIIRRYYC

SEQ ID NO: 276 - protein, 15 aa, synthetic construct
  REGION 1..15: note = Synthesized polypeptide
  MOD_RES 3: note = METHYLATION
  SITE 7: note = MISC_FEATURE - Xaa is F4C
  MOD_RES 14: note = METHYLATION
AVFVWNXYIIRRYYC

SEQ ID NO: 277 - protein, 15 aa, synthetic construct
  REGION 1..15: note = Synthesized polypeptide
  MOD_RES 3: note = METHYLATION
  SITE 7: note = MISC_FEATURE - Xaa is Ahp
  MOD_RES 14: note = METHYLATION
AVFVWNXYIIRRYYC

SEQ ID NO: 278 - protein, 15 aa, synthetic construct
  REGION 1..15: note = Synthesized polypeptide
  MOD_RES 3: note = METHYLATION
  SITE 8: note = MISC_FEATURE - Xaa is 4Py
  SITE 13: note = MISC_FEATURE - Xaa is 4Py
  MOD_RES 14: note = METHYLATION
AVFVWNYXIIRRXYC

SEQ ID NO: 279 - protein, 15 aa, synthetic construct
  REGION 1..15: note = Synthesized polypeptide
  MOD_RES 3: note = METHYLATION
  SITE 8: note = MISC_FEATURE - Xaa is 4Py
  SITE 10: note = MISC_FEATURE - Xaa is KCOpipzaa
  SITE 13: note = MISC_FEATURE - Xaa is 4Py
  MOD_RES 14: note = METHYLATION
AVFVWNYXIXRRXYC

SEQ ID NO: 280 - protein, 15 aa, synthetic construct
  REGION 1..15: note = Synthesized polypeptide
  MOD_RES 3: note = METHYLATION
  SITE 8: note = MISC_FEATURE - Xaa is 4Py
  SITE 10: note = MISC_FEATURE - Xaa is KCOpipzaa
  SITE 13: note = MISC_FEATURE - Xaa is KCOpipzaa
  MOD_RES 14: note = METHYLATION
AVFVWNYXIXRRXYC

SEQ ID NO: 281 - protein, 15 aa, synthetic construct
  REGION 1..15: note = Synthesized polypeptide
  MOD_RES 3: note = METHYLATION
  SITE 8: note = MISC_FEATURE - Xaa is 4Py
  SITE 10: note = MISC_FEATURE - Xaa is KCOpipzaa
  SITE 11: note = MISC_FEATURE - Xaa is KCOpipzaa
  SITE 13: note = MISC_FEATURE - Xaa is 4Py
  MOD_RES 14: note = METHYLATION
AVFVWNYXIXXRXYC

SEQ ID NO: 282 - protein, 15 aa, synthetic construct
  REGION 1..15: note = Synthesized polypeptide
  MOD_RES 3: note = METHYLATION
  SITE 9: note = MISC_FEATURE - Xaa is Chg
  MOD_RES 14: note = METHYLATION
AVFVWNYYXIRRYYC

SEQ ID NO: 283 - protein, 15 aa, synthetic construct
  REGION 1..15: note = Synthesized polypeptide
  MOD_RES 3: note = METHYLATION
  SITE 9: note = MISC_FEATURE - Xaa is Chg
  MOD_RES 14: note = METHYLATION
AVFVWNYYXIRRYYC

SEQ ID NO: 284 - protein, 15 aa, synthetic construct
  REGION 1..15: note = Synthesized polypeptide
  MOD_RES 3: note = METHYLATION
  SITE 10: note = MISC_FEATURE - Xaa is KCOpipzaa
  SITE 13: note = MISC_FEATURE - Xaa is KCOpipzaa
  MOD_RES 14: note = METHYLATION
AVFVWNYYIXRRXYC

SEQ ID NO: 285 - protein, 15 aa, synthetic construct
  REGION 1..15: note = Synthesized polypeptide
  MOD_RES 3: note = METHYLATION
  SITE 10: note = MISC_FEATURE - Xaa is KCOpipzaa
  SITE 11: note = MISC_FEATURE - Xaa is KCOpipzaa
  MOD_RES 14: note = METHYLATION
AVFVWNYYIXXRYYC

SEQ ID NO: 286 - protein, 15 aa, synthetic construct
  REGION 1..15: note = Synthesized polypeptide
  MOD_RES 3: note = METHYLATION
  SITE 11: note = MISC_FEATURE - Xaa is KCOpipzaa
  MOD_RES 14: note = METHYLATION
AVFVWNYYIIXRYYC

SEQ ID NO: 287 - protein, 15 aa, synthetic construct
  REGION 1..15: note = Synthesized polypeptide
  MOD_RES 3: note = METHYLATION
  SITE 11: note = MISC_FEATURE - Xaa is KCOpipzaa
  SITE 13: note = MISC_FEATURE - Xaa is KCOpipzaa
  MOD_RES 14: note = METHYLATION
AVFVWNYYIIXRXYC

SEQ ID NO: 288 - protein, 15 aa, synthetic construct
  REGION 1..15: note = Synthesized polypeptide
  MOD_RES 3: note = METHYLATION
  SITE 13: note = MISC_FEATURE - Xaa is KCOpipzaa
  MOD_RES 14: note = METHYLATION
AVFVWNYYIIERXYC

SEQ ID NO: 289 - protein, 15 aa, synthetic construct
  REGION 1..15: note = Synthesized polypeptide
  MOD_RES 3: note = METHYLATION
  SITE 12: note = MISC_FEATURE - Xaa is KCOpipzaa
  MOD_RES 14: note = METHYLATION
AVFVWNYYIIEXYYC

SEQ ID NO: 290 - protein, 15 aa, synthetic construct
  REGION 1..15: note = Synthesized polypeptide
  MOD_RES 3: note = METHYLATION
  SITE 11: note = MISC_FEATURE - Xaa is Aib
  SITE 12: note = MISC_FEATURE - Xaa is KCOpipzMe
  MOD_RES 14: note = METHYLATION
AVFVWNYYIIXXYYC

SEQ ID NO: 291 - protein, 15 aa, synthetic construct
  REGION 1..15: note = Synthesized polypeptide
  MOD_RES 3: note = METHYLATION
  MOD_RES 14: note = METHYLATION
AVFVWNYYIIARYYC

SEQ ID NO: 292 - protein, 15 aa, synthetic construct
  REGION 1..15: note = Synthesized polypeptide
  MOD_RES 3: note = METHYLATION
  MOD_RES 11: note = METHYLATION
  MOD_RES 14: note = METHYLATION
AVFVWNYYIIKRYYC

SEQ ID NO: 293 - protein, 15 aa, synthetic construct
  REGION 1..15: note = Synthesized polypeptide
  MOD_RES 3: note = METHYLATION
  MOD_RES 14: note = METHYLATION
AVFVWNYYIIKRYYC

SEQ ID NO: 294 - protein, 15 aa, synthetic construct
  REGION 1..15: note = Synthesized polypeptide
  MOD_RES 3: note = METHYLATION
  SITE 12: note = MISC_FEATURE - Xaa is KCOpipzaa
  SITE 13: note = MISC_FEATURE - Xaa is KCOpipzaa
  MOD_RES 14: note = METHYLATION
AVFVWNYYIIRXXYC

SEQ ID NO: 295 - protein, 15 aa, synthetic construct
  REGION 1..15: note = Synthesized polypeptide
  MOD_RES 3: note = METHYLATION
  SITE 13: note = MISC_FEATURE - Xaa is KCOpipzaa
  MOD_RES 14: note = METHYLATION
AVFVWNYYIIREXYC

SEQ ID NO: 296 - protein, 15 aa, synthetic construct
  REGION 1..15: note = Synthesized polypeptide
  MOD_RES 3: note = METHYLATION
  MOD_RES 14: note = METHYLATION
AVFVWNYYIIRRYYC

SEQ ID NO: 297 - protein, 15 aa, synthetic construct
  REGION 1..15: note = Synthesized polypeptide
  MOD_RES 3: note = METHYLATION
  MOD_RES 14: note = METHYLATION
AVFVWNYYIIRRYYC

SEQ ID NO: 298 - protein, 15 aa, synthetic construct
  REGION 1..15: note = Synthesized polypeptide
  MOD_RES 3: note = METHYLATION
  MOD_RES 14: note = METHYLATION
AVFVWNYYIIRRYYC

SEQ ID NO: 299 - protein, 15 aa, synthetic construct
  REGION 1..15: note = Synthesized polypeptide
  MOD_RES 3: note = METHYLATION
  MOD_RES 5: note = METHYLATION
  MOD_RES 14: note = METHYLATION
AVFVWNYYIIRRYYC

SEQ ID NO: 300 - protein, 15 aa, synthetic construct
  REGION 1..15: note = Synthesized polypeptide
  MOD_RES 3: note = METHYLATION
  MOD_RES 5: note = METHYLATION
  MOD_RES 14: note = METHYLATION
AVFVWNYYIIKRYYC

SEQ ID NO: 301 - protein, 15 aa, synthetic construct
  REGION 1..15: note = Synthesized polypeptide
  MOD_RES 3: note = METHYLATION
  MOD_RES 5: note = METHYLATION
  SITE 8: note = MISC_FEATURE - Xaa is F4OMe
  SITE 11: note = MISC_FEATURE - Xaa is Aib
  SITE 12: note = MISC_FEATURE - Xaa is dr
  MOD_RES 14: note = METHYLATION
AVFVWNYXIIXXFYC

SEQ ID NO: 302 - protein, 15 aa, synthetic construct
  REGION 1..15: note = Synthesized polypeptide
  SITE 3: note = MISC_FEATURE - Xaa is MeF35dC
  MOD_RES 5: note = METHYLATION
  SITE 12: note = MISC_FEATURE - Xaa is dr
  MOD_RES 14: note = METHYLATION
AVXVWNYYIIRXFYC

SEQ ID NO: 303 - protein, 15 aa, synthetic construct
  REGION 1..15: note = Synthesized polypeptide
  SITE 3: note = MISC_FEATURE - Xaa is MeF3C
  SITE 5: note = MISC_FEATURE - Xaa is W1aa
  SITE 8: note = MISC_FEATURE - Xaa is F4OMe
  SITE 11: note = MISC_FEATURE - Xaa is Aib
  SITE 12: note = MISC_FEATURE - Xaa is dr
  MOD_RES 14: note = METHYLATION
AVXVXNYXIIXXFYC

SEQ ID NO: 304 - protein, 15 aa, synthetic construct
  REGION 1..15: note = Synthesized polypeptide
  SITE 3: note = MISC_FEATURE - Xaa is MeF3C
  SITE 5: note = MISC_FEATURE - Xaa is W1mCON
  SITE 8: note = MISC_FEATURE - Xaa is F4OMe
  SITE 11: note = MISC_FEATURE - Xaa is Aib
  SITE 12: note = MISC_FEATURE - Xaa is dr
  MOD_RES 14: note = METHYLATION
AVXVXNYXIIXXFYC

SEQ ID NO: 305 - protein, 15 aa, synthetic construct
  REGION 1..15: note = Synthesized polypeptide
  SITE 3: note = MISC_FEATURE - Xaa is MeF3C
  SITE 5: note = MISC_FEATURE - Xaa is W1EtOH
  SITE 8: note = MISC_FEATURE - Xaa is F4OMe
  SITE 11: note = MISC_FEATURE - Xaa is Aib
  SITE 12: note = MISC_FEATURE - Xaa is dr
  MOD_RES 14: note = METHYLATION
AVXVXNYXIIXXFYC

SEQ ID NO: 306 - protein, 15 aa, synthetic construct
  REGION 1..15: note = Synthesized polypeptide
  SITE 3: note = MISC_FEATURE - Xaa is MeF3C
  SITE 5: note = MISC_FEATURE - Xaa is W1aa
  SITE 8: note = MISC_FEATURE - Xaa is F4OMe
  SITE 12: note = MISC_FEATURE - Xaa is dr
  MOD_RES 14: note = METHYLATION
AVXVXNYXIIRXFYC

SEQ ID NO: 307 - protein, 15 aa, synthetic construct
  REGION 1..15: note = Synthesized polypeptide
  SITE 3: note = MISC_FEATURE - Xaa is MeF3C
  MOD_RES 14: note = METHYLATION
AVXVWNYYIIDKFYC

SEQ ID NO: 308 - protein, 15 aa, synthetic construct
  REGION 1..15: note = Synthesized polypeptide
  SITE 3: note = MISC_FEATURE - Xaa is MeF3C
  SITE 11: note = MISC_FEATURE - Xaa is E(PEG8Me)
  SITE 12: note = MISC_FEATURE - Xaa is KCOpipzaa
  SITE 13: note = MISC_FEATURE - Xaa is KCOpipzaa
  MOD_RES 14: note = METHYLATION
AVXVWNYYIIXXXYC

SEQ ID NO: 309 - protein, 15 aa, synthetic construct
  REGION 1..15: note = Synthesized polypeptide
  SITE 3: note = MISC_FEATURE - Xaa is MeF3C
  SITE 12: note = MISC_FEATURE - Xaa is KCOpipzaa
  SITE 13: note = MISC_FEATURE - Xaa is KCOpipzaa
  MOD_RES 14: note = METHYLATION
AVXVWNYYIIRXXYC

SEQ ID NO: 310 - protein, 15 aa, synthetic construct
  REGION 1..15: note = Synthesized polypeptide
  SITE 3: note = MISC_FEATURE - Xaa is MeF3C
  SITE 8: note = MISC_FEATURE - Xaa is F4OMe
  SITE 11: note = MISC_FEATURE - Xaa is Aib
  SITE 12: note = MISC_FEATURE - Xaa is dr
  MOD_RES 14: note = METHYLATION
AVXVWNYXIIXXFYC

SEQ ID NO: 311 - protein, 15 aa, synthetic construct
  REGION 1..15: note = Synthesized polypeptide
  SITE 3: note = MISC_FEATURE - Xaa is MeF3C
  SITE 8: note = MISC_FEATURE - Xaa is F4OMe
  SITE 12: note = MISC_FEATURE - Xaa is dr
  MOD_RES 14: note = METHYLATION
AVXVWNYXIIRXFYC

SEQ ID NO: 312 - protein, 15 aa, synthetic construct
  REGION 1..15: note = Synthesized polypeptide
  SITE 3: note = MISC_FEATURE - Xaa is MeF3C
  SITE 8: note = MISC_FEATURE - Xaa is F4OMe
  MOD_RES 14: note = METHYLATION
AVXVWNYXIIRRFYC

SEQ ID NO: 313 - protein, 15 aa, synthetic construct
  REGION 1..15: note = Synthesized polypeptide
  SITE 3: note = MISC_FEATURE - Xaa is MeF3C
  SITE 8: note = MISC_FEATURE - Xaa is F4OMe
  SITE 12: note = MISC_FEATURE - Xaa is dk
  MOD_RES 14: note = METHYLATION
AVXVWNYXIIRXFYC

SEQ ID NO: 314 - protein, 15 aa, synthetic construct
  REGION 1..15: note = Synthesized polypeptide
  SITE 3: note = MISC_FEATURE - Xaa is MeF3C
  SITE 8: note = MISC_FEATURE - Xaa is F4OMe
  SITE 12: note = MISC_FEATURE - Xaa is dr
  MOD_RES 14: note = METHYLATION
AVXVWNYXIIKXFYC

SEQ ID NO: 315 - protein, 15 aa, synthetic construct
  REGION 1..15: note = Synthesized polypeptide
  SITE 3: note = MISC_FEATURE - Xaa is MeF3C
  MOD_RES 5: note = METHYLATION
  SITE 7: note = MISC_FEATURE - Xaa is 3Py6NH2
  SITE 8: note = MISC_FEATURE - Xaa is F4OMe
  SITE 12: note = MISC_FEATURE - Xaa is dr
  MOD_RES 14: note = METHYLATION
AVXVWNXXIIRXFYC

SEQ ID NO: 316 - protein, 15 aa, synthetic construct
  REGION 1..15: note = Synthesized polypeptide
  SITE 3: note = MISC_FEATURE - Xaa is MeF3C
  MOD_RES 5: note = METHYLATION
  SITE 7: note = MISC_FEATURE - Xaa is 4Py2NH2
  SITE 8: note = MISC_FEATURE - Xaa is F4OMe
  SITE 12: note = MISC_FEATURE - Xaa is dr
  MOD_RES 14: note = METHYLATION
AVXVWNXXIIRXFYC

SEQ ID NO: 317 - protein, 15 aa, synthetic construct
  REGION 1..15: note = Synthesized polypeptide
  SITE 3: note = MISC_FEATURE - Xaa is MeF3C
  MOD_RES 5: note = METHYLATION
  SITE 7: note = MISC_FEATURE - Xaa is F3H
  SITE 8: note = MISC_FEATURE - Xaa is F4OMe
  SITE 12: note = MISC_FEATURE - Xaa is dr
  MOD_RES 14: note = METHYLATION
AVXVWNXXIIRXFYC

SEQ ID NO: 318 - protein, 15 aa, synthetic construct
  REGION 1..15: note = Synthesized polypeptide
  SITE 3: note = MISC_FEATURE - Xaa is MeF3C
  MOD_RES 5: note = METHYLATION
  SITE 8: note = MISC_FEATURE - Xaa is F34dOMe
  SITE 12: note = MISC_FEATURE - Xaa is dr
  MOD_RES 14: note = METHYLATION
AVXVWNYXIIRXFYC

SEQ ID NO: 319 - protein, 15 aa, synthetic construct
  REGION 1..15: note = Synthesized polypeptide
  SITE 3: note = MISC_FEATURE - Xaa is MeF3C
  MOD_RES 5: note = METHYLATION
  SITE 8: note = MISC_FEATURE - Xaa is F4OEt
  SITE 12: note = MISC_FEATURE - Xaa is dr
  MOD_RES 14: note = METHYLATION
AVXVWNYXIIRXFYC

SEQ ID NO: 320 - protein, 15 aa, synthetic construct
  REGION 1..15: note = Synthesized polypeptide
  SITE 3: note = MISC_FEATURE - Xaa is MeF3C
  MOD_RES 5: note = METHYLATION
  SITE 8: note = MISC_FEATURE - Xaa is F4aao
  SITE 12: note = MISC_FEATURE - Xaa is dr
  MOD_RES 14: note = METHYLATION
AVXVWNYXIIRXFYC

SEQ ID NO: 321 - protein, 15 aa, synthetic construct
  REGION 1..15: note = Synthesized polypeptide
  SITE 3: note = MISC_FEATURE - Xaa is MeF3C
  MOD_RES 5: note = METHYLATION
  SITE 8: note = MISC_FEATURE - Xaa is Yae
  SITE 12: note = MISC_FEATURE - Xaa is dr
  MOD_RES 14: note = METHYLATION
AVXVWNYXIIRXFYC

SEQ ID NO: 322 - protein, 15 aa, synthetic construct
  REGION 1..15: note = Synthesized polypeptide
  SITE 3: note = MISC_FEATURE - Xaa is MeF3C
  MOD_RES 5: note = METHYLATION
  SITE 11: note = MISC_FEATURE - Xaa is Aib
  SITE 12: note = MISC_FEATURE - Xaa is dr
  MOD_RES 14: note = METHYLATION
AVXVWNYYIIXXFYC

SEQ ID NO: 323 - protein, 15 aa, synthetic construct
  REGION 1..15: note = Synthesized polypeptide
  SITE 3: note = MISC_FEATURE - Xaa is MeF3C
  MOD_RES 5: note = METHYLATION
  SITE 8: note = MISC_FEATURE - Xaa is 3Py6OMe
  SITE 11: note = MISC_FEATURE - Xaa is Aib
  SITE 12: note = MISC_FEATURE - Xaa is dr
  MOD_RES 14: note = METHYLATION
AVXVWNYXIIXXFYC

SEQ ID NO: 324 - protein, 15 aa, synthetic construct
  REGION 1..15: note = Synthesized polypeptide
  SITE 3: note = MISC_FEATURE - Xaa is MeF3C
  MOD_RES 5: note = METHYLATION
  SITE 8: note = MISC_FEATURE - Xaa is F4aao
  SITE 11: note = MISC_FEATURE - Xaa is Aib
  SITE 12: note = MISC_FEATURE - Xaa is dr
  MOD_RES 14: note = METHYLATION
AVXVWNYXIIXXFYC

SEQ ID NO: 325 - protein, 15 aa, synthetic construct
  REGION 1..15: note = Synthesized polypeptide
  SITE 3: note = MISC_FEATURE - Xaa is MeF3C
  MOD_RES 5: note = METHYLATION
  SITE 8: note = MISC_FEATURE - Xaa is F4OMe
  SITE 10: note = MISC_FEATURE - Xaa is Abu
  SITE 12: note = MISC_FEATURE - Xaa is dr
  MOD_RES 14: note = METHYLATION
AVXVWNYXIXRXFYC

SEQ ID NO: 326 - protein, 15 aa, synthetic construct
  REGION 1..15: note = Synthesized polypeptide
  SITE 3: note = MISC_FEATURE - Xaa is MeF3C
  MOD_RES 5: note = METHYLATION
  SITE 8: note = MISC_FEATURE - Xaa is F4OMe
  SITE 10: note = MISC_FEATURE - Xaa is Nva
  SITE 12: note = MISC_FEATURE - Xaa is dr
  MOD_RES 14: note = METHYLATION
AVXVWNYXIXRXFYC

SEQ ID NO: 327 - protein, 15 aa, synthetic construct
  REGION 1..15: note = Synthesized polypeptide
  SITE 3: note = MISC_FEATURE - Xaa is MeF3C
  MOD_RES 5: note = METHYLATION
  SITE 8: note = MISC_FEATURE - Xaa is F4OMe
  SITE 10: note = MISC_FEATURE - Xaa is Tbg
  SITE 12: note = MISC_FEATURE - Xaa is dr
  MOD_RES 14: note = METHYLATION
AVXVWNYXIXRXFYC

SEQ ID NO: 328 - protein, 15 aa, synthetic construct
  REGION 1..15: note = Synthesized polypeptide
  SITE 3: note = MISC_FEATURE - Xaa is MeF3C
  MOD_RES 5: note = METHYLATION
  SITE 8: note = MISC_FEATURE - Xaa is F4OMe
  SITE 10: note = MISC_FEATURE - Xaa is Acpr
  SITE 12: note = MISC_FEATURE - Xaa is dr
  MOD_RES 14: note = METHYLATION
AVXVWNYXIXRXFYC

SEQ ID NO: 329 - protein, 15 aa, synthetic construct
  REGION 1..15: note = Synthesized polypeptide
  SITE 3: note = MISC_FEATURE - Xaa is MeF3C
  MOD_RES 5: note = METHYLATION
  SITE 8: note = MISC_FEATURE - Xaa is F4OMe
  SITE 10: note = MISC_FEATURE - Xaa is Atb
  SITE 12: note = MISC_FEATURE - Xaa is dr
  MOD_RES 14: note = METHYLATION
AVXVWNYXIXRXFYC

SEQ ID NO: 330 - protein, 15 aa, synthetic construct
  REGION 1..15: note = Synthesized polypeptide
  SITE 3: note = MISC_FEATURE - Xaa is MeF3C
  MOD_RES 5: note = METHYLATION
  SITE 8: note = MISC_FEATURE - Xaa is F4OMe
  SITE 10: note = MISC_FEATURE - Xaa is alI
  SITE 12: note = MISC_FEATURE - Xaa is dr
  MOD_RES 14: note = METHYLATION
AVXVWNYXIXRXFYC

SEQ ID NO: 331 - protein, 15 aa, synthetic construct
  REGION 1..15: note = Synthesized polypeptide
  SITE 3: note = MISC_FEATURE - Xaa is MeF3C
  MOD_RES 5: note = METHYLATION
  SITE 8: note = MISC_FEATURE - Xaa is F4OMe
  SITE 12: note = MISC_FEATURE - Xaa is dr
  MOD_RES 14: note = METHYLATION
AVXVWNYXITRXFYC

SEQ ID NO: 332 - protein, 15 aa, synthetic construct
  REGION 1..15: note = Synthesized polypeptide
  SITE 3: note = MISC_FEATURE - Xaa is MeF3C
  MOD_RES 5: note = METHYLATION
  SITE 8: note = MISC_FEATURE - Xaa is F4OMe
  SITE 10: note = MISC_FEATURE - Xaa is alT
  SITE 12: note = MISC_FEATURE - Xaa is dr
  MOD_RES 14: note = METHYLATION
AVXVWNYXIXRXFYC

SEQ ID NO: 333 - protein, 15 aa, synthetic construct
  REGION 1..15: note = Synthesized polypeptide
  SITE 3: note = MISC_FEATURE - Xaa is MeF3C
  MOD_RES 5: note = METHYLATION
  SITE 8: note = MISC_FEATURE - Xaa is F4OMe
  SITE 10: note = MISC_FEATURE - Xaa is Aib
  SITE 12: note = MISC_FEATURE - Xaa is dr
  MOD_RES 14: note = METHYLATION
AVXVWNYXIXRXFYC

SEQ ID NO: 334 - protein, 15 aa, synthetic construct
  REGION 1..15: note = Synthesized polypeptide
  SITE 3: note = MISC_FEATURE - Xaa is MeF3C
  MOD_RES 5: note = METHYLATION
  SITE 8: note = MISC_FEATURE - Xaa is F4OMe
  SITE 10: note = MISC_FEATURE - Xaa is Nle
  SITE 12: note = MISC_FEATURE - Xaa is dr
  MOD_RES 14: note = METHYLATION
AVXVWNYXIXRXFYC

SEQ ID NO: 335 - protein, 15 aa, synthetic construct
  REGION 1..15: note = Synthesized polypeptide
  SITE 3: note = MISC_FEATURE - Xaa is MeF3C
  MOD_RES 5: note = METHYLATION
  SITE 8: note = MISC_FEATURE - Xaa is F4OMe
  SITE 10: note = MISC_FEATURE - Xaa is Ahp
  SITE 12: note = MISC_FEATURE - Xaa is dr
  MOD_RES 14: note = METHYLATION
AVXVWNYXIXRXFYC

SEQ ID NO: 336 - protein, 15 aa, synthetic construct
  REGION 1..15: note = Synthesized polypeptide
  SITE 3: note = MISC_FEATURE - Xaa is MeF3C
  MOD_RES 5: note = METHYLATION
  SITE 8: note = MISC_FEATURE - Xaa is F4OMe
  SITE 10: note = MISC_FEATURE - Xaa is Dap
  SITE 12: note = MISC_FEATURE - Xaa is dr
  MOD_RES 14: note = METHYLATION
AVXVWNYXIXRXFYC

SEQ ID NO: 337 - protein, 15 aa, synthetic construct
  REGION 1..15: note = Synthesized polypeptide
  SITE 3: note = MISC_FEATURE - Xaa is MeF3C
  MOD_RES 5: note = METHYLATION
  SITE 8: note = MISC_FEATURE - Xaa is F4OMe
  SITE 10: note = MISC_FEATURE - Xaa is Dab
  SITE 12: note = MISC_FEATURE - Xaa is dr
  MOD_RES 14: note = METHYLATION
AVXVWNYXIXRXFYC

SEQ ID NO: 338 - protein, 15 aa, synthetic construct
  REGION 1..15: note = Synthesized polypeptide
  SITE 3: note = MISC_FEATURE - Xaa is MeF3C
  MOD_RES 5: note = METHYLATION
  SITE 8: note = MISC_FEATURE - Xaa is F4OMe
  SITE 10: note = MISC_FEATURE - Xaa is dorn
  SITE 12: note = MISC_FEATURE - Xaa is dr
  MOD_RES 14: note = METHYLATION
AVXVWNYXIXRXFYC

SEQ ID NO: 339 - protein, 15 aa, synthetic construct
  REGION 1..15: note = Synthesized polypeptide
  SITE 3: note = MISC_FEATURE - Xaa is MeF3C
  MOD_RES 5: note = METHYLATION
  SITE 8: note = MISC_FEATURE - Xaa is F4OMe
  SITE 10: note = MISC_FEATURE - Xaa is Hly
  SITE 12: note = MISC_FEATURE - Xaa is dr
  MOD_RES 14: note = METHYLATION
AVXVWNYXIXRXFYC

SEQ ID NO: 340 - protein, 15 aa, synthetic construct
  REGION 1..15: note = Synthesized polypeptide
  SITE 3: note = MISC_FEATURE - Xaa is MeF3C
  MOD_RES 5: note = METHYLATION
  SITE 8: note = MISC_FEATURE - Xaa is F4OMe
  SITE 12: note = MISC_FEATURE - Xaa is dr
  MOD_RES 14: note = METHYLATION
AVXVWNYXIERXFYC

SEQ ID NO: 341 - protein, 15 aa, synthetic construct
  REGION 1..15: note = Synthesized polypeptide
  SITE 3: note = MISC_FEATURE - Xaa is MeF3C
  MOD_RES 5: note = METHYLATION
  SITE 8: note = MISC_FEATURE - Xaa is F4OMe
  SITE 10: note = MISC_FEATURE - Xaa is Hly
  SITE 12: note = MISC_FEATURE - Xaa is dr
  MOD_RES 14: note = METHYLATION
AVXVWNYXIXRXFYC

SEQ ID NO: 342 - protein, 15 aa, synthetic construct
  REGION 1..15: note = Synthesized polypeptide
  SITE 3: note = MISC_FEATURE - Xaa is MeF3C
  MOD_RES 5: note = METHYLATION
  SITE 8: note = MISC_FEATURE - Xaa is F4OMe
  SITE 12: note = MISC_FEATURE - Xaa is dr
  MOD_RES 14: note = METHYLATION
AVXVWNYXIERXFYC

SEQ ID NO: 343 - protein, 15 aa, synthetic construct
  REGION 1..15: note = Synthesized polypeptide
  SITE 3: note = MISC_FEATURE - Xaa is MeF3C
  MOD_RES 5: note = METHYLATION
  SITE 8: note = MISC_FEATURE - Xaa is F4OMe
  SITE 10: note = MISC_FEATURE - Xaa is Dap
  SITE 12: note = MISC_FEATURE - Xaa is dr
  MOD_RES 14: note = METHYLATION
AVXVWNYXIXRXFYC

SEQ ID NO: 344 - protein, 15 aa, synthetic construct
  REGION 1..15: note = Synthesized polypeptide
  SITE 3: note = MISC_FEATURE - Xaa is MeF3C
  MOD_RES 5: note = METHYLATION
  SITE 8: note = MISC_FEATURE - Xaa is F4OMe
  SITE 12: note = MISC_FEATURE - Xaa is dr
  MOD_RES 14: note = METHYLATION
AVXVWNYXIKRXFYC

SEQ ID NO: 345 - protein, 15 aa, synthetic construct
  REGION 1..15: note = Synthesized polypeptide
  SITE 3: note = MISC_FEATURE - Xaa is MeF3C
  MOD_RES 5: note = METHYLATION
  SITE 8: note = MISC_FEATURE - Xaa is F4OMe
  SITE 10: note = MISC_FEATURE - Xaa is E(PEG8Me)
  SITE 12: note = MISC_FEATURE - Xaa is dr
  MOD_RES 14: note = METHYLATION
AVXVWNYXIXRXFYC

SEQ ID NO: 346 - protein, 15 aa, synthetic construct
  REGION 1..15: note = Synthesized polypeptide
  SITE 3: note = MISC_FEATURE - Xaa is MeF3C
  MOD_RES 5: note = METHYLATION
  SITE 8: note = MISC_FEATURE - Xaa is F4OMe
  SITE 10: note = MISC_FEATURE - Xaa is E(e-Medk)
  SITE 12: note = MISC_FEATURE - Xaa is dr
  MOD_RES 14: note = METHYLATION
AVXVWNYXIXRXFYC

SEQ ID NO: 347 - protein, 15 aa, synthetic construct
  REGION 1..15: note = Synthesized polypeptide
  SITE 3: note = MISC_FEATURE - Xaa is MeF3C
  MOD_RES 5: note = METHYLATION
  SITE 8: note = MISC_FEATURE - Xaa is F4OMe
  SITE 10: note = MISC_FEATURE - Xaa is E(de)
  SITE 12: note = MISC_FEATURE - Xaa is dr
  MOD_RES 14: note = METHYLATION
AVXVWNYXIXRXFYC

SEQ ID NO: 348 - protein, 15 aa, synthetic construct
  REGION 1..15: note = Synthesized polypeptide
  SITE 3: note = MISC_FEATURE - Xaa is MeF3C
  MOD_RES 5: note = METHYLATION
  SITE 8: note = MISC_FEATURE - Xaa is F4OMe
  SITE 12: note = MISC_FEATURE - Xaa is dr
  MOD_RES 14: note = METHYLATION
AVXVWNYXIIEXFYC

SEQ ID NO: 349 - protein, 15 aa, synthetic construct
  REGION 1..15: note = Synthesized polypeptide
  SITE 3: note = MISC_FEATURE - Xaa is MeF3C
  MOD_RES 5: note = METHYLATION
  SITE 8: note = MISC_FEATURE - Xaa is F4OMe
  SITE 12: note = MISC_FEATURE - Xaa is dr
  MOD_RES 14: note = METHYLATION
AVXVWNYXIIAXFYC

SEQ ID NO: 350 - protein, 15 aa, synthetic construct
  REGION 1..15: note = Synthesized polypeptide
  SITE 3: note = MISC_FEATURE - Xaa is MeF3C
  MOD_RES 5: note = METHYLATION
  SITE 8: note = MISC_FEATURE - Xaa is F4OMe
  SITE 11: note = MISC_FEATURE - Xaa is Aib
  SITE 12: note = MISC_FEATURE - Xaa is KAc
  MOD_RES 14: note = METHYLATION
AVXVWNYXIIXXFYC

SEQ ID NO: 351 - protein, 15 aa, synthetic construct
  REGION 1..15: note = Synthesized polypeptide
  SITE 3: note = MISC_FEATURE - Xaa is MeF3C
  MOD_RES 5: note = METHYLATION
  SITE 8: note = MISC_FEATURE - Xaa is F4OMe
  SITE 11: note = MISC_FEATURE - Xaa is Aib
  MOD_RES 14: note = METHYLATION
AVXVWNYXIIXRFYC

SEQ ID NO: 352 - protein, 15 aa, synthetic construct
  REGION 1..15: note = Synthesized polypeptide
  SITE 3: note = MISC_FEATURE - Xaa is MeF3C
  MOD_RES 5: note = METHYLATION
  SITE 8: note = MISC_FEATURE - Xaa is F4OMe
  SITE 11: note = MISC_FEATURE - Xaa is Aib
  SITE 12: note = MISC_FEATURE - Xaa is dr
AVXVWNYXIIXXFYC

SEQ ID NO: 353 - protein, 15 aa, synthetic construct
  REGION 1..15: note = Synthesized polypeptide
  SITE 3: note = MISC_FEATURE - Xaa is MeF3C
  MOD_RES 5: note = METHYLATION
  SITE 8: note = MISC_FEATURE - Xaa is F4OMe
  SITE 11: note = MISC_FEATURE - Xaa is Aib
  SITE 12: note = MISC_FEATURE - Xaa is dr
  MOD_RES 14: note = METHYLATION
AVXVWNYXIIXXFYC

SEQ ID NO: 354 - protein, 15 aa, synthetic construct
  REGION 1..15: note = Synthesized polypeptide
  SITE 3: note = MISC_FEATURE - Xaa is MeF3C
  MOD_RES 5: note = METHYLATION
  SITE 8: note = MISC_FEATURE - Xaa is F4OMe
  SITE 11: note = MISC_FEATURE - Xaa is Aib
  SITE 12: note = MISC_FEATURE - Xaa is dr
  MOD_RES 14: note = METHYLATION
AVXVWNYXIIXXFYC

SEQ ID NO: 355 - protein, 15 aa, synthetic construct
  REGION 1..15: note = Synthesized polypeptide
  SITE 3: note = MISC_FEATURE - Xaa is MeF3C
  MOD_RES 5: note = METHYLATION
  SITE 8: note = MISC_FEATURE - Xaa is F4OMe
  SITE 11: note = MISC_FEATURE - Xaa is Aib
  SITE 12: note = MISC_FEATURE - Xaa is dr
  MOD_RES 14: note = METHYLATION
AVXVWNYXIIXXFYC

SEQ ID NO: 356 - protein, 15 aa, synthetic construct
  REGION 1..15: note = Synthesized polypeptide
  SITE 3: note = MISC_FEATURE - Xaa is MeF3C
  MOD_RES 5: note = METHYLATION
  SITE 8: note = MISC_FEATURE - Xaa is F4OMe
  SITE 11: note = MISC_FEATURE - Xaa is Aib
  SITE 12: note = MISC_FEATURE - Xaa is dr
  MOD_RES 14: note = METHYLATION
AVXVWNYXIIXXFYC

SEQ ID NO: 357 - protein, 15 aa, synthetic construct
  REGION 1..15: note = Synthesized polypeptide
  SITE 3: note = MISC_FEATURE - Xaa is MeF3C
  MOD_RES 5: note = METHYLATION
  SITE 8: note = MISC_FEATURE - Xaa is F4OMe
  SITE 11: note = MISC_FEATURE - Xaa is Aib
  SITE 12: note = MISC_FEATURE - Xaa is dr
  MOD_RES 14: note = METHYLATION
AVXVWNYXIIXXFYC

SEQ ID NO: 358 - protein, 15 aa, synthetic construct
  REGION 1..15: note = Synthesized polypeptide
  SITE 3: note = MISC_FEATURE - Xaa is MeF3C
  MOD_RES 5: note = METHYLATION
  SITE 8: note = MISC_FEATURE - Xaa is F4OMe
  SITE 11: note = MISC_FEATURE - Xaa is Aib
  SITE 12: note = MISC_FEATURE - Xaa is dr
  MOD_RES 14: note = METHYLATION
AVXVWNYXIIXXFYC

SEQ ID NO: 359 - protein, 15 aa, synthetic construct
  REGION 1..15: note = Synthesized polypeptide
  SITE 3: note = MISC_FEATURE - Xaa is MeF3C
  MOD_RES 5: note = METHYLATION
  SITE 8: note = MISC_FEATURE - Xaa is F4OMe
  SITE 11: note = MISC_FEATURE - Xaa is Abu
  SITE 12: note = MISC_FEATURE - Xaa is dr
  MOD_RES 14: note = METHYLATION
AVXVWNYXIIXXFYC

SEQ ID NO: 360 - protein, 15 aa, synthetic construct
  REGION 1..15: note = Synthesized polypeptide
  SITE 3: note = MISC_FEATURE - Xaa is MeF3C
  MOD_RES 5: note = METHYLATION
  SITE 8: note = MISC_FEATURE - Xaa is F4OMe
  SITE 11: note = MISC_FEATURE - Xaa is Nva
  SITE 12: note = MISC_FEATURE - Xaa is dr
  MOD_RES 14: note = METHYLATION
AVXVWNYXIIXXFYC

SEQ ID NO: 361 - protein, 15 aa, synthetic construct
  REGION 1..15: note = Synthesized polypeptide
  SITE 3: note = MISC_FEATURE - Xaa is MeF3C
  MOD_RES 5: note = METHYLATION
  SITE 8: note = MISC_FEATURE - Xaa is F4OMe
  SITE 11: note = MISC_FEATURE - Xaa is Nle
  SITE 12: note = MISC_FEATURE - Xaa is dr
  MOD_RES 14: note = METHYLATION
AVXVWNYXIIXXFYC

SEQ ID NO: 362 - protein, 15 aa, synthetic construct
  REGION 1..15: note = Synthesized polypeptide
  SITE 3: note = MISC_FEATURE - Xaa is MeF3C
  MOD_RES 5: note = METHYLATION
  SITE 8: note = MISC_FEATURE - Xaa is F4OMe
  SITE 11: note = MISC_FEATURE - Xaa is Ahp
  SITE 12: note = MISC_FEATURE - Xaa is dr
  MOD_RES 14: note = METHYLATION
AVXVWNYXIIXXFYC

SEQ ID NO: 363 - protein, 15 aa, synthetic construct
  REGION 1..15: note = Synthesized polypeptide
  SITE 3: note = MISC_FEATURE - Xaa is MeF3C
  MOD_RES 5: note = METHYLATION
  SITE 8: note = MISC_FEATURE - Xaa is F4OMe
  SITE 11: note = MISC_FEATURE - Xaa is E(PEG8Me)
  SITE 12: note = MISC_FEATURE - Xaa is dr
  MOD_RES 14: note = METHYLATION
AVXVWNYXIIXXFYC

SEQ ID NO: 364 - protein, 15 aa, synthetic construct
  REGION 1..15: note = Synthesized polypeptide
  SITE 3: note = MISC_FEATURE - Xaa is MeF3C
  MOD_RES 5: note = METHYLATION
  SITE 8: note = MISC_FEATURE - Xaa is F4OMe
  SITE 11: note = MISC_FEATURE - Xaa is A1Me4pip
  SITE 12: note = MISC_FEATURE - Xaa is dr
  MOD_RES 14: note = METHYLATION
AVXVWNYXIIXXFYC

SEQ ID NO: 365 - protein, 15 aa, synthetic construct
  REGION 1..15: note = Synthesized polypeptide
  SITE 3: note = MISC_FEATURE - Xaa is MeF3C
  MOD_RES 5: note = METHYLATION
  SITE 8: note = MISC_FEATURE - Xaa is F4OMe
  SITE 11: note = MISC_FEATURE - Xaa is Dap
  SITE 12: note = MISC_FEATURE - Xaa is dr
  MOD_RES 14: note = METHYLATION
AVXVWNYXIIXXFYC

SEQ ID NO: 366 - protein, 15 aa, synthetic construct
  REGION 1..15: note = Synthesized polypeptide
  SITE 3: note = MISC_FEATURE - Xaa is MeF3C
  MOD_RES 5: note = METHYLATION
  SITE 8: note = MISC_FEATURE - Xaa is F4OMe
  SITE 11: note = MISC_FEATURE - Xaa is Dab
  SITE 12: note = MISC_FEATURE - Xaa is dr
  MOD_RES 14: note = METHYLATION
AVXVWNYXIIXXFYC

SEQ ID NO: 367 - protein, 15 aa, synthetic construct
  REGION 1..15: note = Synthesized polypeptide
  SITE 3: note = MISC_FEATURE - Xaa is MeF3C
  MOD_RES 5: note = METHYLATION
  SITE 8: note = MISC_FEATURE - Xaa is F4OMe
  SITE 11: note = MISC_FEATURE - Xaa is Dap
  SITE 12: note = MISC_FEATURE - Xaa is dr
  MOD_RES 14: note = METHYLATION
AVXVWNYXIIXXFYC

SEQ ID NO: 368 - protein, 15 aa, synthetic construct
  REGION 1..15: note = Synthesized polypeptide
  SITE 3: note = MISC_FEATURE - Xaa is MeF3C
  MOD_RES 5: note = METHYLATION
  SITE 8: note = MISC_FEATURE - Xaa is F4OMe
  SITE 11: note = MISC_FEATURE - Xaa is dorn
  SITE 12: note = MISC_FEATURE - Xaa is dr
  MOD_RES 14: note = METHYLATION
AVXVWNYXIIXXFYC

SEQ ID NO: 369 - protein, 15 aa, synthetic construct
  REGION 1..15: note = Synthesized polypeptide
  SITE 3: note = MISC_FEATURE - Xaa is MeF3C
  MOD_RES 5: note = METHYLATION
  SITE 8: note = MISC_FEATURE - Xaa is F4OMe
  SITE 11: note = MISC_FEATURE - Xaa is Hly
  SITE 12: note = MISC_FEATURE - Xaa is dr
  MOD_RES 14: note = METHYLATION
AVXVWNYXIIXXFYC

SEQ ID NO: 370 - protein, 15 aa, synthetic construct
  REGION 1..15: note = Synthesized polypeptide
  SITE 3: note = MISC_FEATURE - Xaa is MeF3C
  MOD_RES 5: note = METHYLATION
  SITE 8: note = MISC_FEATURE - Xaa is F4OMe
  SITE 11: note = MISC_FEATURE - Xaa is Hly
  SITE 12: note = MISC_FEATURE - Xaa is dr
  MOD_RES 14: note = METHYLATION
AVXVWNYXIIXXFYC

SEQ ID NO: 371 - protein, 15 aa, synthetic construct
  REGION 1..15: note = Synthesized polypeptide
  SITE 3: note = MISC_FEATURE - Xaa is MeF3C
  MOD_RES 5: note = METHYLATION
  SITE 8: note = MISC_FEATURE - Xaa is F4OMe
  MOD_RES 14: note = METHYLATION
AVXVWNYXIIKRFYC

SEQ ID NO: 372 - protein, 15 aa, synthetic construct
  REGION 1..15: note = Synthesized polypeptide
  SITE 3: note = MISC_FEATURE - Xaa is MeF3C
  MOD_RES 5: note = METHYLATION
  SITE 8: note = MISC_FEATURE - Xaa is F4OMe
  SITE 12: note = MISC_FEATURE - Xaa is da
  MOD_RES 14: note = METHYLATION
AVXVWNYXIIKXFYC

SEQ ID NO: 373 - protein, 15 aa, synthetic construct
  REGION 1..15: note = Synthesized polypeptide
  SITE 3: note = MISC_FEATURE - Xaa is MeF3C
  MOD_RES 5: note = METHYLATION
  SITE 8: note = MISC_FEATURE - Xaa is F4OMe
  SITE 12: note = MISC_FEATURE - Xaa is dr
  MOD_RES 14: note = METHYLATION
AVXVWNYXIIKXFYC

SEQ ID NO: 374 - protein, 15 aa, synthetic construct
  REGION 1..15: note = Synthesized polypeptide
  SITE 3: note = MISC_FEATURE - Xaa is MeF3C
  MOD_RES 5: note = METHYLATION
  SITE 8: note = MISC_FEATURE - Xaa is F4OMe
  SITE 12: note = MISC_FEATURE - Xaa is dr
  MOD_RES 14: note = METHYLATION
AVXVWNYXIIKXFYC

SEQ ID NO: 375 - protein, 15 aa, synthetic construct
  REGION 1..15: note = Synthesized polypeptide
  SITE 3: note = MISC_FEATURE - Xaa is MeF3C
  MOD_RES 5: note = METHYLATION
  SITE 8: note = MISC_FEATURE - Xaa is F4OMe
  SITE 12: note = MISC_FEATURE - Xaa is dr
  MOD_RES 14: note = METHYLATION
AVXVWNYXIIKXFYC

SEQ ID NO: 376 - protein, 15 aa, synthetic construct
  REGION 1..15: note = Synthesized polypeptide
  SITE 3: note = MISC_FEATURE - Xaa is MeF3C
  MOD_RES 5: note = METHYLATION
  SITE 8: note = MISC_FEATURE - Xaa is F4OMe
  SITE 12: note = MISC_FEATURE - Xaa is dr
  MOD_RES 14: note = METHYLATION
AVXVWNYXIIKXFYC

SEQ ID NO: 377 - protein, 15 aa, synthetic construct
  REGION 1..15: note = Synthesized polypeptide
  SITE 3: note = MISC_FEATURE - Xaa is MeF3C
  MOD_RES 5: note = METHYLATION
  SITE 8: note = MISC_FEATURE - Xaa is F4OMe
  MOD_RES 11: note = METHYLATION
  SITE 12: note = MISC_FEATURE - Xaa is dr
  MOD_RES 14: note = METHYLATION
AVXVWNYXIIKXFYC

SEQ ID NO: 378 - protein, 15 aa, synthetic construct
  REGION 1..15: note = Synthesized polypeptide
  SITE 3: note = MISC_FEATURE - Xaa is MeF3C
  MOD_RES 5: note = METHYLATION
  SITE 8: note = MISC_FEATURE - Xaa is F4OMe
  MOD_RES 11: note = METHYLATION
  SITE 12: note = MISC_FEATURE - Xaa is da
  MOD_RES 14: note = METHYLATION
AVXVWNYXIIKXFYC

SEQ ID NO: 379 - protein, 15 aa, synthetic construct
  REGION 1..15: note = Synthesized polypeptide
  SITE 3: note = MISC_FEATURE - Xaa is MeF3C
  MOD_RES 5: note = METHYLATION
  SITE 8: note = MISC_FEATURE - Xaa is F4OMe
  SITE 11: note = MISC_FEATURE - Xaa is aMeK
  MOD_RES 14: note = METHYLATION
AVXVWNYXIIXRFYC

SEQ ID NO: 380 - protein, 15 aa, synthetic construct
  REGION 1..15: note = Synthesized polypeptide
  SITE 3: note = MISC_FEATURE - Xaa is MeF3C
  MOD_RES 5: note = METHYLATION
  SITE 8: note = MISC_FEATURE - Xaa is F4OMe
  SITE 11: note = MISC_FEATURE - Xaa is aMeK
  SITE 12: note = MISC_FEATURE - Xaa is dr
  MOD_RES 14: note = METHYLATION
AVXVWNYXIIXXFYC

SEQ ID NO: 381 - protein, 15 aa, synthetic construct
  REGION 1..15: note = Synthesized polypeptide
  SITE 3: note = MISC_FEATURE - Xaa is MeF3C
  MOD_RES 5: note = METHYLATION
  SITE 8: note = MISC_FEATURE - Xaa is F4OMe
  MOD_RES 11: note = METHYLATION
  MOD_RES 14: note = METHYLATION
AVXVWNYXIIRRFYC

SEQ ID NO: 382 - protein, 15 aa, synthetic construct
  REGION 1..15: note = Synthesized polypeptide
  SITE 3: note = MISC_FEATURE - Xaa is MeF3C
  MOD_RES 5: note = METHYLATION
  SITE 8: note = MISC_FEATURE - Xaa is F4OMe
  MOD_RES 11: note = METHYLATION
  SITE 12: note = MISC_FEATURE - Xaa is dr
  MOD_RES 14: note = METHYLATION
AVXVWNYXIIRXFYC

SEQ ID NO: 383 - protein, 15 aa, synthetic construct
  REGION 1..15: note = Synthesized polypeptide
  SITE 3: note = MISC_FEATURE - Xaa is MeF3C
  MOD_RES 5: note = METHYLATION
  SITE 8: note = MISC_FEATURE - Xaa is F4OMe
  MOD_RES 11: note = METHYLATION
  SITE 12: note = MISC_FEATURE - Xaa is da
  MOD_RES 14: note = METHYLATION
AVXVWNYXIIRXFYC

SEQ ID NO: 384 - protein, 15 aa, synthetic construct
  REGION 1..15: note = Synthesized polypeptide
  SITE 3: note = MISC_FEATURE - Xaa is MeF3C
  MOD_RES 5: note = METHYLATION
  SITE 8: note = MISC_FEATURE - Xaa is F4OMe
  SITE 12: note = MISC_FEATURE - Xaa is E(PEG8Me)
  MOD_RES 14: note = METHYLATION
AVXVWNYXIIRXFYC

SEQ ID NO: 385 - protein, 15 aa, synthetic construct
  REGION 1..15: note = Synthesized polypeptide
  SITE 3: note = MISC_FEATURE - Xaa is MeF3C
  MOD_RES 5: note = METHYLATION
  SITE 8: note = MISC_FEATURE - Xaa is F4OMe
  SITE 12: note = MISC_FEATURE - Xaa is E(de)
  MOD_RES 14: note = METHYLATION
AVXVWNYXIIRXFYC

SEQ ID NO: 386 - protein, 15 aa, synthetic construct
  REGION 1..15: note = Synthesized polypeptide
  SITE 3: note = MISC_FEATURE - Xaa is MeF3C
  MOD_RES 5: note = METHYLATION
  SITE 8: note = MISC_FEATURE - Xaa is F4OMe
  MOD_RES 14: note = METHYLATION
AVXVWNYXIIRRFYC

SEQ ID NO: 387 - protein, 15 aa, synthetic construct
  REGION 1..15: note = Synthesized polypeptide
  SITE 3: note = MISC_FEATURE - Xaa is MeF3C
  MOD_RES 5: note = METHYLATION
  SITE 8: note = MISC_FEATURE - Xaa is F4OMe
  MOD_RES 14: note = METHYLATION
AVXVWNYXIIRRFYC

SEQ ID NO: 388 - protein, 15 aa, synthetic construct
  REGION 1..15: note = Synthesized polypeptide
  SITE 3: note = MISC_FEATURE - Xaa is MeF3C
  MOD_RES 5: note = METHYLATION
  SITE 8: note = MISC_FEATURE - Xaa is F4OMe
  MOD_RES 14: note = METHYLATION
AVXVWNYXIIRRFYC

SEQ ID NO: 389 - protein, 15 aa, synthetic construct
  REGION 1..15: note = Synthesized polypeptide
  SITE 3: note = MISC_FEATURE - Xaa is MeF3C
  MOD_RES 5: note = METHYLATION
  SITE 8: note = MISC_FEATURE - Xaa is F4OMe
  SITE 12: note = MISC_FEATURE - Xaa is dr
  SITE 13: note = MISC_FEATURE - Xaa is E(PEG8Me)
  MOD_RES 14: note = METHYLATION
AVXVWNYXIIRXXYC

SEQ ID NO: 390 - protein, 15 aa, synthetic construct
  REGION 1..15: note = Synthesized polypeptide
  SITE 3: note = MISC_FEATURE - Xaa is MeF3C
  MOD_RES 5: note = METHYLATION
  SITE 8: note = MISC_FEATURE - Xaa is F4OMe
  SITE 12: note = MISC_FEATURE - Xaa is dr
  SITE 13: note = MISC_FEATURE - Xaa is E(e-Medk)
  MOD_RES 14: note = METHYLATION
AVXVWNYXIIRXXYC

SEQ ID NO: 391 - protein, 15 aa, synthetic construct
  REGION 1..15: note = Synthesized polypeptide
  SITE 3: note = MISC_FEATURE - Xaa is MeF3C
  MOD_RES 5: note = METHYLATION
  SITE 8: note = MISC_FEATURE - Xaa is F4OMe
  SITE 12: note = MISC_FEATURE - Xaa is dr
  SITE 13: note = MISC_FEATURE - Xaa is E(de)
  MOD_RES 14: note = METHYLATION
AVXVWNYXIIRXXYC

SEQ ID NO: 392 - protein, 15 aa, synthetic construct
  REGION 1..15: note = Synthesized polypeptide
  SITE 3: note = MISC_FEATURE - Xaa is MeF3C
  MOD_RES 5: note = METHYLATION
  SITE 8: note = MISC_FEATURE - Xaa is F4OMe
  SITE 12: note = MISC_FEATURE - Xaa is dr
  SITE 13: note = MISC_FEATURE - Xaa is F4C
  MOD_RES 14: note = METHYLATION
AVXVWNYXIIRXXYC

SEQ ID NO: 393 - protein, 15 aa, synthetic construct
  REGION 1..15: note = Synthesized polypeptide
  SITE 3: note = MISC_FEATURE - Xaa is MeF3C
  MOD_RES 5: note = METHYLATION
  SITE 8: note = MISC_FEATURE - Xaa is F4OMe
  SITE 12: note = MISC_FEATURE - Xaa is dr
  SITE 13: note = MISC_FEATURE - Xaa is F3C
  MOD_RES 14: note = METHYLATION
AVXVWNYXIIRXXYC

SEQ ID NO: 394 - protein, 15 aa, synthetic construct
  REGION 1..15: note = Synthesized polypeptide
  SITE 3: note = MISC_FEATURE - Xaa is MeF3C
  MOD_RES 5: note = METHYLATION
  SITE 8: note = MISC_FEATURE - Xaa is F4OMe
  SITE 12: note = MISC_FEATURE - Xaa is dr
  SITE 13: note = MISC_FEATURE - Xaa is F3OMe
  MOD_RES 14: note = METHYLATION
AVXVWNYXIIRXXYC

SEQ ID NO: 395 - protein, 15 aa, synthetic construct
  REGION 1..15: note = Synthesized polypeptide
  SITE 3: note = MISC_FEATURE - Xaa is MeF3C
  MOD_RES 5: note = METHYLATION
  SITE 8: note = MISC_FEATURE - Xaa is F4OMe
  SITE 12: note = MISC_FEATURE - Xaa is dr
  SITE 13: note = MISC_FEATURE - Xaa is F3H
  MOD_RES 14: note = METHYLATION
AVXVWNYXIIRXXYC

SEQ ID NO: 396 - protein, 15 aa, synthetic construct
  REGION 1..15: note = Synthesized polypeptide
  SITE 3: note = MISC_FEATURE - Xaa is MeF3C
  MOD_RES 5: note = METHYLATION
  SITE 8: note = MISC_FEATURE - Xaa is F4OMe
  SITE 12: note = MISC_FEATURE - Xaa is dr
  MOD_RES 14: note = METHYLATION
  SITE 15: note = MISC_FEATURE - Xaa is dc
AVXVWNYXIIRXFYX

SEQ ID NO: 397 - protein, 15 aa, synthetic construct
  REGION 1..15: note = Synthesized polypeptide
  SITE 3: note = MISC_FEATURE - Xaa is MeF3C
  MOD_RES 5: note = METHYLATION
  SITE 8: note = MISC_FEATURE - Xaa is F4OMe
  SITE 12: note = MISC_FEATURE - Xaa is dr
  MOD_RES 14: note = METHYLATION
AVXVWNYXIIRXFYC

SEQ ID NO: 398 - protein, 15 aa, synthetic construct
  REGION 1..15: note = Synthesized polypeptide
  SITE 3: note = MISC_FEATURE - Xaa is MeF3C
  MOD_RES 5: note = METHYLATION
  SITE 8: note = MISC_FEATURE - Xaa is F4OMe
  SITE 12: note = MISC_FEATURE - Xaa is dr
  MOD_RES 14: note = METHYLATION
AVXVWNYXIIRXFYC

SEQ ID NO: 399 - protein, 15 aa, synthetic construct
  REGION 1..15: note = Synthesized polypeptide
  SITE 3: note = MISC_FEATURE - Xaa is MeF3C
  MOD_RES 5: note = METHYLATION
  SITE 8: note = MISC_FEATURE - Xaa is F4OMe
  SITE 12: note = MISC_FEATURE - Xaa is dr
  MOD_RES 14: note = METHYLATION
AVXVWNYXIIRXFYC

SEQ ID NO: 400 - protein, 15 aa, synthetic construct
  REGION 1..15: note = Synthesized polypeptide
  SITE 3: note = MISC_FEATURE - Xaa is MeF3C
  MOD_RES 5: note = METHYLATION
  SITE 8: note = MISC_FEATURE - Xaa is F4OMe
  SITE 12: note = MISC_FEATURE - Xaa is dr
  MOD_RES 14: note = METHYLATION
AVXVWNYXIIRXFYC

SEQ ID NO: 401 - protein, 15 aa, synthetic construct
  REGION 1..15: note = Synthesized polypeptide
  SITE 3: note = MISC_FEATURE - Xaa is MeF3C
  MOD_RES 5: note = METHYLATION
  SITE 8: note = MISC_FEATURE - Xaa is F4OMe
  SITE 12: note = MISC_FEATURE - Xaa is dr
  MOD_RES 14: note = METHYLATION
AVXVWNYXIIRXFYC

SEQ ID NO: 402 - protein, 15 aa, synthetic construct
  REGION 1..15: note = Synthesized polypeptide
  SITE 3: note = MISC_FEATURE - Xaa is MeF3C
  MOD_RES 5: note = METHYLATION
  SITE 8: note = MISC_FEATURE - Xaa is F4OMe
  SITE 12: note = MISC_FEATURE - Xaa is dr
  MOD_RES 14: note = METHYLATION
AVXVWNYXIIRXFYC

SEQ ID NO: 403 - protein, 15 aa, synthetic construct
  REGION 1..15: note = Synthesized polypeptide
  SITE 3: note = MISC_FEATURE - Xaa is MeF3C
  MOD_RES 5: note = METHYLATION
  SITE 8: note = MISC_FEATURE - Xaa is F4OMe
  SITE 12: note = MISC_FEATURE - Xaa is dr
  MOD_RES 14: note = METHYLATION
AVXVWNYXIIRXFYC

SEQ ID NO: 404 - protein, 15 aa, synthetic construct
  REGION 1..15: note = Synthesized polypeptide
  SITE 3: note = MISC_FEATURE - Xaa is MeF3C
  MOD_RES 5: note = METHYLATION
  SITE 8: note = MISC_FEATURE - Xaa is F4OMe
  SITE 12: note = MISC_FEATURE - Xaa is dr
  MOD_RES 14: note = METHYLATION
AVXVWNYXIIRXFYC

SEQ ID NO: 405 - protein, 15 aa, synthetic construct
  REGION 1..15: note = Synthesized polypeptide
  SITE 3: note = MISC_FEATURE - Xaa is MeF3C
  MOD_RES 5: note = METHYLATION
  SITE 8: note = MISC_FEATURE - Xaa is F4OMe
  SITE 12: note = MISC_FEATURE - Xaa is dr
  MOD_RES 14: note = METHYLATION
AVXVWNYXIIRXFYC

SEQ ID NO: 406 - protein, 15 aa, synthetic construct
  REGION 1..15: note = Synthesized polypeptide
  SITE 3: note = MISC_FEATURE - Xaa is MeF3C
  MOD_RES 5: note = METHYLATION
  SITE 8: note = MISC_FEATURE - Xaa is F4OMe
  SITE 12: note = MISC_FEATURE - Xaa is dk
  MOD_RES 14: note = METHYLATION
AVXVWNYXIIRXFYC

SEQ ID NO: 407 - protein, 15 aa, synthetic construct
  REGION 1..15: note = Synthesized polypeptide
  SITE 3: note = MISC_FEATURE - Xaa is MeF3C
  MOD_RES 5: note = METHYLATION
  SITE 8: note = MISC_FEATURE - Xaa is F4OMe
  SITE 12: note = MISC_FEATURE - Xaa is dk
  MOD_RES 14: note = METHYLATION
AVXVWNYXIIRXFYC

SEQ ID NO: 408 - protein, 15 aa, synthetic construct
  REGION 1..15: note = Synthesized polypeptide
  MOD_RES 14: note = METHYLATION
  SITE 15: note = MISC_FEATURE - Xaa is Hgl
AVFVWNYYIIRRYYX

SEQ ID NO: 409 - protein, 15 aa, synthetic construct
  REGION 1..15: note = Synthesized polypeptide
  SITE 2: note = MISC_FEATURE - Xaa is Hgl
  SITE 3: note = MISC_FEATURE - Xaa is MeF3C
  MOD_RES 5: note = METHYLATION
  MOD_RES 14: note = METHYLATION
AXXVWNYYIIKRYYC

SEQ ID NO: 410 - protein, 15 aa, synthetic construct
  REGION 1..15: note = Synthesized polypeptide
  SITE 2: note = MISC_FEATURE - Xaa is Hgl
  SITE 3: note = MISC_FEATURE - Xaa is MeF3C
  MOD_RES 5: note = METHYLATION
  SITE 11: note = MISC_FEATURE - Xaa is Hly
  MOD_RES 14: note = METHYLATION
AXXVWNYYIIXRYYC

SEQ ID NO: 411 - protein, 15 aa, synthetic construct
  REGION 1..15: note = Synthesized polypeptide
  SITE 3: note = MISC_FEATURE - Xaa is MeF3C
  MOD_RES 5: note = METHYLATION
  SITE 11: note = MISC_FEATURE - Xaa is Hly
  MOD_RES 14: note = METHYLATION
AEXVWNYYIIXRYYC

SEQ ID NO: 412 - protein, 15 aa, synthetic construct
  REGION 1..15: note = Synthesized polypeptide
  SITE 3: note = MISC_FEATURE - Xaa is MeF3C
  MOD_RES 5: note = METHYLATION
  MOD_RES 14: note = METHYLATION
AEXVWNYYIIKRYYC

SEQ ID NO: 413 - protein, 15 aa, synthetic construct
  REGION 1..15: note = Synthesized polypeptide
  SITE 3: note = MISC_FEATURE - Xaa is Epyrl2RCOO
  MOD_RES 5: note = METHYLATION
  MOD_RES 14: note = METHYLATION
AVXVWNYKIIRRYYC

SEQ ID NO: 414 - protein, 15 aa, synthetic construct
  REGION 1..15: note = Synthesized polypeptide
  SITE 3: note = MISC_FEATURE - Xaa is Dpyrl2RCOO
  MOD_RES 5: note = METHYLATION
  MOD_RES 14: note = METHYLATION
AVXVWNYKIIRRYYC

SEQ ID NO: 415 - protein, 15 aa, synthetic construct
  REGION 1..15: note = Synthesized polypeptide
  MOD_RES 5: note = METHYLATION
  SITE 8: note = MISC_FEATURE - Xaa is Orn
  MOD_RES 14: note = METHYLATION
AVEVWNYXIIRRYYC

SEQ ID NO: 416 - protein, 15 aa, synthetic construct
  REGION 1..15: note = Synthesized polypeptide
  SITE 2: note = MISC_FEATURE - Xaa is Epyrl2RCOO
  SITE 3: note = MISC_FEATURE - Xaa is MeF3C
  MOD_RES 5: note = METHYLATION
  MOD_RES 14: note = METHYLATION
AXXVWNYYIIKRYYC

SEQ ID NO: 417 - protein, 15 aa, synthetic construct
  REGION 1..15: note = Synthesized polypeptide
  SITE 3: note = MISC_FEATURE - Xaa is MeF3C
  MOD_RES 5: note = METHYLATION
  SITE 11: note = MISC_FEATURE - Xaa is KaAc
  MOD_RES 14: note = METHYLATION
AEXVWNYYIIXRYYC

SEQ ID NO: 418 - protein, 15 aa, synthetic construct
  REGION 1..15: note = Synthesized polypeptide
  SITE 2: note = MISC_FEATURE - Xaa is Hgl
  SITE 3: note = MISC_FEATURE - Xaa is MeF3C
  MOD_RES 5: note = METHYLATION
  SITE 8: note = MISC_FEATURE - Xaa is F4OMe
  SITE 11: note = MISC_FEATURE - Xaa is Hly
  SITE 12: note = MISC_FEATURE - Xaa is dr
  MOD_RES 14: note = METHYLATION
AXXVWNYXIIXXFYC

SEQ ID NO: 419 - protein, 15 aa, synthetic construct
  REGION 1..15: note = Synthesized polypeptide
  SITE 2: note = MISC_FEATURE - Xaa is Hgl
  SITE 3: note = MISC_FEATURE - Xaa is MeF3C
  SITE 5: note = MISC_FEATURE - Xaa is W1aa
  SITE 11: note = MISC_FEATURE - Xaa is Hly
  SITE 12: note = MISC_FEATURE - Xaa is dr
  MOD_RES 14: note = METHYLATION
AXXVXNYYIIXXFYC

SEQ ID NO: 420 - protein, 15 aa, synthetic construct
  REGION 1..15: note = Synthesized polypeptide
  MOD_RES 3: note = METHYLATION
  MOD_RES 14: note = METHYLATION
AVFVWNYYIIRRYYC

SEQ ID NO: 421 - protein, 15 aa, synthetic construct
  REGION 1..15: note = Synthesized polypeptide
  MOD_RES 3: note = METHYLATION
  MOD_RES 14: note = METHYLATION
AVFVWNYYIIRRYYC

SEQ ID NO: 422 - protein, 15 aa, synthetic construct
  REGION 1..15: note = Synthesized polypeptide
  MOD_RES 3: note = METHYLATION
  MOD_RES 14: note = METHYLATION
AVFVWNYYIIRRYYC

SEQ ID NO: 423 - protein, 15 aa, synthetic construct
  REGION 1..15: note = Synthesized polypeptide
  MOD_RES 3: note = METHYLATION
  MOD_RES 14: note = METHYLATION
AVFVWNYYIIRRYYC

SEQ ID NO: 424 - protein, 15 aa, synthetic construct
  REGION 1..15: note = Synthesized polypeptide
  MOD_RES 3: note = METHYLATION
  MOD_RES 14: note = METHYLATION
AVFVWNYYIIRRYYC

SEQ ID NO: 425 - protein, 15 aa, synthetic construct
  REGION 1..15: note = Synthesized polypeptide
  MOD_RES 3: note = METHYLATION
  MOD_RES 14: note = METHYLATION
AVFVWNYYIIRRYYC

SEQ ID NO: 426 - protein, 15 aa, synthetic construct
  REGION 1..15: note = Synthesized polypeptide
  MOD_RES 3: note = METHYLATION
  MOD_RES 14: note = METHYLATION
AVFVWNYYIIRRYYC

SEQ ID NO: 427 - protein, 15 aa, synthetic construct
  REGION 1..15: note = Synthesized polypeptide
  MOD_RES 3: note = METHYLATION
  MOD_RES 14: note = METHYLATION
AVFVWNYYIIRRYYC

SEQ ID NO: 428 - protein, 15 aa, synthetic construct
  REGION 1..15: note = Synthesized polypeptide
  MOD_RES 3: note = METHYLATION
  MOD_RES 14: note = METHYLATION
AVFVWNYYIIRRYYC

SEQ ID NO: 429 - protein, 15 aa, synthetic construct
  REGION 1..15: note = Synthesized polypeptide
  MOD_RES 3: note = METHYLATION
  MOD_RES 14: note = METHYLATION
AVFVWNYYIIRRYYC

SEQ ID NO: 430 - protein, 15 aa, synthetic construct
  REGION 1..15: note = Synthesized polypeptide
  MOD_RES 3: note = METHYLATION
  MOD_RES 14: note = METHYLATION
AVFVWNYYIIRRYYC

SEQ ID NO: 431 - protein, 15 aa, synthetic construct
  REGION 1..15: note = Synthesized polypeptide
  MOD_RES 3: note = METHYLATION
  MOD_RES 14: note = METHYLATION
AVFVWNYYIIRRYYC

SEQ ID NO: 432 - protein, 15 aa, synthetic construct
  REGION 1..15: note = Synthesized polypeptide
  MOD_RES 3: note = METHYLATION
  MOD_RES 14: note = METHYLATION
AVFVWNYYIIRRYYC

SEQ ID NO: 433 - protein, 15 aa, synthetic construct
  REGION 1..15: note = Synthesized polypeptide
  MOD_RES 3: note = METHYLATION
  MOD_RES 14: note = METHYLATION
AVFVWNYYIIRRYYC

SEQ ID NO: 434 - protein, 15 aa, synthetic construct
  REGION 1..15: note = Synthesized polypeptide
  MOD_RES 3: note = METHYLATION
  MOD_RES 14: note = METHYLATION
AVFVWNYYIIRRYYC

SEQ ID NO: 435 - protein, 15 aa, synthetic construct
  REGION 1..15: note = Synthesized polypeptide
  MOD_RES 3: note = METHYLATION
  MOD_RES 14: note = METHYLATION
AVFVWNYYIIRRYYC

SEQ ID NO: 436 - protein, 15 aa, synthetic construct
  REGION 1..15: note = Synthesized polypeptide
  MOD_RES 3: note = METHYLATION
  MOD_RES 14: note = METHYLATION
AVFVWNYYIIRRYYC

SEQ ID NO: 437 - protein, 15 aa, synthetic construct
  REGION 1..15: note = Synthesized polypeptide
  MOD_RES 3: note = METHYLATION
  MOD_RES 14: note = METHYLATION
AVFVWNYYIIRRYYC

SEQ ID NO: 438 - protein, 15 aa, synthetic construct
  REGION 1..15: note = Synthesized polypeptide
  MOD_RES 3: note = METHYLATION
  MOD_RES 14: note = METHYLATION
AVFVWNYYIIRRYYC

SEQ ID NO: 439 - protein, 15 aa, synthetic construct
  REGION 1..15: note = Synthesized polypeptide
  MOD_RES 3: note = METHYLATION
  MOD_RES 14: note = METHYLATION
AVFVWNYYIIRRYYC

SEQ ID NO: 440 - protein, 15 aa, synthetic construct
  REGION 1..15: note = Synthesized polypeptide
  MOD_RES 3: note = METHYLATION
  MOD_RES 14: note = METHYLATION
AVFVWNYYIIRRYYC

SEQ ID NO: 441 - protein, 15 aa, synthetic construct
  REGION 1..15: note = Synthesized polypeptide
  MOD_RES 3: note = METHYLATION
  MOD_RES 14: note = METHYLATION
AVFVWNYYIIRRYYC

SEQ ID NO: 442 - protein, 15 aa, synthetic construct
  REGION 1..15: note = Synthesized polypeptide
  MOD_RES 3: note = METHYLATION
  MOD_RES 14: note = METHYLATION
AVFVWNYYIIRRYYC

SEQ ID NO: 443 - protein, 15 aa, synthetic construct
  REGION 1..15: note = Synthesized polypeptide
  MOD_RES 3: note = METHYLATION
  MOD_RES 14: note = METHYLATION
AVFVWNYYIIRRYYC

SEQ ID NO: 444 - protein, 15 aa, synthetic construct
  REGION 1..15: note = Synthesized polypeptide
  MOD_RES 3: note = METHYLATION
  MOD_RES 14: note = METHYLATION
AVFVWNYYIIRRYYC

SEQ ID NO: 445 - protein, 15 aa, synthetic construct
  REGION 1..15: note = Synthesized polypeptide
  MOD_RES 3: note = METHYLATION
  MOD_RES 14: note = METHYLATION
AVFVWNYYIIRRYYC

SEQ ID NO: 446 - protein, 15 aa, synthetic construct
  REGION 1..15: note = Synthesized polypeptide
  MOD_RES 3: note = METHYLATION
  MOD_RES 14: note = METHYLATION
AVFVWNYYIIRRYYC

SEQ ID NO: 447 - protein, 15 aa, synthetic construct
  REGION 1..15: note = Synthesized polypeptide
  SITE 3: note = MISC_FEATURE - Xaa is MeF3C
  MOD_RES 5: note = METHYLATION
  SITE 8: note = MISC_FEATURE - Xaa is F4OMe
  SITE 11: note = MISC_FEATURE - Xaa is Aib
  SITE 12: note = MISC_FEATURE - Xaa is dr
  MOD_RES 14: note = METHYLATION
AVXVWNYXIIXXFYC

SEQ ID NO: 448 - protein, 15 aa, synthetic construct
  REGION 1..15: note = Synthesized polypeptide
  SITE 3: note = MISC_FEATURE - Xaa is MeF3C
  MOD_RES 5: note = METHYLATION
  SITE 8: note = MISC_FEATURE - Xaa is F4OMe
  SITE 12: note = MISC_FEATURE - Xaa is dr
  MOD_RES 14: note = METHYLATION
AVXVWNYXIIRXFYC

SEQ ID NO: 449 - protein, 15 aa, synthetic construct
  REGION 1..15: note = Synthesized polypeptide
  MOD_RES 2: note = METHYLATION
  SITE 4: note = MISC_FEATURE - Xaa is dr
  SITE 5: note = MISC_FEATURE - Xaa is Aib
  SITE 8: note = MISC_FEATURE - Xaa is F4OMe
  MOD_RES 11: note = METHYLATION
  SITE 13: note = MISC_FEATURE - Xaa is MeF3C
AYFXXIYXYNWVXVC

SEQ ID NO: 450 - protein, 15 aa, synthetic construct
  REGION 1..15: note = Synthesized polypeptide
  SITE 3: note = MISC_FEATURE - Xaa is Me3Py
  MOD_RES 5: note = METHYLATION
  SITE 8: note = MISC_FEATURE - Xaa is F4OMe
  SITE 12: note = MISC_FEATURE - Xaa is dr
  MOD_RES 14: note = METHYLATION
AVXVWNYXIIRXFYC

SEQ ID NO: 451 - protein, 15 aa, synthetic construct
  REGION 1..15: note = Synthesized polypeptide
  SITE 3: note = MISC_FEATURE - Xaa is Me4Py
  MOD_RES 5: note = METHYLATION
  SITE 8: note = MISC_FEATURE - Xaa is F4OMe
  SITE 12: note = MISC_FEATURE - Xaa is dr
  MOD_RES 14: note = METHYLATION
AVXVWNYXIIRXFYC

SEQ ID NO: 452 - protein, 15 aa, synthetic construct
  REGION 1..15: note = Synthesized polypeptide
  SITE 3: note = MISC_FEATURE - Xaa is MeF3COO
  MOD_RES 5: note = METHYLATION
  SITE 8: note = MISC_FEATURE - Xaa is F4OMe
  SITE 12: note = MISC_FEATURE - Xaa is dr
  MOD_RES 14: note = METHYLATION
AVXVWNYXIIRXFYC

SEQ ID NO: 453 - protein, 15 aa, synthetic construct
  REGION 1..15: note = Synthesized polypeptide
  SITE 3: note = MISC_FEATURE - Xaa is MeF3C
  SITE 5: note = MISC_FEATURE - Xaa is W1mCON
  SITE 8: note = MISC_FEATURE - Xaa is F4OMe
  SITE 12: note = MISC_FEATURE - Xaa is dr
  MOD_RES 14: note = METHYLATION
AVXVXNYXIIRXFYC

SEQ ID NO: 454 - protein, 15 aa, synthetic construct
  REGION 1..15: note = Synthesized polypeptide
  SITE 3: note = MISC_FEATURE - Xaa is MeF3C
  MOD_RES 5: note = METHYLATION
  SITE 8: note = MISC_FEATURE - Xaa is 3Py
  SITE 12: note = MISC_FEATURE - Xaa is dr
  MOD_RES 14: note = METHYLATION
AVXVWNYXIIRXFYC

SEQ ID NO: 455 - protein, 15 aa, synthetic construct
  REGION 1..15: note = Synthesized polypeptide
  SITE 3: note = MISC_FEATURE - Xaa is MeF3C
  MOD_RES 5: note = METHYLATION
  SITE 8: note = MISC_FEATURE - Xaa is 4Py
  SITE 12: note = MISC_FEATURE - Xaa is dr
  MOD_RES 14: note = METHYLATION
AVXVWNYXIIRXFYC

SEQ ID NO: 456 - protein, 15 aa, synthetic construct
  REGION 1..15: note = Synthesized polypeptide
  SITE 3: note = MISC_FEATURE - Xaa is MeF3C
  MOD_RES 5: note = METHYLATION
  SITE 8: note = MISC_FEATURE - Xaa is 3Imp
  SITE 12: note = MISC_FEATURE - Xaa is dr
  MOD_RES 14: note = METHYLATION
AVXVWNYXIIRXFYC

SEQ ID NO: 457 - protein, 15 aa, synthetic construct
  REGION 1..15: note = Synthesized polypeptide
  SITE 3: note = MISC_FEATURE - Xaa is MeF3C
  MOD_RES 5: note = METHYLATION
  SITE 8: note = MISC_FEATURE - Xaa is F3CON
  SITE 12: note = MISC_FEATURE - Xaa is dr
  MOD_RES 14: note = METHYLATION
AVXVWNYXIIRXFYC

SEQ ID NO: 458 - protein, 15 aa, synthetic construct
  REGION 1..15: note = Synthesized polypeptide
  SITE 3: note = MISC_FEATURE - Xaa is MeF3C
  MOD_RES 5: note = METHYLATION
  SITE 8: note = MISC_FEATURE - Xaa is F3COO
  SITE 12: note = MISC_FEATURE - Xaa is dr
  MOD_RES 14: note = METHYLATION
AVXVWNYXIIRXFYC

SEQ ID NO: 459 - protein, 15 aa, synthetic construct
  REGION 1..15: note = Synthesized polypeptide
  SITE 3: note = MISC_FEATURE - Xaa is MeF3C
  MOD_RES 5: note = METHYLATION
  SITE 8: note = MISC_FEATURE - Xaa is F4OMe
  SITE 12: note = MISC_FEATURE - Xaa is dr
  SITE 13: note = MISC_FEATURE - Xaa is 4Py
  MOD_RES 14: note = METHYLATION
AVXVWNYXIIRXXYC

SEQ ID NO: 460 - protein, 15 aa, synthetic construct
  REGION 1..15: note = Synthesized polypeptide
  SITE 3: note = MISC_FEATURE - Xaa is MeF3C
  MOD_RES 5: note = METHYLATION
  SITE 8: note = MISC_FEATURE - Xaa is F4OMe
  SITE 12: note = MISC_FEATURE - Xaa is dr
  SITE 13: note = MISC_FEATURE - Xaa is 3Py
  MOD_RES 14: note = METHYLATION
AVXVWNYXIIRXXYC

SEQ ID NO: 461 - protein, 15 aa, synthetic construct
  REGION 1..15: note = Synthesized polypeptide
  SITE 3: note = MISC_FEATURE - Xaa is MeF3C
  MOD_RES 5: note = METHYLATION
  SITE 8: note = MISC_FEATURE - Xaa is F4OMe
  SITE 12: note = MISC_FEATURE - Xaa is dr
  SITE 13: note = MISC_FEATURE - Xaa is F3COO
  MOD_RES 14: note = METHYLATION
AVXVWNYXIIRXXYC

SEQ ID NO: 462 - protein, 15 aa, synthetic construct
  REGION 1..15: note = Synthesized polypeptide
  SITE 3: note = MISC_FEATURE - Xaa is MeF3C
  MOD_RES 5: note = METHYLATION
  SITE 8: note = MISC_FEATURE - Xaa is F4OMe
  SITE 12: note = MISC_FEATURE - Xaa is dr
  SITE 13: note = MISC_FEATURE - Xaa is F3CON
  MOD_RES 14: note = METHYLATION
AVXVWNYXIIRXXYC

SEQ ID NO: 463 - protein, 15 aa, synthetic construct
  REGION 1..15: note = Synthesized polypeptide
  SITE 3: note = MISC_FEATURE - Xaa is MeF3C
  SITE 5: note = MISC_FEATURE - Xaa is W4OMe
  SITE 8: note = MISC_FEATURE - Xaa is F4OMe
  SITE 12: note = MISC_FEATURE - Xaa is dr
  MOD_RES 14: note = METHYLATION
AVXVXNYXIIRXFYC

SEQ ID NO: 464 - protein, 15 aa, synthetic construct
  REGION 1..15: note = Synthesized polypeptide
  SITE 3: note = MISC_FEATURE - Xaa is MeF3C
  SITE 5: note = MISC_FEATURE - Xaa is W5C
  SITE 8: note = MISC_FEATURE - Xaa is F4OMe
  SITE 12: note = MISC_FEATURE - Xaa is dr
  MOD_RES 14: note = METHYLATION
AVXVXNYXIIRXFYC

SEQ ID NO: 465 - protein, 15 aa, synthetic construct
  REGION 1..15: note = Synthesized polypeptide
  SITE 3: note = MISC_FEATURE - Xaa is MeF3C
  MOD_RES 5: note = METHYLATION
  SITE 8: note = MISC_FEATURE - Xaa is F4C
  SITE 12: note = MISC_FEATURE - Xaa is dr
  MOD_RES 14: note = METHYLATION
AVXVWNYXIIRXFYC

SEQ ID NO: 466 - protein, 15 aa, synthetic construct
  REGION 1..15: note = Synthesized polypeptide
  SITE 3: note = MISC_FEATURE - Xaa is MeF3C
  MOD_RES 5: note = METHYLATION
  SITE 8: note = MISC_FEATURE - Xaa is F3C
  SITE 12: note = MISC_FEATURE - Xaa is dr
  MOD_RES 14: note = METHYLATION
AVXVWNYXIIRXFYC

SEQ ID NO: 467 - protein, 15 aa, synthetic construct
  REGION 1..15: note = Synthesized polypeptide
  SITE 3: note = MISC_FEATURE - Xaa is MeF3C
  MOD_RES 5: note = METHYLATION
  SITE 8: note = MISC_FEATURE - Xaa is F4F
  SITE 12: note = MISC_FEATURE - Xaa is dr
  MOD_RES 14: note = METHYLATION
AVXVWNYXIIRXFYC

SEQ ID NO: 468 - protein, 15 aa, synthetic construct
  REGION 1..15: note = Synthesized polypeptide
  SITE 3: note = MISC_FEATURE - Xaa is MeF3C
  MOD_RES 5: note = METHYLATION
  SITE 8: note = MISC_FEATURE - Xaa is F4F
  SITE 12: note = MISC_FEATURE - Xaa is dr
  MOD_RES 14: note = METHYLATION
AVXVWNYXIIRXFYC

SEQ ID NO: 469 - protein, 15 aa, synthetic construct
  REGION 1..15: note = Synthesized polypeptide
  MOD_RES 3: note = METHYLATION
  SITE 5: note = MISC_FEATURE - Xaa is W1aa
  SITE 11: note = MISC_FEATURE - Xaa is Aib
  MOD_RES 14: note = METHYLATION
AVFVXNYYIIXRYYC

SEQ ID NO: 470 - protein, 15 aa, synthetic construct
  REGION 1..15: note = Synthesized polypeptide
  SITE 3: note = MISC_FEATURE - Xaa is MeF3C
  SITE 5: note = MISC_FEATURE - Xaa is W1aa
  SITE 8: note = MISC_FEATURE - Xaa is F4OMe
  MOD_RES 14: note = METHYLATION
AVXVXNYXIEKRFYC

SEQ ID NO: 471 - protein, 15 aa, synthetic construct
  REGION 1..15: note = Synthesized polypeptide
  SITE 3: note = MISC_FEATURE - Xaa is MeF3C
  SITE 5: note = MISC_FEATURE - Xaa is W1aa
  SITE 8: note = MISC_FEATURE - Xaa is F4OMe
  MOD_RES 14: note = METHYLATION
AVXVXNYXIERRFYC

SEQ ID NO: 472 - protein, 15 aa, synthetic construct
  REGION 1..15: note = Synthesized polypeptide
  SITE 3: note = MISC_FEATURE - Xaa is MeF3C
  SITE 5: note = MISC_FEATURE - Xaa is W1aa
  SITE 8: note = MISC_FEATURE - Xaa is F4OMe
  SITE 12: note = MISC_FEATURE - Xaa is dr
  MOD_RES 14: note = METHYLATION
AVXVXNYXIERXFYC

SEQ ID NO: 473 - protein, 15 aa, synthetic construct
  REGION 1..15: note = Synthesized polypeptide
  MOD_RES 3: note = METHYLATION
  SITE 5: note = MISC_FEATURE - Xaa is W1aa
  SITE 12: note = MISC_FEATURE - Xaa is dr
  MOD_RES 14: note = METHYLATION
AVFVXNYYIERXYYC

SEQ ID NO: 474 - protein, 15 aa, synthetic construct
  REGION 1..15: note = Synthesized polypeptide
  MOD_RES 3: note = METHYLATION
  SITE 5: note = MISC_FEATURE - Xaa is W5C
  MOD_RES 14: note = METHYLATION
AVFVXNYYIIRRFYC

SEQ ID NO: 475 - protein, 15 aa, synthetic construct
  REGION 1..15: note = Synthesized polypeptide
  MOD_RES 3: note = METHYLATION
  SITE 5: note = MISC_FEATURE - Xaa is W5C
  SITE 8: note = MISC_FEATURE - Xaa is F4OMe
  MOD_RES 14: note = METHYLATION
AVFVXNYXIIRRFYC

SEQ ID NO: 476 - protein, 15 aa, synthetic construct
  REGION 1..15: note = Synthesized polypeptide
  MOD_RES 3: note = METHYLATION
  SITE 5: note = MISC_FEATURE - Xaa is W5C
  SITE 12: note = MISC_FEATURE - Xaa is dr
  MOD_RES 14: note = METHYLATION
AVFVXNYYIIRXFYC

SEQ ID NO: 477 - protein, 15 aa, synthetic construct
  REGION 1..15: note = Synthesized polypeptide
  MOD_RES 3: note = METHYLATION
  SITE 5: note = MISC_FEATURE - Xaa is W5C
  SITE 8: note = MISC_FEATURE - Xaa is F4OMe
  SITE 12: note = MISC_FEATURE - Xaa is dr
  MOD_RES 14: note = METHYLATION
AVFVXNYXIIRXFYC

SEQ ID NO: 478 - protein, 15 aa, synthetic construct
  REGION 1..15: note = Synthesized polypeptide
  SITE 3: note = MISC_FEATURE - Xaa is MeF4F
  SITE 5: note = MISC_FEATURE - Xaa is W5C
  MOD_RES 14: note = METHYLATION
AVXVXNYYIIRRFYC

SEQ ID NO: 479 - protein, 15 aa, synthetic construct
  REGION 1..15: note = Synthesized polypeptide
  SITE 3: note = MISC_FEATURE - Xaa is MeF4F
  SITE 5: note = MISC_FEATURE - Xaa is W5C
  SITE 8: note = MISC_FEATURE - Xaa is F4OMe
  MOD_RES 14: note = METHYLATION
AVXVXNYXIIRRFYC

SEQ ID NO: 480 - protein, 15 aa, synthetic construct
  REGION 1..15: note = Synthesized polypeptide
  SITE 3: note = MISC_FEATURE - Xaa is MeF4F
  SITE 5: note = MISC_FEATURE - Xaa is W5C
  SITE 12: note = MISC_FEATURE - Xaa is dr
  MOD_RES 14: note = METHYLATION
AVXVXNYYIIRXFYC

SEQ ID NO: 481 - protein, 15 aa, synthetic construct
  REGION 1..15: note = Synthesized polypeptide
  SITE 3: note = MISC_FEATURE - Xaa is MeF4F
  SITE 5: note = MISC_FEATURE - Xaa is W5C
  MOD_RES 11: note = METHYLATION
  SITE 12: note = MISC_FEATURE - Xaa is dr
  MOD_RES 14: note = METHYLATION
AVXVXNYYIIRXFYC

SEQ ID NO: 482 - protein, 15 aa, synthetic construct
  REGION 1..15: note = Synthesized polypeptide
  SITE 3: note = MISC_FEATURE - Xaa is MeF4F
  SITE 5: note = MISC_FEATURE - Xaa is W5C
  SITE 8: note = MISC_FEATURE - Xaa is F4OMe
  SITE 12: note = MISC_FEATURE - Xaa is dr
  MOD_RES 14: note = METHYLATION
AVXVXNYXIIRXFYC

SEQ ID NO: 483 - protein, 15 aa, synthetic construct
  REGION 1..15: note = Synthesized polypeptide
  SITE 3: note = MISC_FEATURE - Xaa is MeF4F
  SITE 5: note = MISC_FEATURE - Xaa is W5C
  SITE 8: note = MISC_FEATURE - Xaa is F4OMe
  MOD_RES 11: note = METHYLATION
  SITE 12: note = MISC_FEATURE - Xaa is dr
  MOD_RES 14: note = METHYLATION
AVXVXNYXIIRXFYC

SEQ ID NO: 484 - protein, 15 aa, synthetic construct
  REGION 1..15: note = Synthesized polypeptide
  SITE 3: note = MISC_FEATURE - Xaa is MeF4F
  MOD_RES 5: note = METHYLATION
  SITE 12: note = MISC_FEATURE - Xaa is dr
  MOD_RES 14: note = METHYLATION
AVXVWNYYIIRXFYC

SEQ ID NO: 485 - protein, 15 aa, synthetic construct
  REGION 1..15: note = Synthesized polypeptide
  SITE 3: note = MISC_FEATURE - Xaa is MeF4F
  MOD_RES 5: note = METHYLATION
  SITE 8: note = MISC_FEATURE - Xaa is F4OMe
  SITE 12: note = MISC_FEATURE - Xaa is dr
  MOD_RES 14: note = METHYLATION
AVXVWNYXIIRXFYC

SEQ ID NO: 486 - protein, 15 aa, synthetic construct
  REGION 1..15: note = Synthesized polypeptide
  SITE 3: note = MISC_FEATURE - Xaa is MeF4F
  MOD_RES 5: note = METHYLATION
  SITE 8: note = MISC_FEATURE - Xaa is F4OMe
  MOD_RES 11: note = METHYLATION
  SITE 12: note = MISC_FEATURE - Xaa is dr
  MOD_RES 14: note = METHYLATION
AVXVWNYXIIRXFYC

SEQ ID NO: 487 - protein, 15 aa, synthetic construct
  REGION 1..15: note = Synthesized polypeptide
  MOD_RES 3: note = METHYLATION
  SITE 11: note = MISC_FEATURE - Xaa is K(MePEG4c)
  MOD_RES 14: note = METHYLATION
AVFVWNYYIIXRFYC

SEQ ID NO: 488 - protein, 15 aa, synthetic construct
  REGION 1..15: note = Synthesized polypeptide
  MOD_RES 3: note = METHYLATION
  SITE 12: note = MISC_FEATURE - Xaa is K(MePEG4c)
  MOD_RES 14: note = METHYLATION
AVFVWNYYIIRXFYC

SEQ ID NO: 489 - protein, 15 aa, synthetic construct
  REGION 1..15: note = Synthesized polypeptide
  SITE 3: note = MISC_FEATURE - Xaa is MeF4F
  SITE 5: note = MISC_FEATURE - Xaa is W5C
  MOD_RES 11: note = METHYLATION
  SITE 12: note = MISC_FEATURE - Xaa is K(MePEG4c)
  MOD_RES 14: note = METHYLATION
AVXVXNYYIIRXFYC

SEQ ID NO: 490 - protein, 15 aa, synthetic construct
  REGION 1..15: note = Synthesized polypeptide
  SITE 3: note = MISC_FEATURE - Xaa is MeF4F
  SITE 5: note = MISC_FEATURE - Xaa is W5C
  SITE 8: note = MISC_FEATURE - Xaa is F4OMe
  MOD_RES 11: note = METHYLATION
  SITE 12: note = MISC_FEATURE - Xaa is K(MePEG4c)
  MOD_RES 14: note = METHYLATION
AVXVXNYXIIRXFYC

SEQ ID NO: 491 - protein, 15 aa, synthetic construct
  REGION 1..15: note = Synthesized polypeptide
  SITE 3: note = MISC_FEATURE - Xaa is MeF4F
  MOD_RES 5: note = METHYLATION
  SITE 11: note = MISC_FEATURE - Xaa is K(MePEG4c)
  SITE 12: note = MISC_FEATURE - Xaa is dr
  MOD_RES 14: note = METHYLATION
AVXVWNYYIIXXFYC

SEQ ID NO: 492 - protein, 15 aa, synthetic construct
  REGION 1..15: note = Synthesized polypeptide
  SITE 3: note = MISC_FEATURE - Xaa is MeF4F
  MOD_RES 5: note = METHYLATION
  SITE 8: note = MISC_FEATURE - Xaa is F4OMe
  SITE 11: note = MISC_FEATURE - Xaa is K(MePEG4c)
  SITE 12: note = MISC_FEATURE - Xaa is dr
  MOD_RES 14: note = METHYLATION
AVXVWNYXIIXXFYC

SEQ ID NO: 493 - protein, 15 aa, synthetic construct
  REGION 1..15: note = Synthesized polypeptide
  SITE 3: note = MISC_FEATURE - Xaa is MeF4F
  MOD_RES 5: note = METHYLATION
  MOD_RES 11: note = METHYLATION
  SITE 12: note = MISC_FEATURE - Xaa is K(MePEG4c)
  MOD_RES 14: note = METHYLATION
AVXVWNYYIIRXFYC

SEQ ID NO: 494 - protein, 15 aa, synthetic construct
  REGION 1..15: note = Synthesized polypeptide
  SITE 3: note = MISC_FEATURE - Xaa is MeF4F
  MOD_RES 5: note = METHYLATION
  SITE 8: note = MISC_FEATURE - Xaa is F4OMe
  MOD_RES 11: note = METHYLATION
  SITE 12: note = MISC_FEATURE - Xaa is K(MePEG4c)
  MOD_RES 14: note = METHYLATION
AVXVWNYXIIRXFYC

SEQ ID NO: 495 - protein, 15 aa, synthetic construct
  REGION 1..15: note = Synthesized polypeptide
  MOD_RES 3: note = METHYLATION
  SITE 5: note = MISC_FEATURE - Xaa is W1aa
  MOD_RES 14: note = METHYLATION
AVFVXNYYIIRRYYC

SEQ ID NO: 496 - protein, 15 aa, synthetic construct
  REGION 1..15: note = Synthesized polypeptide
  MOD_RES 3: note = METHYLATION
  SITE 8: note = MISC_FEATURE - Xaa is F4aao
  MOD_RES 14: note = METHYLATION
AVFVWNYXIIRRYYC

SEQ ID NO: 497 - protein, 15 aa, synthetic construct
  REGION 1..15: note = Synthesized polypeptide
  MOD_RES 3: note = METHYLATION
  SITE 5: note = MISC_FEATURE - Xaa is W1aa
  SITE 8: note = MISC_FEATURE - Xaa is F4aao
  MOD_RES 14: note = METHYLATION
AVFVXNYXIIRRYYC

SEQ ID NO: 498 - protein, 15 aa, synthetic construct
  REGION 1..15: note = Synthesized polypeptide
  MOD_RES 3: note = METHYLATION
  MOD_RES 14: note = METHYLATION
AVFVWNYYIIRRYYC

SEQ ID NO: 499 - protein, 15 aa, synthetic construct
  REGION 1..15: note = Synthesized polypeptide
  MOD_RES 3: note = METHYLATION
  MOD_RES 14: note = METHYLATION
AVFVWNYYIIRRYYC

SEQ ID NO: 500 - protein, 15 aa, synthetic construct
  REGION 1..15: note = Synthesized polypeptide
  MOD_RES 3: note = METHYLATION
  MOD_RES 14: note = METHYLATION
AVFVWNYYIIRRYYC

SEQ ID NO: 501 - protein, 15 aa, synthetic construct
  REGION 1..15: note = Synthesized polypeptide
  MOD_RES 3: note = METHYLATION
  MOD_RES 14: note = METHYLATION
AVFVWNYYIIRRYYC

SEQ ID NO: 502 - protein, 15 aa, synthetic construct
  REGION 1..15: note = Synthesized polypeptide
  SITE 3: note = MISC_FEATURE - Xaa is MeF3C
  SITE 8: note = MISC_FEATURE - Xaa is F4OMe
  MOD_RES 14: note = METHYLATION
AVXVWNYXIIRRFYC

SEQ ID NO: 503 - protein, 15 aa, synthetic construct
  REGION 1..15: note = Synthesized polypeptide
  SITE 3: note = MISC_FEATURE - Xaa is MeF3C
  SITE 8: note = MISC_FEATURE - Xaa is F4OMe
  MOD_RES 14: note = METHYLATION
AVXVWNYXIIKRFYC

SEQ ID NO: 504 - protein, 15 aa, synthetic construct
  REGION 1..15: note = Synthesized polypeptide
  MOD_RES 3: note = METHYLATION
  MOD_RES 14: note = METHYLATION
AVFVWNYYIIRRYYC

SEQ ID NO: 505 - protein, 15 aa, synthetic construct
  REGION 1..15: note = Synthesized polypeptide
  MOD_RES 3: note = METHYLATION
  MOD_RES 14: note = METHYLATION
AVFVWNYYIIRRYYC

SEQ ID NO: 506 - protein, 15 aa, synthetic construct
  REGION 1..15: note = Synthesized polypeptide
  MOD_RES 3: note = METHYLATION
  MOD_RES 14: note = METHYLATION
AVFVWNYYIIRRYYC

SEQ ID NO: 507 - protein, 15 aa, synthetic construct
  REGION 1..15: note = Synthesized polypeptide
  MOD_RES 3: note = METHYLATION
  MOD_RES 14: note = METHYLATION
AVFVWNYYIIRRYYC

SEQ ID NO: 508 - protein, 15 aa, synthetic construct
  REGION 1..15: note = Synthesized polypeptide
  MOD_RES 3: note = METHYLATION
  MOD_RES 14: note = METHYLATION
AVFVWNYYIIRRYYC

SEQ ID NO: 509 - protein, 15 aa, synthetic construct
  REGION 1..15: note = Synthesized polypeptide
  MOD_RES 3: note = METHYLATION
  MOD_RES 14: note = METHYLATION
AVFVWNYYIIRRYYC

SEQ ID NO: 510 - protein, 15 aa, synthetic construct
  REGION 1..15: note = Synthesized polypeptide
  SITE 3: note = MISC_FEATURE - Xaa is MeF3C
  MOD_RES 5: note = METHYLATION
  SITE 8: note = MISC_FEATURE - Xaa is F4OMe
  SITE 12: note = MISC_FEATURE - Xaa is dr
  MOD_RES 14: note = METHYLATION
AVXVWNYXIIRXFYC

SEQ ID NO: 511 - protein, 15 aa, synthetic construct
  REGION 1..15: note = Synthesized polypeptide
  SITE 3: note = MISC_FEATURE - Xaa is MeF3C
  MOD_RES 5: note = METHYLATION
  SITE 8: note = MISC_FEATURE - Xaa is F4OMe
  SITE 12: note = MISC_FEATURE - Xaa is dr
  MOD_RES 14: note = METHYLATION
AVXVWNYXIIRXFYC

SEQ ID NO: 512 - protein, 15 aa, synthetic construct
  REGION 1..15: note = Synthesized polypeptide
  SITE 3: note = MISC_FEATURE - Xaa is MeF3C
  MOD_RES 5: note = METHYLATION
  SITE 8: note = MISC_FEATURE - Xaa is F4OMe
  SITE 12: note = MISC_FEATURE - Xaa is dr
  MOD_RES 14: note = METHYLATION
AVXVWNYXIIRXFYC

SEQ ID NO: 513 - protein, 15 aa, synthetic construct
  REGION 1..15: note = Synthesized polypeptide
  SITE 3: note = MISC_FEATURE - Xaa is MeF3C
  MOD_RES 5: note = METHYLATION
  SITE 8: note = MISC_FEATURE - Xaa is F4OMe
  SITE 12: note = MISC_FEATURE - Xaa is dr
  MOD_RES 14: note = METHYLATION
AVXVWNYXIIRXFYC

SEQ ID NO: 514 - protein, 15 aa, synthetic construct
  REGION 1..15: note = Synthesized polypeptide
  SITE 3: note = MISC_FEATURE - Xaa is MeF3C
  MOD_RES 5: note = METHYLATION
  SITE 8: note = MISC_FEATURE - Xaa is F4OMe
  SITE 12: note = MISC_FEATURE - Xaa is dr
  MOD_RES 14: note = METHYLATION
AVXVWNYXIIRXFYC

SEQ ID NO: 515 - protein, 15 aa, synthetic construct
  REGION 1..15: note = Synthesized polypeptide
  MOD_RES 3: note = METHYLATION
  SITE 5: note = MISC_FEATURE - Xaa is W1aa
  MOD_RES 14: note = METHYLATION
AVFVXNYYIIKRYYC

SEQ ID NO: 516 - protein, 15 aa, synthetic construct
  REGION 1..15: note = Synthesized polypeptide
  MOD_RES 3: note = METHYLATION
  SITE 5: note = MISC_FEATURE - Xaa is W1aa
  MOD_RES 14: note = METHYLATION
AVFVXNYYIIRRYYC

SEQ ID NO: 517 - protein, 15 aa, synthetic construct
  REGION 1..15: note = Synthesized polypeptide
  MOD_RES 3: note = METHYLATION
  SITE 5: note = MISC_FEATURE - Xaa is W1aa
  SITE 12: note = MISC_FEATURE - Xaa is dr
  MOD_RES 14: note = METHYLATION
AVFVXNYYIIRXYYC

SEQ ID NO: 518 - protein, 15 aa, synthetic construct
  REGION 1..15: note = Synthesized polypeptide
  SITE 3: note = MISC_FEATURE - Xaa is MeF3C
  SITE 5: note = MISC_FEATURE - Xaa is W1aa
  SITE 8: note = MISC_FEATURE - Xaa is F4OMe
  SITE 11: note = MISC_FEATURE - Xaa is Aib
  MOD_RES 14: note = METHYLATION
AVXVXNYXIEXRFYC

SEQ ID NO: 519 - protein, 15 aa, synthetic construct
  REGION 1..15: note = Synthesized polypeptide
  MOD_RES 3: note = METHYLATION
  SITE 5: note = MISC_FEATURE - Xaa is W1aa
  MOD_RES 14: note = METHYLATION
AVFVXNYYIEKRYYC

SEQ ID NO: 520 - protein, 15 aa, synthetic construct
  REGION 1..15: note = Synthesized polypeptide
  MOD_RES 3: note = METHYLATION
  SITE 5: note = MISC_FEATURE - Xaa is W1aa
  SITE 11: note = MISC_FEATURE - Xaa is Aib
  MOD_RES 14: note = METHYLATION
AVFVXNYYIEXRYYC

SEQ ID NO: 521 - protein, 15 aa, synthetic construct
  REGION 1..15: note = Synthesized polypeptide
  MOD_RES 3: note = METHYLATION
  SITE 8: note = MISC_FEATURE - Xaa is Yae
  MOD_RES 14: note = METHYLATION
AVFVWNYXIIKRFYC

SEQ ID NO: 522 - protein, 15 aa, synthetic construct
  REGION 1..15: note = Synthesized polypeptide
  MOD_RES 3: note = METHYLATION
  SITE 8: note = MISC_FEATURE - Xaa is Yae
  MOD_RES 14: note = METHYLATION
AVFVWNYXIIRRFYC

SEQ ID NO: 523 - protein, 15 aa, synthetic construct
  REGION 1..15: note = Synthesized polypeptide
  MOD_RES 3: note = METHYLATION
  SITE 8: note = MISC_FEATURE - Xaa is Yae
  SITE 12: note = MISC_FEATURE - Xaa is dr
  MOD_RES 14: note = METHYLATION
AVFVWNYXIIRXFYC

SEQ ID NO: 524 - protein, 15 aa, synthetic construct
  REGION 1..15: note = Synthesized polypeptide
  MOD_RES 3: note = METHYLATION
  SITE 8: note = MISC_FEATURE - Xaa is Yae
  SITE 11: note = MISC_FEATURE - Xaa is Aib
  MOD_RES 14: note = METHYLATION
AVFVWNYXIIXRFYC

SEQ ID NO: 525 - protein, 15 aa, synthetic construct
  REGION 1..15: note = Synthesized polypeptide
  MOD_RES 3: note = METHYLATION
  MOD_RES 14: note = METHYLATION
AVFVWNYYIIRRYYC

SEQ ID NO: 526 - protein, 15 aa, synthetic construct
  REGION 1..15: note = Synthesized polypeptide
  MOD_RES 3: note = METHYLATION
  MOD_RES 14: note = METHYLATION
AVFVWNYYIIKRYYC

SEQ ID NO: 527 - protein, 15 aa, synthetic construct
  REGION 1..15: note = Synthesized polypeptide
  SITE 3: note = MISC_FEATURE - Xaa is MeF3C
  MOD_RES 5: note = METHYLATION
  SITE 8: note = MISC_FEATURE - Xaa is F4OMe
  SITE 12: note = MISC_FEATURE - Xaa is dr
  MOD_RES 14: note = METHYLATION
AVXVWNYXIIRXFYC

SEQ ID NO: 528 - protein, 15 aa, synthetic construct
  REGION 1..15: note = Synthesized polypeptide
  SITE 3: note = MISC_FEATURE - Xaa is MeF3C
  MOD_RES 5: note = METHYLATION
  SITE 8: note = MISC_FEATURE - Xaa is F4OMe
  SITE 12: note = MISC_FEATURE - Xaa is dr
  MOD_RES 14: note = METHYLATION
AEXVWNYXIIRXFYC

SEQ ID NO: 529 - protein, 15 aa, synthetic construct
  REGION 1..15: note = Synthesized polypeptide
  SITE 3: note = MISC_FEATURE - Xaa is MeF3C
  MOD_RES 5: note = METHYLATION
  SITE 8: note = MISC_FEATURE - Xaa is F4OMe
  SITE 12: note = MISC_FEATURE - Xaa is dr
  MOD_RES 14: note = METHYLATION
AVXVWNYXIIEXFYC

SEQ ID NO: 530 - protein, 15 aa, synthetic construct
  REGION 1..15: note = Synthesized polypeptide
  SITE 3: note = MISC_FEATURE - Xaa is MeF3C
  MOD_RES 5: note = METHYLATION
  SITE 8: note = MISC_FEATURE - Xaa is F4OMe
  SITE 11: note = MISC_FEATURE - Xaa is Hgl
  SITE 12: note = MISC_FEATURE - Xaa is dr
  MOD_RES 14: note = METHYLATION
AVXVWNYXIIXXFYC

SEQ ID NO: 531 - protein, 15 aa, synthetic construct
  REGION 1..15: note = Synthesized polypeptide
  SITE 3: note = MISC_FEATURE - Xaa is MeF3C
  MOD_RES 5: note = METHYLATION
  SITE 8: note = MISC_FEATURE - Xaa is F4OMe
  SITE 12: note = MISC_FEATURE - Xaa is dr
  MOD_RES 14: note = METHYLATION
AVXVWNYXIIKXFYC

SEQ ID NO: 532 - protein, 15 aa, synthetic construct
  REGION 1..15: note = Synthesized polypeptide
  SITE 3: note = MISC_FEATURE - Xaa is MeF3C
  MOD_RES 5: note = METHYLATION
  SITE 8: note = MISC_FEATURE - Xaa is F4OMe
  SITE 11: note = MISC_FEATURE - Xaa is Hly
  SITE 12: note = MISC_FEATURE - Xaa is dr
  MOD_RES 14: note = METHYLATION
AVXVWNYXIIXXFYC

SEQ ID NO: 533 - protein, 15 aa, synthetic construct
  REGION 1..15: note = Synthesized polypeptide
  SITE 3: note = MISC_FEATURE - Xaa is MeF3C
  MOD_RES 5: note = METHYLATION
  SITE 8: note = MISC_FEATURE - Xaa is F4OMe
  SITE 12: note = MISC_FEATURE - Xaa is dk
  MOD_RES 14: note = METHYLATION
AVXVWNYXIIRXFYC

SEQ ID NO: 534 - protein, 15 aa, synthetic construct
  REGION 1..15: note = Synthesized polypeptide
  SITE 3: note = MISC_FEATURE - Xaa is MeF3C
  MOD_RES 5: note = METHYLATION
  SITE 8: note = MISC_FEATURE - Xaa is F4OMe
  SITE 11: note = MISC_FEATURE - Xaa is Hly
  SITE 12: note = MISC_FEATURE - Xaa is dk
  MOD_RES 14: note = METHYLATION
AVXVWNYXIIXXFYC

SEQ ID NO: 535 - protein, 12 aa, synthetic construct
  REGION 1..12: note = Synthesized polypeptide
AVFVWNYYIISC

SEQ ID NO: 536 - protein, 12 aa, synthetic construct
  REGION 1..12: note = Synthesized polypeptide
AVFVWNYYIISC

SEQ ID NO: 537 - protein, 15 aa, synthetic construct
  REGION 1..15: note = Synthesized polypeptide
  MOD_RES 3: note = METHYLATION
  MOD_RES 14: note = METHYLATION
AVFVWNYYIIRRYYC

SEQ ID NO: 538 - protein, 15 aa, synthetic construct
  REGION 1..15: note = Synthesized polypeptide
  MOD_RES 3: note = METHYLATION
  MOD_RES 14: note = METHYLATION
AVFVWNYYIIRRYYC

SEQ ID NO: 539 - protein, 15 aa, synthetic construct
  REGION 1..15: note = Synthesized polypeptide
  SITE 3: note = MISC_FEATURE - Xaa is MeF3C
  MOD_RES 5: note = METHYLATION
  SITE 8: note = MISC_FEATURE - Xaa is F4OMe
  SITE 12: note = MISC_FEATURE - Xaa is dr
  MOD_RES 14: note = METHYLATION
AVXVWNYXIIRXFYC

SEQ ID NO: 540 - protein, 15 aa, synthetic construct
  REGION 1..15: note = Synthesized polypeptide
  SITE 3: note = MISC_FEATURE - Xaa is MeF3C
  MOD_RES 5: note = METHYLATION
  SITE 8: note = MISC_FEATURE - Xaa is F4OMe
  SITE 12: note = MISC_FEATURE - Xaa is dr
  MOD_RES 14: note = METHYLATION
AVXVWNYXIIRXFYC

SEQ ID NO: 541 - protein, 15 aa, synthetic construct
  REGION 1..15: note = Synthesized polypeptide
  SITE 3: note = MISC_FEATURE - Xaa is MeF3C
  MOD_RES 5: note = METHYLATION
  SITE 8: note = MISC_FEATURE - Xaa is F4OMe
  SITE 12: note = MISC_FEATURE - Xaa is dr
  MOD_RES 14: note = METHYLATION
AVXVWNYXIIRXFYC

SEQ ID NO: 542 - protein, 15 aa, synthetic construct
  REGION 1..15: note = Synthesized polypeptide
  SITE 3: note = MISC_FEATURE - Xaa is MeF3C
  MOD_RES 5: note = METHYLATION
  SITE 8: note = MISC_FEATURE - Xaa is F4OMe
  SITE 12: note = MISC_FEATURE - Xaa is dr
  MOD_RES 14: note = METHYLATION
AVXVWNYXIIRXFYC

SEQ ID NO: 543 - protein, 15 aa, synthetic construct
  REGION 1..15: note = Synthesized polypeptide
  SITE 3: note = MISC_FEATURE - Xaa is MeF3C
  MOD_RES 5: note = METHYLATION
  SITE 8: note = MISC_FEATURE - Xaa is F4OMe
  SITE 11: note = MISC_FEATURE - Xaa is Aib
  SITE 12: note = MISC_FEATURE - Xaa is dr
  MOD_RES 14: note = METHYLATION
AVXVWNYXIIXXFYC

SEQ ID NO: 544 - protein, 15 aa, synthetic construct
  REGION 1..15: note = Synthesized polypeptide
  SITE 3: note = MISC_FEATURE - Xaa is MeF3C
  MOD_RES 5: note = METHYLATION
  SITE 8: note = MISC_FEATURE - Xaa is F4OMe
  SITE 11: note = MISC_FEATURE - Xaa is Aib
  SITE 12: note = MISC_FEATURE - Xaa is dr
  MOD_RES 14: note = METHYLATION
AVXVWNYXIIXXFYC

SEQ ID NO: 545 - protein, 15 aa, synthetic construct
  REGION 1..15: note = Synthesized polypeptide
  SITE 3: note = MISC_FEATURE - Xaa is MeF3C
  MOD_RES 5: note = METHYLATION
  SITE 8: note = MISC_FEATURE - Xaa is F4OMe
  SITE 11: note = MISC_FEATURE - Xaa is Aib
  SITE 12: note = MISC_FEATURE - Xaa is dr
  MOD_RES 14: note = METHYLATION
AVXVWNYXIIXXFYC

SEQ ID NO: 546 - protein, 15 aa, synthetic construct
  REGION 1..15: note = Synthesized polypeptide
  SITE 3: note = MISC_FEATURE - Xaa is MeF3C
  MOD_RES 5: note = METHYLATION
  SITE 8: note = MISC_FEATURE - Xaa is F4OMe
  SITE 11: note = MISC_FEATURE - Xaa is Aib
  SITE 12: note = MISC_FEATURE - Xaa is dr
  MOD_RES 14: note = METHYLATION
AVXVWNYXIIXXFYC

SEQ ID NO: 547 - protein, 15 aa, synthetic construct
  REGION 1..15: note = Synthesized polypeptide
  MOD_RES 3: note = METHYLATION
  MOD_RES 5: note = METHYLATION
  MOD_RES 14: note = METHYLATION
AVFVWNYYIIKRYYC

SEQ ID NO: 548 - protein, 15 aa, synthetic construct
  REGION 1..15: note = Synthesized polypeptide
  MOD_RES 14: note = METHYLATION
AVFVWNYYIIKRYYC

SEQ ID NO: 549 - protein, 15 aa, synthetic construct
  REGION 1..15: note = Synthesized polypeptide
AVFVWNYYIIDRFRC

SEQ ID NO: 550 - protein, 15 aa, synthetic construct
  REGION 1..15: note = Synthesized polypeptide
  MOD_RES 3: note = METHYLATION
  MOD_RES 5: note = METHYLATION
  SITE 8: note = MISC_FEATURE - Xaa is F4OMe
  SITE 10: note = MISC_FEATURE - Xaa is alI
  SITE 12: note = MISC_FEATURE - Xaa is dr
  MOD_RES 14: note = METHYLATION
AVFVWNYXIXRXFYC

SEQ ID NO: 551 - protein, 15 aa, synthetic construct
  REGION 1..15: note = Synthesized polypeptide
  SITE 3: note = MISC_FEATURE - Xaa is MeNal1
  SITE 5: note = MISC_FEATURE - Xaa is MeNal2
  SITE 7: note = MISC_FEATURE - Xaa is Nal1
  SITE 8: note = MISC_FEATURE - Xaa is Nal1
  MOD_RES 14: note = METHYLATION
AVXVXNXXIIKKYYC

SEQ ID NO: 552 - protein, 15 aa, synthetic construct
  REGION 1..15: note = Synthesized polypeptide
  MOD_RES 1: note = METHYLATION
  SITE 3: note = MISC_FEATURE - Xaa is MeF3C
  MOD_RES 5: note = METHYLATION
  SITE 8: note = MISC_FEATURE - Xaa is F4OMe
  SITE 12: note = MISC_FEATURE - Xaa is da
  MOD_RES 14: note = METHYLATION
AVXVWNYXIIRXFYC

SEQ ID NO: 553-558 - skipped (6 entries)

SEQ ID NO: 559 - protein, 5 aa, synthetic construct
  REGION 1..5: note = Synthesized polypeptide
  SITE 5: note = MISC_FEATURE - Xaa is K(Maleimide)
GGSSX

SEQ ID NO: 560 - protein, 6 aa, synthetic construct
  REGION 1..6: note = Synthesized polypeptide
  SITE 6: note = MISC_FEATURE - Xaa is K(Maleimide)
GGGSSX

SEQ ID NO: 561 - protein, 6 aa, synthetic construct
  REGION 1..6: note = Synthesized polypeptide
GGGGSS

SEQ ID NO: 562 - protein, 6 aa, synthetic construct
  REGION 1..6: note = Synthesized polypeptide
GGSGSG

SEQ ID NO: 563 - protein, 6 aa, synthetic construct
  REGION 1..6: note = Synthesized polypeptide
  SITE 1: note = MISC_FEATURE - Xaa is de
XGGGSS

SEQ ID NO: 564 - protein, 6 aa, synthetic construct
  REGION 1..6: note = Synthesized polypeptide
  SITE 2: note = MISC_FEATURE - Xaa is de
  SITE 4: note = MISC_FEATURE - Xaa is de
GXGXSS

SEQ ID NO: 565 - protein, 6 aa, synthetic construct
  REGION 1..6: note = Synthesized polypeptide
  SITE 2: note = MISC_FEATURE - Xaa is dk
  SITE 4: note = MISC_FEATURE - Xaa is dk
GXGXSS

SEQ ID NO: 566 - protein, 6 aa, synthetic construct
  REGION 1..6: note = Synthesized polypeptide
  SITE 2: note = MISC_FEATURE - Xaa is de
  SITE 4: note = MISC_FEATURE - Xaa is dk
GXGXSS

SEQ ID NO: 567 - protein, 6 aa, synthetic construct
  REGION 1..6: note = Synthesized polypeptide
GGGGSS

SEQ ID NO: 568 - protein, 7 aa, synthetic construct
  REGION 1..7: note = Synthesized polypeptide
  SITE 7: note = MISC_FEATURE - Xaa is K(Maleimide)
GGRGRSX

SEQ ID NO: 569 - protein, 7 aa, synthetic construct
  REGION 1..7: note = Synthesized polypeptide
  SITE 7: note = MISC_FEATURE - Xaa is K(Maleimide)
GGGGSSX

SEQ ID NO: 570 - protein, 7 aa, synthetic construct
  REGION 1..7: note = Synthesized polypeptide
  MOD_RES 2: note = METHYLATION
  MOD_RES 4: note = METHYLATION
  SITE 7: note = MISC_FEATURE - Xaa is K(Maleimide)
GGSGSSX

SEQ ID NO: 571 - protein, 7 aa, synthetic construct
  REGION 1..7: note = Synthesized polypeptide
  SITE 7: note = MISC_FEATURE - Xaa is KTrzMal
GGGGSSX

SEQ ID NO: 572 - protein, 7 aa, synthetic construct
  REGION 1..7: note = Synthesized polypeptide
  MOD_RES 2: note = METHYLATION
  MOD_RES 4: note = METHYLATION
  SITE 7: note = MISC_FEATURE - Xaa is K(Maleimide)
GGSGSSX

SEQ ID NO: 573 - protein, 7 aa, synthetic construct
  REGION 1..7: note = Synthesized polypeptide
  SITE 7: note = MISC_FEATURE - Xaa is K(Maleimide)
GGGGSSX

SEQ ID NO: 574 - protein, 7 aa, synthetic construct
  REGION 1..7: note = Synthesized polypeptide
  SITE 7: note = MISC_FEATURE - Xaa is K(Maleimide)
GGSGSSX

SEQ ID NO: 575 - protein, 7 aa, synthetic construct
  REGION 1..7: note = Synthesized polypeptide
  SITE 7: note = MISC_FEATURE - Xaa is K(Maleimide)
GGSGESX

SEQ ID NO: 576 - protein, 7 aa, synthetic construct
  REGION 1..7: note = Synthesized polypeptide
  SITE 7: note = MISC_FEATURE - Xaa is K(Maleimide)
GGESESX

SEQ ID NO: 577 - protein, 7 aa, synthetic construct
  REGION 1..7: note = Synthesized polypeptide
  SITE 7: note = MISC_FEATURE - Xaa is K(Maleimide)
GSSGSSX

SEQ ID NO: 578 - protein, 7 aa, synthetic construct
  REGION 1..7: note = Synthesized polypeptide
  SITE 7: note = MISC_FEATURE - Xaa is K(Maleimide)
GGRGRSX

SEQ ID NO: 579 - protein, 7 aa, synthetic construct
  REGION 1..7: note = Synthesized polypeptide
  SITE 7: note = MISC_FEATURE - Xaa is K(Maleimide)
GGRSESX

SEQ ID NO: 580 - protein, 7 aa, synthetic construct
  REGION 1..7: note = Synthesized polypeptide
  SITE 7: note = MISC_FEATURE - Xaa is K(Maleimide)
GGGGSSX

SEQ ID NO: 581 - protein, 7 aa, synthetic construct
  REGION 1..7: note = Synthesized polypeptide
  SITE 7: note = MISC_FEATURE - Xaa is C(AcNMe)
GGGGSSX

SEQ ID NO: 582 - skipped

SEQ ID NO: 583 - protein, 7 aa, synthetic construct
  REGION 1..7: note = Synthesized polypeptide
  SITE 2: note = MISC_FEATURE - Xaa is KCOpipzaa
  SITE 3: note = MISC_FEATURE - Xaa is KCOpipzaa
  SITE 7: note = MISC_FEATURE - Xaa is C(AcNMe)
GXXGSSX

SEQ ID NO: 584 - skipped

SEQ ID NO: 585 - protein, 7 aa, synthetic construct
  REGION 1..7: note = Synthesized polypeptide
  SITE 2: note = MISC_FEATURE - Xaa is de
  SITE 3: note = MISC_FEATURE - Xaa is de
  SITE 7: note = MISC_FEATURE - Xaa is C(AcNMe)
GXXGSSX

SEQ ID NO: 586 - protein, 7 aa, synthetic construct
  REGION 1..7: note = Synthesized polypeptide
  SITE 2: note = MISC_FEATURE - Xaa is KCOmeglumine
  SITE 7: note = MISC_FEATURE - Xaa is C(AcNMe)
GXGGSSX

SEQ ID NO: 587 - protein, 7 aa, synthetic construct
  REGION 1..7: note = Synthesized polypeptide
  SITE 2: note = MISC_FEATURE - Xaa is KCOpipzaa
  SITE 4: note = MISC_FEATURE - Xaa is de
  SITE 7: note = MISC_FEATURE - Xaa is C(AcNMe)
GXGXSSX

SEQ ID NO: 588 - protein, 7 aa, synthetic construct
  REGION 1..7: note = Synthesized polypeptide
  SITE 3: note = MISC_FEATURE - Xaa is KCOpipzaa
  SITE 4: note = MISC_FEATURE - Xaa is de
  SITE 7: note = MISC_FEATURE - Xaa is C(AcNMe)
GGXXSSX

SEQ ID NO: 589 - protein, 7 aa, synthetic construct
  REGION 1..7: note = Synthesized polypeptide
  SITE 2: note = MISC_FEATURE - Xaa is KCOpipzaa
  SITE 7: note = MISC_FEATURE - Xaa is C(AcNMe)
GXGGSSX

SEQ ID NO: 590 - protein, 7 aa, synthetic construct
  REGION 1..7: note = Synthesized polypeptide
  SITE 3: note = MISC_FEATURE - Xaa is KCOpipzaa
  SITE 7: note = MISC_FEATURE - Xaa is C(AcNMe)
GGXGSSX

SEQ ID NO: 591 - protein, 7 aa, synthetic construct
  REGION 1..7: note = Synthesized polypeptide
  SITE 4: note = MISC_FEATURE - Xaa is KCOpipzaa
  SITE 7: note = MISC_FEATURE - Xaa is C(AcNMe)
GGGXSSX

SEQ ID NO: 592 - protein, 7 aa, synthetic construct
  REGION 1..7: note = Synthesized polypeptide
  SITE 2: note = MISC_FEATURE - Xaa is KCOmeglumine
  SITE 4: note = MISC_FEATURE - Xaa is de
  SITE 7: note = MISC_FEATURE - Xaa is C(AcNMe)
GXGXSSX

SEQ ID NO: 593 - protein, 7 aa, synthetic construct
  REGION 1..7: note = Synthesized polypeptide
  SITE 3: note = MISC_FEATURE - Xaa is KCOmeglumine
  SITE 4: note = MISC_FEATURE - Xaa is de
  SITE 7: note = MISC_FEATURE - Xaa is C(AcNMe)
GGXXSSX

SEQ ID NO: 594 - protein, 7 aa, synthetic construct
  REGION 1..7: note = Synthesized polypeptide
  SITE 2: note = MISC_FEATURE - Xaa is de
  SITE 4: note = MISC_FEATURE - Xaa is KCOpipzaa
  SITE 7: note = MISC_FEATURE - Xaa is C(AcNMe)
GXGXSSX

SEQ ID NO: 595 - protein, 7 aa, synthetic construct
  REGION 1..7: note = Synthesized polypeptide
  SITE 3: note = MISC_FEATURE - Xaa is de
  SITE 4: note = MISC_FEATURE - Xaa is KCOpipzaa
  SITE 7: note = MISC_FEATURE - Xaa is C(AcNMe)
GGXXSSX

SEQ ID NO: 596 - protein, 7 aa, synthetic construct
  REGION 1..7: note = Synthesized polypeptide
  SITE 2: note = MISC_FEATURE - Xaa is de
  SITE 4: note = MISC_FEATURE - Xaa is KCOmeglumine
  SITE 7: note = MISC_FEATURE - Xaa is C(AcNMe)
GXGXSSX

SEQ ID NO: 597 - protein, 7 aa, synthetic construct
  REGION 1..7: note = Synthesized polypeptide
  SITE 3: note = MISC_FEATURE - Xaa is de
  SITE 4: note = MISC_FEATURE - Xaa is KCOmeglumine
  SITE 7: note = MISC_FEATURE - Xaa is C(AcNMe)
GGXXSSX

SEQ ID NO: 598 - protein, 7 aa, synthetic construct
  REGION 1..7: note = Synthesized polypeptide
  SITE 3: note = MISC_FEATURE - Xaa is KCOmeglumine
  SITE 7: note = MISC_FEATURE - Xaa is C(AcNMe)
GGXGSSX

SEQ ID NO: 599 - protein, 7 aa, synthetic construct
  REGION 1..7: note = Synthesized polypeptide
  SITE 4: note = MISC_FEATURE - Xaa is KCOmeglumine
  SITE 7: note = MISC_FEATURE - Xaa is C(AcNMe)
GGGXSSX

SEQ ID NO: 600-603 - skipped (4 entries)

SEQ ID NO: 604 - protein, 10 aa, synthetic construct
  REGION 1..10: note = Synthesized polypeptide
GGSGSSGGSG

SEQ ID NO: 605 - protein, 10 aa, synthetic construct
  REGION 1..10: note = Synthesized polypeptide
  SITE 10: note = MISC_FEATURE - Xaa is K(Maleimide)
GGSGSSGSSX

SEQ ID NO: 606 - protein, 12 aa, synthetic construct
  REGION 1..12: note = Synthesized polypeptide
GGRGRSGGRGRS

SEQ ID NO: 607 - protein, 12 aa, synthetic construct
  REGION 1..12: note = Synthesized polypeptide
GGQGQSGGQGQS

SEQ ID NO: 608-636 - skipped (29 entries)

SEQ ID NO: 637 - protein, 7 aa, synthetic construct
  REGION 1..7: note = Synthesized polypeptide
  SITE 7: note = MISC_FEATURE - Xaa is gAbu
GGRGRSX

SEQ ID NO: 638 - skipped

SEQ ID NO: 639 - protein, 7 aa, synthetic construct
  REGION 1..7: note = Synthesized polypeptide
  SITE 7: note = MISC_FEATURE - Xaa is gAbu
GGQGQSX

SEQ ID NO: 640 - protein, 13 aa, synthetic construct
  REGION 1..13: note = Synthesized polypeptide
  SITE 13: note = MISC_FEATURE - Xaa is gAbu
GGGGSSGGGGSSX

SEQ ID NO: 641 - protein, 8 aa, synthetic construct
  REGION 1..8: note = Synthesized polypeptide
  SITE 7: note = MISC_FEATURE - Xaa is dk(CHO4PhCO)
  SITE 8: note = MISC_FEATURE - Xaa is NH2
GGGGSSXX

SEQ ID NO: 642 - skipped

SEQ ID NO: 643 - protein, 4 aa, synthetic construct
  REGION 1..4: note = Synthesized polypeptide
GGGG

SEQ ID NO: 644 - protein, 7 aa, synthetic construct
  REGION 1..7: note = Synthesized polypeptide
GGGGSSC

SEQ ID NO: 645 - protein, 15 aa, synthetic construct
  REGION 1..15: note = Synthesized polypeptide
  SITE 3: note = MISC_FEATURE - Xaa is MeF3C
  SITE 5: note = MISC_FEATURE - Xaa is W1aa
  SITE 8: note = MISC_FEATURE - Xaa is F4OMe
  MOD_RES 14: note = METHYLATION
AVXVXNYXIERRFYC

SEQ ID NO: 646 - DNA, 212 bp, Homo sapiens
  source 1..212: mol_type = genomic DNA
ttgaaagaattcagaatcagtgggatgaagtacaagaacaccttcagaaccggaggcaacagttgaatgaaatgttaaaggattcaacacaatggctggaagctaaggaagaagctgagcaggtcttaggacaggccagagccaagcttgagtcatggaaggagggtccctatacagtagatgcaatccaaaagaaaatcacagaaaccaag

SEQ ID NO: 647 - DNA, 35 bp, synthetic construct
  misc_feature 1..35: note = Synthesized DNA
  source 1..35: mol_type = other DNA
tacaagaacaccttcagaaccggaggcaacagttg

SEQ ID NO: 648 - DNA, 25 bp, synthetic construct
  misc_feature 1..25: note = Synthesized DNA
  source 1..25: mol_type = other DNA
gaacaccttcagaaccggaggcaac

SEQ ID NO: 649 - DNA, 21 bp, synthetic construct
  misc_feature 1..21: note = Synthesized DNA
  source 1..21: mol_type = other DNA
gaacaccttcagaaccggagg

SEQ ID NO: 650 - DNA, 119 bp, Homo sapiens
  source 1..119: mol_type = genomic DNA
gcgatttgacagatctgttgagaaatggcggcgttttcattatgatataaagatatttaatcagtggctaacagaagctgaacagtttctcagaaagacacaaattcctgagaattggg

SEQ ID NO: 651 - DNA, 45 bp, synthetic construct
  misc_feature 1..45: note = Synthesized DNA
  source 1..45: mol_type = other DNA
ggcgatttgacagatctgttgagaaatggcggcgttttcattatg

SEQ ID NO: 652 - DNA, 58 bp, synthetic construct
  misc_feature 1..58: note = Synthesized DNA
  source 1..58: mol_type = other DNA
taatcagtggctaacagaagctgaacagtttctcagaaagacacaaattcctgagaat

SEQ ID NO: 653 - DNA, 14 bp, synthetic construct
  misc_feature 1..14: note = Synthesized DNA
  source 1..14: mol_type = other DNA
tgagaaatggcggc

SEQ ID NO: 654 - DNA, 12 bp, synthetic construct
  misc_feature 1..12: note = Synthesized DNA
  source 1..12: mol_type = other DNA
aaatggcggcgt

SEQ ID NO: 655 - DNA, 12 bp, synthetic construct
  misc_feature 1..12: note = Synthesized DNA
  source 1..12: mol_type = other DNA
gaaatggcggcg

SEQ ID NO: 656 - DNA, 13 bp, synthetic construct
  misc_feature 1..13: note = Synthesized DNA
  source 1..13: mol_type = other DNA
ctcagaaagacac

SEQ ID NO: 657 - DNA, 12 bp, synthetic construct
  misc_feature 1..12: note = Synthesized DNA
  source 1..12: mol_type = other DNA
gtggctaacaga

SEQ ID NO: 658 - DNA, 12 bp, synthetic construct
  misc_feature 1..12: note = Synthesized DNA
  source 1..12: mol_type = other DNA
agtggctaacag

SEQ ID NO: 659 - DNA, 14 bp, synthetic construct
  misc_feature 1..14: note = Synthesized DNA
  source 1..14: mol_type = other DNA
gtggctaacagaag

SEQ ID NO: 660 - DNA, 12 bp, synthetic construct
  misc_feature 1..12: note = Synthesized DNA
  source 1..12: mol_type = other DNA
agaaagacacaa

SEQ ID NO: 661 - DNA, 26 bp, synthetic construct
  misc_feature 1..26: note = Synthesized DNA
  source 1..26: mol_type = other DNA
acagatctgttgagaaatggcggcgt

SEQ ID NO: 662 - DNA, 26 bp, synthetic construct
  misc_feature 1..26: note = Synthesized DNA
  source 1..26: mol_type = other DNA
aatggcggcgttttcattatgatata

SEQ ID NO: 663 - DNA, 176 bp, Homo sapiens
  source 1..176: mol_type = genomic DNA
gaactccaggatggcattgggcagcggcaaactgttgtcagaacattgaatgcaactggggaagaaataattcagcaatcctcaaaaacagatgccagtattctacaggaaaaattgggaagcctgaatctgcggtggcaggaggtctgcaaacagctgtcagacagaaaaaagag

SEQ ID NO: 664 - DNA, 34 bp, synthetic construct
  misc_feature 1..34: note = Synthesized DNA
  source 1..34: mol_type = other DNA
caagtccaggatggcattgggcagcggcaaactg

SEQ ID NO: 665 - DNA, 30 bp, synthetic construct
  misc_feature 1..30: note = Synthesized DNA
  source 1..30: mol_type = other DNA
tccaggatggcattgggcagcggcaaactg

SEQ ID NO: 666 - DNA, 30 bp, synthetic construct
  misc_feature 1..30: note = Synthesized DNA
  source 1..30: mol_type = other DNA
caagtccaggatggcattgggcagcggcaa

SEQ ID NO: 667 - DNA, 26 bp, synthetic construct
  misc_feature 1..26: note = Synthesized DNA
  source 1..26: mol_type = other DNA
ggatggcattgggcagcggcaaactg

SEQ ID NO: 668 - DNA, 15 bp, synthetic construct
  misc_feature 1..15: note = Synthesized DNA
  source 1..15: mol_type = other DNA
gcattgggcagcggc

SEQ ID NO: 669 - DNA, 18 bp, synthetic construct
  misc_feature 1..18: note = Synthesized DNA
  source 1..18: mol_type = other DNA
ggatggcattgggcagcg

SEQ ID NO: 670 - DNA, 18 bp, synthetic construct
  misc_feature 1..18: note = Synthesized DNA
  source 1..18: mol_type = other DNA
ttgggcagcggcaaactg

SEQ ID NO: 671 - DNA, 26 bp, synthetic construct
  misc_feature 1..26: note = Synthesized DNA
  source 1..26: mol_type = other DNA
ttacaggaactccaggatggcattgg

SEQ ID NO: 672 - DNA, 22 bp, synthetic construct
  misc_feature 1..22: note = Synthesized DNA
  source 1..22: mol_type = other DNA
caggaactccaggatggcattg

SEQ ID NO: 673 - DNA, 35 bp, synthetic construct
  misc_feature 1..35: note = Synthesized DNA
  source 1..35: mol_type = other DNA
caggaactccaggatggcattgggcagcggcaaac

SEQ ID NO: 674 - DNA, 148 bp, Homo sapiens
  source 1..148: mol_type = genomic DNA
gctagaagaacaaaagaatatcttgtcagaatttcaaagagatttaaatgaatttgttttatggttggaggaagcagataacattgctagtatcccacttgaacctggaaaagagcagcaactaaaagaaaagcttgagcaagtcaag

SEQ ID NO: 675 - DNA, 43 bp, synthetic construct
  misc_feature 1..43: note = Synthesized DNA
  source 1..43: mol_type = other DNA
tatcccacttgaacctggaaaagagcagcaactaaaagaaaag

SEQ ID NO: 676 - DNA, 30 bp, synthetic construct
  misc_feature 1..30: note = Synthesized DNA
  source 1..30: mol_type = other DNA
tatcccacttgaacctggaaaagagcagca

SEQ ID NO: 677 - DNA, 30 bp, synthetic construct
  misc_feature 1..30: note = Synthesized DNA
  source 1..30: mol_type = other DNA
ttgaacctggaaaagagcagcaactaaaag

SEQ ID NO: 678 - DNA, 30 bp, synthetic construct
  misc_feature 1..30: note = Synthesized DNA
  source 1..30: mol_type = other DNA
cctggaaaagagcagcaactaaaagaaaag

SEQ ID NO: 679 - DNA, 30 bp, synthetic construct
  misc_feature 1..30: note = Synthesized DNA
  source 1..30: mol_type = other DNA
cacttgaacctggaaaagagcagcaactaa

SEQ ID NO: 680 - DNA, 129 bp, Homo sapiens
  source 1..129: mol_type = genomic DNA
aggaagttagaagatctgagctctgagtggaaggcggtaaaccgtttacttcaagagctgagggcaaagcagcctgacctagctcctggactgaccactattggagcctgtaagtatactggatcccat

SEQ ID NO: 681 - DNA, 25 bp, synthetic construct
  misc_feature 1..25: note = Synthesized DNA
  source 1..25: mol_type = other DNA
agcctgtaagtatactggatcccat

SEQ ID NO: 682 - DNA, 233 bp, Homo sapiens
  source 1..233: mol_type = genomic DNA
ctcctactcagactgttactctggtgacacaacctgtggttactaaggaaactgccatctccaaactagaaatgccatcttccttgatgttggaggtacctgctctggcagatttcaaccgggcttggacagaacttaccgactggctttctctgcttgatcaagttataaaatcacagagggtgatggtgggtgaccttgaggatatcaacgagatgatcatcaagcagaag

SEQ ID NO: 683 - DNA, 30 bp, synthetic construct
  misc_feature 1..30: note = Synthesized DNA
  source 1..30: mol_type = other DNA
ctagaaatgccatcttccttgatgttggag

SEQ ID NO: 684 - DNA, 20 bp, synthetic construct
  misc_feature 1..20: note = Synthesized DNA
  source 1..20: mol_type = other DNA
agaaatgccatcttccttga

SEQ ID NO: 685 - DNA, 190 bp, Homo sapiens
  source 1..190: mol_type = genomic DNA
ggtgagtgagcgagaggctgctttggaagaaactcatagattactgcaacagttccccctggacctggaaaagtttcttgcctggcttacagaagctgaaacaactgccaatgtcctacaggatgctacccgtaaggaaaggctcctagaagactccaagggagtaaaagagctgatgaaacaatggcaa

SEQ ID NO: 686 - DNA, 38 bp, synthetic construct
  misc_feature 1..38: note = Synthesized DNA
  source 1..38: mol_type = other DNA
agggtgagtgagcgagaggctgctttggaagaaactca

SEQ ID NO: 687 - DNA, 25 bp, synthetic construct
  misc_feature 1..25: note = Synthesized DNA
  source 1..25: mol_type = other DNA
gttgcctccggttctgaaggtgttc

SEQ ID NO: 688 - DNA, 21 bp, synthetic construct
  misc_feature 1..21: note = Synthesized DNA
  source 1..21: mol_type = other DNA
cctccggttctgaaggtgttc

SEQ ID NO: 689 - DNA, 26 bp, synthetic construct
  misc_feature 1..26: note = Synthesized DNA
  source 1..26: mol_type = other DNA
gtgtctttctgagccgccatttctca

SEQ ID NO: 690 - DNA, 22 bp, synthetic construct
  misc_feature 1..22: note = Synthesized DNA
  source 1..22: mol_type = other DNA
tctgttagccacgccgccattt

SEQ ID NO: 691 - DNA, 24 bp, synthetic construct
  misc_feature 1..24: note = Synthesized DNA
  source 1..24: mol_type = other DNA
ctgttagccactcgccgccatttc

SEQ ID NO: 692 - DNA, 24 bp, synthetic construct
  misc_feature 1..24: note = Synthesized DNA
  source 1..24: mol_type = other DNA
ttgtgtctttcttctgttagccac

SEQ ID NO: 693 - DNA, 30 bp, synthetic construct
  misc_feature 1..30: note = Synthesized DNA
  source 1..30: mol_type = other DNA
cagtttgccgctgcccaatgccatcctgga

SEQ ID NO: 694 - DNA, 30 bp, synthetic construct
  misc_feature 1..30: note = Synthesized DNA
  source 1..30: mol_type = other DNA
ttgccgctgcccaatgccatcctggagttc

SEQ ID NO: 695 - DNA, 15 bp, synthetic construct
  misc_feature 1..15: note = Synthesized DNA
  source 1..15: mol_type = other DNA
gccgctgcccaatgc

SEQ ID NO: 696 - DNA, 18 bp, synthetic construct
  misc_feature 1..18: note = Synthesized DNA
  source 1..18: mol_type = other DNA
cgctgcccaatgccatcc

SEQ ID NO: 697 - DNA, 18 bp, synthetic construct
  misc_feature 1..18: note = Synthesized DNA
  source 1..18: mol_type = other DNA
cagtttgccgctgcccaa

SEQ ID NO: 698 - DNA, 26 bp, synthetic construct
  misc_feature 1..26: note = Synthesized DNA
  source 1..26: mol_type = other DNA
ccaatgccatcctggagttcctgtaa

SEQ ID NO: 699 - DNA, 22 bp, synthetic construct
  misc_feature 1..22: note = Synthesized DNA
  source 1..22: mol_type = other DNA
caatgccatcctggagttcctg

SEQ ID NO: 700 - DNA, 30 bp, synthetic construct
  misc_feature 1..30: note = Synthesized DNA
  source 1..30: mol_type = other DNA
tgctgctcttttccaggttcaagtgggata

SEQ ID NO: 701 - DNA, 30 bp, synthetic construct
  misc_feature 1..30: note = Synthesized DNA
  source 1..30: mol_type = other DNA
cttttagttgctgctcttttccaggttcaa

SEQ ID NO: 702 - DNA, 30 bp, synthetic construct
  misc_feature 1..30: note = Synthesized DNA
  source 1..30: mol_type = other DNA
cttttcttttagttgctgctcttttccagg

SEQ ID NO: 703 - DNA, 30 bp, synthetic construct
  misc_feature 1..30: note = Synthesized DNA
  source 1..30: mol_type = other DNA
ttagttgctgctcttttccaggttcaagtg

SEQ ID NO: 704 - DNA, 30 bp, synthetic construct
  misc_feature 1..30: note = Synthesized DNA
  source 1..30: mol_type = other DNA
ctccaacatcaaggaagatggcatttctag

SEQ ID NO: 705 - DNA, 20 bp, synthetic construct
  misc_feature 1..20: note = Synthesized DNA
  source 1..20: mol_type = other DNA
tcaaggaagatggcatttct

SEQ ID NO: 706 - DNA, 25 bp, synthetic construct
  misc_feature 1..25: note = Synthesized DNA
  source 1..25: mol_type = other DNA
ggccaaacctcggcttacctgaaat

SEQ ID NO: 707 - DNA, 25 bp, synthetic construct
  misc_feature 1..25: note = Synthesized DNA
  source 1..25: mol_type = other DNA
gaacaccttcagaaccggaggcaac

SEQ ID NO: 708 - DNA, 16 bp, synthetic construct
  misc_feature 1..16: note = Synthesized DNA
  source 1..16: mol_type = other DNA
gaacaccttcagaacc

SEQ ID NO: 709 - DNA, 21 bp, synthetic construct
  misc_feature 1..21: note = Synthesized DNA
  source 1..21: mol_type = other DNA
gaacaccttcagaaccggagg

SEQ ID NO: 710 - DNA, 16 bp, synthetic construct
  misc_feature 1..16: note = Synthesized DNA
  source 1..16: mol_type = other DNA
ccttcagaaccggagg

SEQ ID NO: 711 - DNA, 16 bp, synthetic construct
  misc_feature 1..16: note = Synthesized DNA
  source 1..16: mol_type = other DNA
cagaaccggaggcaac

SEQ ID NO: 712 - DNA, 19 bp, synthetic construct
  misc_feature 1..19: note = Synthesized polynucleotide
  source 1..19: mol_type = other DNA
  modified_base 12: mod_base = OTHER; note = This t is uracil.
gaacacctaaatcagaacc

SEQ ID NO: 713 - DNA, 25 bp, synthetic construct
  misc_feature 1..25: note = Synthesized DNA
  source 1..25: mol_type = other DNA
gaacacaaattcagaaaaacggagg

SEQ ID NO: 714 - DNA, 19 bp, synthetic construct
  misc_feature 1..19: note = Synthesized DNA
  source 1..19: mol_type = other DNA
tcagaacaccttcagaacc

SEQ ID NO: 715 - RNA, 21 nt, synthetic construct
  misc_feature 1..21: note = Synthesized RNA
  source 1..21: mol_type = other RNA
gaacaccttcagaaccggagg

SEQ ID NO: 716 - RNA, 25 nt, synthetic construct
  misc_feature 1..25: note = Synthesized RNA
  source 1..25: mol_type = other RNA
atttcaggtaagccgaggtttggcc

SEQ ID NO: 717 - RNA, 16 nt, synthetic construct
  misc_feature 1..16: note = Synthesized RNA
  source 1..16: mol_type = other RNA
atttcaggtaagccga

SEQ ID NO: 718 - DNA, 25 bp, synthetic construct
  misc_feature 1..25: note = Synthesized polynucletide
  source 1..25: mol_type = other DNA
  modified_base 2..3: mod_base = OTHER; note = This t is uracil.
atttcaggtaagccgaggtttggcc

SEQ ID NO: 719 - RNA, 25 nt, synthetic construct
  misc_feature 1..25: note = Synthesized RNA
  source 1..25: mol_type = other RNA
atttcaaaagtaagccaaaaggttt

SEQ ID NO: 720 - DNA, 16 bp, synthetic construct
  misc_feature 1..16: note = Synthesized polynucleotide
  source 1..16: mol_type = other DNA
  modified_base 2..3: mod_base = OTHER; note = This t is uracil.
atttcaggtaagccga

SEQ ID NO: 721 - DNA, 16 bp, synthetic construct
  misc_feature 1..16: note = Synthesized DNA
  source 1..16: mol_type = other DNA
atttcaggtaagccga

SEQ ID NO: 722 - DNA, 25 bp, synthetic construct
  misc_feature 1..25: note = Synthesized DNA
  source 1..25: mol_type = other DNA
atttcaggtaagccgaggtttggcc

SEQ ID NO: 723 - protein, 15 aa, synthetic construct
  REGION 1..15: note = Synthesized polypeptide
  SITE 3: note = MISC_FEATURE - Xaa is MeF3C
  SITE 5: note = MISC_FEATURE - Xaa is W1aa
  SITE 8: note = MISC_FEATURE - Xaa is F4aao
  MOD_RES 14: note = METHYLATION
AVXVXNYXIIRRFYC

SEQ ID NO: 724 - protein, 15 aa, synthetic construct
  REGION 1..15: note = Synthesized polypeptide
  SITE 3: note = MISC_FEATURE - Xaa is MeF3C
  SITE 5: note = MISC_FEATURE - Xaa is W1aa
  SITE 8: note = MISC_FEATURE - Xaa is F4OMe
  MOD_RES 14: note = METHYLATION
AVXVXNYXIERRFYC

SEQ ID NO: 725 - protein, 15 aa, synthetic construct
  REGION 1..15: note = Synthesized polypeptide
  SITE 3: note = MISC_FEATURE - Xaa is MeF3C
  SITE 5: note = MISC_FEATURE - Xaa is W1aa
  SITE 8: note = MISC_FEATURE - Xaa is F4aao
  MOD_RES 14: note = METHYLATION
AVXVXNYXIIRRFYC

SEQ ID NO: 726 - protein, 5 aa, synthetic construct
GGGGS

SEQ ID NO: 727 - protein, 5 aa, synthetic construct
SSSSG

SEQ ID NO: 728 - DNA, 25 bp, synthetic construct
  source 1..25: mol_type = other DNA
  misc_feature 1..25: note = These nucleotides are morpholino nucleotides.
gttgcctccggttctgaaggtgttc

SEQ ID NO: 729 - DNA, 21 bp, synthetic construct
  source 1..21: mol_type = other DNA
  misc_feature 1..21: note = These nucleotides are morpholino nucleotides.
cctccggttctgaaggtgttc

SEQ ID NO: 730 - DNA, 25 bp, synthetic construct
  source 1..25: mol_type = other DNA
  misc_feature 1..25: note = These nucleotides are morpholino nucleotides.
ggccaaacctcggcttacctgaaat

SEQ ID NO: 731 - DNA, 25 bp, synthetic construct
  source 1..25: mol_type = other DNA
  misc_feature 4: note = DNA
  misc_feature 6..10: note = DNA
  misc_feature 15..16: note = DNA
  misc_feature 22: note = DNA
  modified_base 1: mod_base = gm
  modified_base 2..3: mod_base = OTHER; note = These bases are 2-O-methyl nucleosides
  modified_base 23..24: mod_base = OTHER; note = These bases are 2-O-methyl nucleosides
  modified_base 25: mod_base = cm
  misc_feature 1..3: note = These nucleotides are bound via phosphorothioate linkages.
  misc_feature 22..24: note = These nucleotides are bound via phosphorothioate linkages.
gaacaccttcagaaccggaggcaac

SEQ ID NO: 732 - RNA, 25 nt, synthetic construct
  source 1..25: mol_type = other RNA
  modified_base 1: mod_base = gm
  modified_base 25: mod_base = cm
  modified_base 25: mod_base = cm
  modified_base 2..3: mod_base = OTHER; note = These bases are 2-O-methyl nucleosides.
  modified_base 23..24: mod_base = OTHER; note = These bases are 2-O-methyl nucleosides.
  modified_base 1..3: mod_base = OTHER; note = These nucleotides are bound via phosphorothioate linkages.
  modified_base 22..24: mod_base = OTHER; note = These nucleotides are bound via phosphorothioate linkages.
gaacaccttcagaaccggaggcaac

SEQ ID NO: 733 - DNA, 25 bp, synthetic construct
  source 1..25: mol_type = other DNA
  modified_base 1..3: mod_base = OTHER; note = These nucleotides are bound via phosphorothioate linkages.
  modified_base 22..24: mod_base = OTHER; note = These nucleotides are bound via phosphorothioate linkages.
  modified_base 16: mod_base = OTHER; note = This cytosine is a 5-methyle cytosine.
gaacaccttcagaaccggaggcaac

SEQ ID NO: 734 - RNA, 16 nt, synthetic construct
  source 1..16: mol_type = other RNA
  modified_base 1..3: mod_base = OTHER; note = These nucleotides are bound via phosphorothioate linkages.
  modified_base 1: mod_base = gm
  modified_base 2..3: mod_base = OTHER; note = These bases are 2-O-methyl nucleosides.
  modified_base 14: mod_base = OTHER; note = These bases are 2-O-methyl nucleosides.
  modified_base 15..16: mod_base = cm
  modified_base 13..15: mod_base = OTHER; note = These nucleotides are bound via phosphorothioate linkages.
gaacaccttcagaacc

SEQ ID NO: 735 - DNA, 25 bp, synthetic construct
  misc_feature 4..22: note = DNA
  source 1..25: mol_type = other DNA
  modified_base 1..3: mod_base = OTHER; note = These nucleotides are bound via phosphorothioate linkages.
  modified_base 25: mod_base = cm
  modified_base 16: mod_base = OTHER; note = This cytosine is a 5-methyle cytosine.
  misc_feature 22..24: note = These nucleotides are bound via phosphorothioate linkages.
  modified_base 1: mod_base = gm
  modified_base 2..3: mod_base = OTHER; note = These bases are 2-O-methyl nucleosides.
  modified_base 23..24: mod_base = OTHER; note = These bases are 2-O-methyl nucleosides.
gaacaccttcagaaccggaggcaac

SEQ ID NO: 736 - RNA, 25 nt, synthetic construct
  source 1..25: mol_type = other RNA
  modified_base 1..3: mod_base = OTHER; note = These nucleotides are bound via phosphorothioate linkages.
  modified_base 22..24: mod_base = OTHER; note = These nucleotides are bound via phosphorothioate linkages.
  modified_base 1: mod_base = gm
  modified_base 2..3: mod_base = OTHER; note = These bases are 2-O-methyl nucleosides.
  modified_base 4: mod_base = cm
  modified_base 6..7: mod_base = cm
  modified_base 8..9: mod_base = um
  modified_base 10: mod_base = cm
  modified_base 15..16: mod_base = cm
  modified_base 22: mod_base = cm
  modified_base 23..24: mod_base = OTHER; note = These bases are 2-O-methyl nucleosides.
  modified_base 25: mod_base = cm
gaacaccttcagaaccggaggcaac

SEQ ID NO: 737 - DNA, 25 bp, synthetic construct
  misc_feature 4: note = DNA
  source 1..25: mol_type = other DNA
  misc_feature 6..10: note = DNA
  misc_feature 15..16: note = DNA
  misc_feature 22: note = DNA
  modified_base 25: mod_base = OTHER; note = This cytosine is a 5-methyle cytosine.
  modified_base 1..3: mod_base = OTHER; note = These nucleosides are 2-4-BNA NC [N-Me] nucleosides.
  modified_base 22..24: mod_base = OTHER; note = These nucleotides are bound via phosphorothioate linkages.
  modified_base 23..25: mod_base = OTHER; note = These nucleosides are 2-4-BNA NC [N-Me] nucleosides.
  modified_base 1..3: mod_base = OTHER; note = These nucleotides are bound via phosphorothioate linkages.
gaacaccttcagaaccggaggcaac

SEQ ID NO: 738 - DNA, 25 bp, synthetic construct
  misc_feature 4: note = DNA
  source 1..25: mol_type = other DNA
  misc_feature 6..10: note = DNA
  misc_feature 15..16: note = DNA
  misc_feature 22: note = DNA
  modified_base 1..3: mod_base = OTHER; note = These nucleosides are 2-4-BNA NC [N-Me] nucleosides.
  modified_base 23..25: mod_base = OTHER; note = These nucleosides are 2-4-BNA NC [N-Me] nucleosides.
  modified_base 25: mod_base = OTHER; note = This cytosine is a 5-methyle cytosine.
gaacaccttcagaaccggaggcaac

SEQ ID NO: 739 - RNA, 25 nt, synthetic construct
  source 1..25: mol_type = other RNA
  modified_base 1..3: mod_base = OTHER; note = These nucleosides are 2-4-BNA NC [N-Me] nucleosides.
  modified_base 23..25: mod_base = OTHER; note = These nucleosides are 2-4-BNA NC [N-Me] nucleosides.
  modified_base 25: mod_base = OTHER; note = This cytosine is a 5-methyle cytosine.
  modified_base 1..3: mod_base = OTHER; note = These nucleotides are bound via phosphorothioate linkages.
  modified_base 22..24: mod_base = OTHER; note = These nucleotides are bound via phosphorothioate linkages.
gaacaccttcagaaccggaggcaac

SEQ ID NO: 740 - DNA, 21 bp, synthetic construct
  misc_feature 4..18: note = DNA
  source 1..21: mol_type = other DNA
  modified_base 1..3: mod_base = OTHER; note = These nucleotides are bound via phosphorothioate linkages.
  modified_base 18..20: mod_base = OTHER; note = These nucleotides are bound via phosphorothioate linkages.
  modified_base 1: mod_base = gm
  modified_base 2..3: mod_base = OTHER; note = These bases are 2-O-methyl nucleosides.
  modified_base 19: mod_base = OTHER; note = These bases are 2-O-methyl nucleosides.
  modified_base 20..21: mod_base = gm
gaacaccttcagaaccggagg

SEQ ID NO: 741 - DNA, 21 bp, synthetic construct
  misc_feature 4: note = DNA
  source 1..21: mol_type = other DNA
  misc_feature 6..10: note = DNA
  misc_feature 15..16: note = DNA
  modified_base 1: mod_base = gm
  modified_base 2..3: mod_base = OTHER; note = These bases are 2-O-methyl nucleosides.
  modified_base 19: mod_base = OTHER; note = These bases are 2-O-methyl nucleosides.
  modified_base 20..21: mod_base = gm
  modified_base 1..3: mod_base = OTHER; note = These nucleotides are bound via phosphorothioate linkages.
  modified_base 18..20: mod_base = OTHER; note = These nucleotides are bound via phosphorothioate linkages.
gaacaccttcagaaccggagg

SEQ ID NO: 742 - RNA, 21 nt, synthetic construct
  source 1..21: mol_type = other RNA
  modified_base 1: mod_base = gm
  modified_base 2..3: mod_base = OTHER; note = These bases are 2-O-methyl nucleosides.
  modified_base 4: mod_base = cm
  modified_base 6..7: mod_base = cm
  modified_base 8..9: mod_base = um
  modified_base 10: mod_base = cm
  modified_base 15..16: mod_base = cm
  modified_base 19: mod_base = OTHER; note = These bases are 2-O-methyl nucleosides.
  modified_base 20..21: mod_base = gm
  modified_base 1..3: mod_base = OTHER; note = These nucleotides are bound via phosphorothioate linkages.
  modified_base 18..20: mod_base = OTHER; note = These nucleotides are bound via phosphorothioate linkages.
gaacaccttcagaaccggagg

SEQ ID NO: 743 - DNA, 21 bp, synthetic construct
  misc_feature 5: note = DNA
  source 1..21: mol_type = other DNA
  misc_feature 11..14: note = DNA
  misc_feature 17..18: note = DNA
  modified_base 1: mod_base = gm
  modified_base 2..3: mod_base = OTHER; note = These bases are 2-O-methyl nucleosides.
  modified_base 4: mod_base = cm
  modified_base 6..7: mod_base = cm
  modified_base 8..9: mod_base = um
  modified_base 10: mod_base = cm
  modified_base 15..16: mod_base = cm
  modified_base 19: mod_base = OTHER; note = These bases are 2-O-methyl nucleosides.
  modified_base 20..21: mod_base = gm
  modified_base 1..3: mod_base = OTHER; note = These nucleotides are bound via phosphorothioate linkages.
  modified_base 18..20: mod_base = OTHER; note = These nucleotides are bound via phosphorothioate linkages.
gaacaccttcagaaccggagg

SEQ ID NO: 744 - RNA, 21 nt, synthetic construct
  source 1..21: mol_type = other RNA
  modified_base 1..3: mod_base = OTHER; note = These nucleosides are 2-4-BNA NC [N-Me] nucleosides.
  modified_base 19..21: mod_base = OTHER; note = These nucleosides are 2-4-BNA NC [N-Me] nucleosides.
  modified_base 1..3: mod_base = OTHER; note = These nucleotides are bound via phosphorothioate linkages.
  modified_base 18..20: mod_base = OTHER; note = These nucleotides are bound via phosphorothioate linkages.
gaacaccttcagaaccggagg

SEQ ID NO: 745 - DNA, 21 bp, synthetic construct
  misc_feature 4..18: note = DNA
  source 1..21: mol_type = other DNA
  modified_base 16: mod_base = OTHER; note = This cytosine is a 5-methyle cytosine.
  modified_base 1..3: mod_base = OTHER; note = These nucleosides are 2-4-BNA NC [N-Me] nucleosides.
  modified_base 19..21: mod_base = OTHER; note = These nucleosides are 2-4-BNA NC [N-Me] nucleosides.
  modified_base 1..3: mod_base = OTHER; note = These nucleotides are bound via phosphorothioate linkages.
  modified_base 18..20: mod_base = OTHER; note = These nucleotides are bound via phosphorothioate linkages.
gaacaccttcagaaccggagg

SEQ ID NO: 746 - DNA, 16 bp, synthetic construct
  misc_feature 4: note = DNA
  source 1..16: mol_type = other DNA
  misc_feature 6..10: note = DNA
  modified_base 1: mod_base = gm
  modified_base 2..3: mod_base = OTHER; note = These bases are 2-O-methyl nucleosides.
  modified_base 14: mod_base = OTHER; note = Theis base is 2-O-methyl nucleoside.
  modified_base 15..16: mod_base = cm
  modified_base 13..15: mod_base = OTHER; note = These nucleotides are bound via phosphorothioate linkages.
gaacaccttcagaacc

SEQ ID NO: 747 - DNA, 16 bp, synthetic construct
  source 1..16: mol_type = other DNA
  misc_feature 10..11: note = DNA
  misc_feature 4..5: note = DNA
  modified_base 3: mod_base = um
  modified_base 1..2: mod_base = cm
  modified_base 14: mod_base = OTHER; note = This base is a 2-O-methyl nucleoside
  modified_base 15..16: mod_base = gm
  modified_base 1..3: mod_base = OTHER; note = These nucleotides are bound via phosphorothioate linkages.
  modified_base 13..15: mod_base = OTHER; note = These nucleotides are bound via phosphorothioate linkages.
ccttcagaaccggagg

SEQ ID NO: 748 - RNA, 16 nt, synthetic construct
  source 1..16: mol_type = other RNA
  modified_base 1: mod_base = gm
  modified_base 2..3: mod_base = OTHER; note = These bases are 2-O-methyl nucleosides.
  modified_base 4: mod_base = cm
  modified_base 6..7: mod_base = cm
  modified_base 8..9: mod_base = um
  modified_base 10: mod_base = cm
  modified_base 14: mod_base = OTHER; note = These bases are 2-O-methyl nucleosides.
  modified_base 15..16: mod_base = cm
  modified_base 1..3: mod_base = OTHER; note = These nucleotides are bound via phosphorothioate linkages.
  modified_base 13..15: mod_base = OTHER; note = These nucleotides are bound via phosphorothioate linkages.
gaacaccttcagaacc

SEQ ID NO: 749 - RNA, 16 nt, synthetic construct
  source 1..16: mol_type = other RNA
  modified_base 1..2: mod_base = cm
  modified_base 3..4: mod_base = um
  modified_base 5: mod_base = cm
  modified_base 10..11: mod_base = cm
  modified_base 14: mod_base = OTHER; note = This base is a 2-O-methyl nucleoside.
  modified_base 15..16: mod_base = gm
  modified_base 1..3: mod_base = OTHER; note = These nucleotides are bound via phosphorothioate linkages.
  modified_base 13..15: mod_base = OTHER; note = These nucleotides are bound via phosphorothioate linkages.
ccttcagaaccggagg

SEQ ID NO: 750 - RNA, 16 nt, synthetic construct
  source 1..16: mol_type = other RNA
  modified_base 1: mod_base = cm
  modified_base 2: mod_base = OTHER; note = This base is a 2-O-methyl nucleoside.
  modified_base 3: mod_base = gm
  modified_base 6..7: mod_base = cm
  modified_base 13: mod_base = cm
  modified_base 14..15: mod_base = OTHER; note = These bases are 2-O-methyl nucleosides.
  modified_base 16: mod_base = cm
  modified_base 1..3: mod_base = OTHER; note = These nucleotides are bound via phosphorothioate linkages.
  modified_base 13..15: mod_base = OTHER; note = These nucleotides are bound via phosphorothioate linkages.
cagaaccggaggcaac

SEQ ID NO: 751 - DNA, 16 bp, synthetic construct
  misc_feature 5: note = DNA
  source 1..16: mol_type = other DNA
  misc_feature 11..13: note = DNA
  modified_base 1: mod_base = gm
  modified_base 2..3: mod_base = OTHER; note = These bases are 2-O-methyl nucleosides.
  modified_base 4: mod_base = cm
  modified_base 6..7: mod_base = cm
  modified_base 8..9: mod_base = um
  modified_base 10: mod_base = cm
  modified_base 14: mod_base = OTHER; note = This base is a 2-O-methyl nucleoside.
  modified_base 15..16: mod_base = cm
  modified_base 1..3: mod_base = OTHER; note = These nucleotides are bound via phosphorothioate linkages.
  modified_base 13..15: mod_base = OTHER; note = These nucleotides are bound via phosphorothioate linkages.
gaacaccttcagaacc

SEQ ID NO: 752 - DNA, 16 bp, synthetic construct
  misc_feature 4: note = DNA
  source 1..16: mol_type = other DNA
  misc_feature 6: note = DNA
  misc_feature 8: note = DNA
  misc_feature 10..13: note = DNA
  modified_base 1: mod_base = gm
  modified_base 2..3: mod_base = OTHER; note = These bases are 2-O-methyl nucleosides.
  modified_base 14: mod_base = OTHER; note = This base is a 2-O-methyl nucleoside.
  modified_base 15..16: mod_base = cm
  modified_base 1..3: mod_base = OTHER; note = These nucleotides are bound via phosphorothioate linkages.
  modified_base 13..15: mod_base = OTHER; note = These nucleotides are bound via phosphorothioate linkages.
gaacaccttcagaacc

SEQ ID NO: 753 - DNA, 16 bp, synthetic construct
  misc_feature 4..5: note = DNA
  source 1..16: mol_type = other DNA
  misc_feature 8: note = DNA
  misc_feature 10..13: note = DNA
  modified_base 9: mod_base = OTHER; note = This t is uracil.
  modified_base 1: mod_base = gm
  modified_base 2..3: mod_base = OTHER; note = These bases are 2-O-methyl nucleosides.
  modified_base 7: mod_base = cm
  modified_base 14: mod_base = OTHER; note = This base is a 2-O-methyl nucleoside.
  modified_base 15..16: mod_base = cm
  modified_base 1..3: mod_base = OTHER; note = These nucleotides are bound via phosphorothioate linkages.
  modified_base 13..15: mod_base = OTHER; note = These nucleotides are bound via phosphorothioate linkages.
gaacaccttcagaacc

SEQ ID NO: 754 - RNA, 16 nt, synthetic construct
  source 1..16: mol_type = other RNA
  modified_base 1..3: mod_base = OTHER; note = These nucleosides are 2-4-BNA NC [N-Me] nucleosides.
  modified_base 14..16: mod_base = OTHER; note = These nucleosides are 2-4-BNA NC [N-Me] nucleosides.
  modified_base 13..15: mod_base = OTHER; note = These nucleotides are bound via phosphorothioate linkages.
  modified_base 15..16: mod_base = OTHER; note = These cytosines are 5-methyle cytosines.
  modified_base 1..3: mod_base = OTHER; note = These nucleotides are bound via phosphorothioate linkages.
gaacaccttcagaacc

SEQ ID NO: 755 - DNA, 16 bp, synthetic construct
  misc_feature 4: note = DNA
  source 1..16: mol_type = other DNA
  misc_feature 6..10: note = DNA
  modified_base 1..3: mod_base = OTHER; note = These nucleosides are 2-4-BNA NC [N-Me] nucleosides.
  modified_base 14..16: mod_base = OTHER; note = These nucleosides are 2-4-BNA NC [N-Me] nucleosides.
  modified_base 1..3: mod_base = OTHER; note = These nucleotides are bound via phosphorothioate linkages.
  modified_base 13..15: mod_base = OTHER; note = These nucleotides are bound via phosphorothioate linkages.
  modified_base 15..16: mod_base = OTHER; note = These cytosines are 5-methyle cytosines.
gaacaccttcagaacc

SEQ ID NO: 756 - DNA, 16 bp, synthetic construct
  misc_feature 4..5: note = DNA
  source 1..16: mol_type = other DNA
  misc_feature 8: note = DNA
  misc_feature 10..13: note = DNA
  modified_base 1..3: mod_base = OTHER; note = These nucleosides are 2-4-BNA NC [N-Me] nucleosides.
  modified_base 14..16: mod_base = OTHER; note = These nucleosides are 2-4-BNA NC [N-Me] nucleosides.
  modified_base 7: mod_base = cm
  modified_base 9: mod_base = OTHER; note = This t is uracil.
  modified_base 1..3: mod_base = OTHER; note = These nucleotides are bound via phosphorothioate linkages.
  modified_base 13..15: mod_base = OTHER; note = These nucleotides are bound via phosphorothioate linkages.
  modified_base 15..16: mod_base = OTHER; note = These cytosines are 5-methyle cytosines.
gaacaccttcagaacc

SEQ ID NO: 757 - DNA, 19 bp, synthetic construct
  misc_feature 9..11: note = DNA
  source 1..19: mol_type = other DNA
  modified_base 1: mod_base = gm
  modified_base 2..3: mod_base = OTHER; note = These bases are 2-O-methyl nucleosides.
  modified_base 4: mod_base = cm
  modified_base 5: mod_base = OTHER; note = This base is a 2-O-methyl nucleoside.
  modified_base 6..7: mod_base = cm
  modified_base 8: mod_base = um
  modified_base 12: mod_base = um
  modified_base 13: mod_base = cm
  modified_base 14: mod_base = OTHER; note = This base is a 2-O-methyl nucleoside.
  modified_base 15: mod_base = gm
  modified_base 16..17: mod_base = OTHER; note = These bases are 2-O-methyl nucleosides.
  modified_base 18..19: mod_base = cm
  modified_base 1..3: mod_base = OTHER; note = These nucleotides are bound via phosphorothioate linkages.
  modified_base 16..18: mod_base = OTHER; note = These nucleotides are bound via phosphorothioate linkages.
gaacacctaaatcagaacc

SEQ ID NO: 758 - DNA, 25 bp, synthetic construct
  misc_feature 7..9: note = DNA
  source 1..25: mol_type = other DNA
  misc_feature 17..19: note = DNA
  modified_base 1: mod_base = gm
  modified_base 2..3: mod_base = OTHER; note = These bases are 2-O-methyl nucleosides.
  modified_base 4: mod_base = cm
  modified_base 5: mod_base = OTHER; note = This base is a 2-O-methyl nucleoside.
  modified_base 6: mod_base = cm
  modified_base 10..11: mod_base = um
  modified_base 12: mod_base = cm
  modified_base 13: mod_base = OTHER; note = This base is a 2-O-methyl nucleoside.
  modified_base 14: mod_base = gm
  modified_base 15..16: mod_base = OTHER; note = These bases are 2-O-methyl nucleosides.
  modified_base 20: mod_base = cm
  modified_base 21..22: mod_base = gm
  modified_base 23: mod_base = OTHER; note = This base is a 2-O-methyl nucleoside.
  modified_base 24..25: mod_base = gm
  modified_base 1..3: mod_base = OTHER; note = These nucleotides are bound via phosphorothioate linkages.
  modified_base 22..24: mod_base = OTHER; note = These nucleotides are bound via phosphorothioate linkages.
gaacacaaattcagaaaaacggagg

SEQ ID NO: 759 - DNA, 16 bp, synthetic construct
  misc_feature 4: note = DNA
  source 1..16: mol_type = other DNA
  misc_feature 6..10: note = DNA
  modified_base 1: mod_base = gm
  modified_base 2..3: mod_base = OTHER; note = These bases are 2-O-methyl nucleosides.
  modified_base 14: mod_base = OTHER; note = This base is a 2-O-methyl nucleoside.
  modified_base 15..16: mod_base = cm
  modified_base 1..3: mod_base = OTHER; note = These nucleotides are bound via phosphorothioate linkages.
  modified_base 13..15: mod_base = OTHER; note = These nucleotides are bound via phosphorothioate linkages.
gaacaccttcagaacc

SEQ ID NO: 760 - DNA, 19 bp, synthetic construct
  misc_feature 1..3: note = DNA
  source 1..19: mol_type = other DNA
  misc_feature 7: note = DNA
  misc_feature 9..13: note = DNA
  modified_base 17: mod_base = OTHER; note = This base is a 2-O-methyl nucleoside.
  modified_base 18..19: mod_base = cm
  modified_base 16..18: mod_base = OTHER; note = These nucleotides are bound via phosphorothioate linkages.
tcagaacaccttcagaacc

SEQ ID NO: 761 - DNA, 25 bp, synthetic construct
  misc_feature 4: note = DNA
  source 1..25: mol_type = other DNA
  misc_feature 6..10: note = DNA
  misc_feature 15..16: note = DNA
  misc_feature 22: note = DNA
  modified_base 1: mod_base = gm
  modified_base 25: mod_base = cm
  modified_base 1: mod_base = OTHER; note = This nucleotide is bound via a phosphorothioate linkage.
  modified_base 24: mod_base = OTHER; note = This nucleotide is bound via a phosphorothioate linkage.
gaacaccttcagaaccggaggcaac

SEQ ID NO: 762 - DNA, 16 bp, synthetic construct
  source 1..16: mol_type = other DNA
gaacaccttcagaacc

SEQ ID NO: 763 - DNA, 25 bp, synthetic construct
  source 1..25: mol_type = other DNA
  modified_base 16: mod_base = OTHER; note = This cytosine is a 5-methyle cytosine.
gaacaccttcagaaccggaggcaac

SEQ ID NO: 764 - DNA, 21 bp, synthetic construct
  source 1..21: mol_type = other DNA
  modified_base 16: mod_base = OTHER; note = This cytosine is a 5-methyle cytosine.
gaacaccttcagaaccggagg

SEQ ID NO: 765 - RNA, 21 nt, synthetic construct
  source 1..21: mol_type = other RNA
  modified_base 1: mod_base = gm
  modified_base 2..3: mod_base = OTHER; note = These bases are 2-O-methyl nucleosides.
  modified_base 19: mod_base = OTHER; note = This base is a 2-O-methyl nucleoside.
  modified_base 20..21: mod_base = gm
  modified_base 1..3: mod_base = OTHER; note = These nucleotides are bound via phosphorothioate linkages.
  modified_base 18..20: mod_base = OTHER; note = These nucleotides are bound via phosphorothioate linkages.
gaacaccttcagaaccggagg

SEQ ID NO: 766 - RNA, 25 nt, synthetic construct
  source 1..25: mol_type = other RNA
  modified_base 1: mod_base = OTHER; note = This base is a 2-O-methyl nucleoside.
  modified_base 2..3: mod_base = um
  modified_base 23: mod_base = gm
  modified_base 24..25: mod_base = cm
  modified_base 1..3: mod_base = OTHER; note = These nucleotides are bound via phosphorothioate linkages.
  modified_base 22..24: mod_base = OTHER; note = These nucleotides are bound via phosphorothioate linkages.
atttcaggtaagccgaggtttggcc

SEQ ID NO: 767 - RNA, 16 nt, synthetic construct
  source 1..16: mol_type = other RNA
  modified_base 1: mod_base = OTHER; note = This base is a 2-O-methyl nucleoside.
  modified_base 16: mod_base = OTHER; note = This base is a 2-O-methyl nucleoside.
  modified_base 2..3: mod_base = um
  modified_base 14: mod_base = cm
  modified_base 15: mod_base = gm
  modified_base 1..3: mod_base = OTHER; note = These nucleotides are bound via phosphorothioate linkages.
  modified_base 13..15: mod_base = OTHER; note = These nucleotides are bound via phosphorothioate linkages.
atttcaggtaagccga

SEQ ID NO: 768 - DNA, 25 bp, synthetic construct
  misc_feature 4..5: note = DNA
  source 1..25: mol_type = other DNA
  misc_feature 9: note = DNA
  misc_feature 13..14: note = DNA
  misc_feature 19..21: note = DNA
  modified_base 1: mod_base = OTHER; note = This base is a 2-O-methyl nucleoside.
  modified_base 2..3: mod_base = um
  modified_base 23: mod_base = gm
  modified_base 24..25: mod_base = cm
  modified_base 1..3: mod_base = OTHER; note = These nucleotides are bound via phosphorothioate linkages.
  modified_base 22..24: mod_base = OTHER; note = These nucleotides are bound via phosphorothioate linkages.
atttcaggtaagccgaggtttggcc

SEQ ID NO: 769 - DNA, 16 bp, synthetic construct
  misc_feature 4..5: note = DNA
  source 1..16: mol_type = other DNA
  misc_feature 9: note = DNA
  misc_feature 13: note = DNA
  modified_base 1: mod_base = OTHER; note = This base is a 2-O-methyl nucleoside.
  modified_base 2..3: mod_base = um
  modified_base 14: mod_base = cm
  modified_base 15: mod_base = gm
  modified_base 16: mod_base = OTHER; note = This base is a 2-O-methyl nucleoside.
  modified_base 1..3: mod_base = OTHER; note = These nucleotides are bound via phosphorothioate linkages.
  modified_base 13..15: mod_base = OTHER; note = These nucleotides are bound via phosphorothioate linkages.
atttcaggtaagccga

SEQ ID NO: 770 - DNA, 25 bp, synthetic construct
  source 1..25: mol_type = other DNA
  misc_feature 7..9: note = DNA
  misc_feature 17..19: note = DNA
  modified_base 1: mod_base = OTHER; note = This base is a 2-O-methyl nucleoside.
  modified_base 2..4: mod_base = um
  modified_base 5: mod_base = cm
  modified_base 6: mod_base = OTHER; note = This base is a 2-O-methyl nucleoside.
  modified_base 10: mod_base = gm
  modified_base 11: mod_base = um
  modified_base 12..13: mod_base = OTHER; note = These bases are 2-O-methyl nucleosides.
  modified_base 14: mod_base = gm
  modified_base 15..16: mod_base = cm
  modified_base 20: mod_base = OTHER; note = This base is a 2-O-methyl nucleoside.
  modified_base 21..22: mod_base = gm
  modified_base 23..25: mod_base = um
  modified_base 1..3: mod_base = OTHER; note = These nucleotides are bound via phosphorothioate linkages.
  modified_base 22..24: mod_base = OTHER; note = These nucleotides are bound via phosphorothioate linkages.
atttcaaaagtaagccaaaaggttt

SEQ ID NO: 771 - DNA, 16 bp, synthetic construct
  misc_feature 4..5: note = DNA
  source 1..16: mol_type = other DNA
  misc_feature 9: note = DNA
  misc_feature 13: note = DNA
  modified_base 1: mod_base = OTHER; note = This base is a 2-O-methyl nucleoside.
  modified_base 2..3: mod_base = um
  modified_base 14: mod_base = cm
  modified_base 15: mod_base = gm
  modified_base 16: mod_base = OTHER; note = This base is a 2-O-methyl nucleoside.
  modified_base 1..3: mod_base = OTHER; note = These nucleotides are bound via phosphorothioate linkages.
  modified_base 13..15: mod_base = OTHER; note = These nucleotides are bound via phosphorothioate linkages.
  modified_base 16: mod_base = OTHER; note = This nucleotide is modified with Y3.
atttcaggtaagccga

SEQ ID NO: 772 - DNA, 16 bp, synthetic construct
  misc_feature 4..5: note = DNA
  source 1..16: mol_type = other DNA
  misc_feature 9: note = DNA
  misc_feature 13: note = DNA
  modified_base 1..3: mod_base = OTHER; note = These nucleotides are bound via phosphorothioate linkages.
  modified_base 13..15: mod_base = OTHER; note = These nucleotides are bound via phosphorothioate linkages.
  modified_base 1..3: mod_base = OTHER; note = These nucleosides are 2-4-BNA NC [N-Me] nucleosides.
  modified_base 14..16: mod_base = OTHER; note = These nucleosides are 2-4-BNA NC [N-Me] nucleosides.
  modified_base 14: mod_base = OTHER; note = This cytosine is a 5-methyle cytosine.
atttcaggtaagccga

SEQ ID NO: 773 - DNA, 25 bp, synthetic construct
  source 1..25: mol_type = other DNA
  modified_base 14: mod_base = OTHER; note = This cytosine is a 5-methyle cytosine.
atttcaggtaagccgaggtttggcc

SEQ ID NO: 774 - RNA, 25 nt, synthetic construct
  source 1..25: mol_type = other RNA
  modified_base 1..25: mod_base = OTHER; note = These nucleotides are morpholino nucleotides.
  modified_base 1: mod_base = OTHER; note = This nucleotide is modified with Y1.
gttgcctccggttctgaaggtgttc

SEQ ID NO: 775 - RNA, 21 nt, synthetic construct
  source 1..21: mol_type = other RNA
  modified_base 1..21: mod_base = OTHER; note = These nucleotides are morpholino nucleotides.
  modified_base 1: mod_base = OTHER; note = This nucleotide is modified with Y1.
cctccggttctgaaggtgttc

SEQ ID NO: 776 - RNA, 25 nt, synthetic construct
  source 1..25: mol_type = other RNA
  modified_base 1: mod_base = OTHER; note = This nucleotide is modified with Y1.
  modified_base 25: mod_base = OTHER; note = This nucleotide is modified with Y2.
gttgcctccggttctgaaggtgttc

SEQ ID NO: 777 - RNA, 25 nt, synthetic construct
  source 1..25: mol_type = other RNA
  modified_base 1: mod_base = OTHER; note = This nucleotide is modified with Y1.
  modified_base 1..25: mod_base = OTHER; note = These nucleotides are morpholino nucleotides.
ggccaaacctcggcttacctgaaat

SEQ ID NO: 778 - RNA, 25 nt, synthetic construct
  source 1..25: mol_type = other RNA
  modified_base 1..25: mod_base = OTHER; note = These nucleotides are morpholino nucleotides.
  modified_base 1: mod_base = OTHER; note = This nucleotide is modified with Y1.
  modified_base 25: mod_base = OTHER; note = This nucleotide is modified with Y2.
ggccaaacctcggcttacctgaaat

SEQ ID NO: 779 - DNA, 25 bp, synthetic construct
  misc_feature 4: note = DNA
  source 1..25: mol_type = other DNA
  modified_base 1: mod_base = OTHER; note = This nucleotide is modified with Y3.
  misc_feature 6..10: note = DNA
  misc_feature 15..16: note = DNA
  misc_feature 22: note = DNA
  modified_base 1: mod_base = gm
  modified_base 2..3: mod_base = OTHER; note = These bases are 2-O-methyl nucleosides.
  modified_base 23..24: mod_base = OTHER; note = These bases are 2-O-methyl nucleosides.
  modified_base 25: mod_base = cm
  modified_base 1..3: mod_base = OTHER; note = These nucleotides are bound via phosphorothioate linkages.
  modified_base 22..24: mod_base = OTHER; note = These nucleotides are bound via phosphorothioate linkages.
gaacaccttcagaaccggaggcaac

SEQ ID NO: 780 - RNA, 25 nt, synthetic construct
  source 1..25: mol_type = other RNA
  modified_base 1: mod_base = OTHER; note = This nucleotide is modified with Y3.
  modified_base 1: mod_base = gm
  modified_base 2..3: mod_base = OTHER; note = These bases are 2-O-methyl nucleosides.
  modified_base 23..24: mod_base = OTHER; note = These bases are 2-O-methyl nucleosides.
  modified_base 25: mod_base = cm
  modified_base 1..3: mod_base = OTHER; note = These nucleotides are bound via phosphorothioate linkages.
  modified_base 22..24: mod_base = OTHER; note = These nucleotides are bound via phosphorothioate linkages.
gaacaccttcagaaccggaggcaac

SEQ ID NO: 781 - DNA, 25 bp, synthetic construct
  source 1..25: mol_type = other DNA
  modified_base 1: mod_base = OTHER; note = This nucleotide is modified with Y3.
  modified_base 16: mod_base = OTHER; note = This cytosine is a 5-methyle cytosine.
  modified_base 1..3: mod_base = OTHER; note = These nucleotides are bound via phosphorothioate linkages.
  modified_base 22..24: mod_base = OTHER; note = These nucleotides are bound via phosphorothioate linkages.
gaacaccttcagaaccggaggcaac

SEQ ID NO: 782 - RNA, 16 nt, synthetic construct
  source 1..16: mol_type = other RNA
  modified_base 1: mod_base = OTHER; note = This nucleotide is modified with Y3.
  modified_base 1: mod_base = gm
  modified_base 2..3: mod_base = OTHER; note = These bases are 2-O-methyl nucleosides.
  modified_base 14: mod_base = OTHER; note = Theis base is 2-O-methyl nucleoside.
  modified_base 15..16: mod_base = cm
  modified_base 1..3: mod_base = OTHER; note = These nucleotides are bound via phosphorothioate linkages.
  modified_base 13..15: mod_base = OTHER; note = These nucleotides are bound via phosphorothioate linkages.
  modified_base 1: mod_base = gm
gaacaccttcagaacc

SEQ ID NO: 783 - DNA, 25 bp, synthetic construct
  misc_feature 4..22: note = DNA
  source 1..25: mol_type = other DNA
  modified_base 1: mod_base = OTHER; note = This nucleotide is modified with Y3.
  modified_base 1: mod_base = gm
  modified_base 2..3: mod_base = OTHER; note = These bases are 2-O-methyl nucleosides.
  modified_base 23..24: mod_base = OTHER; note = These bases are 2-O-methyl nucleosides.
  modified_base 25: mod_base = cm
  modified_base 1..3: mod_base = OTHER; note = These nucleotides are bound via phosphorothioate linkages.
  modified_base 22..24: mod_base = OTHER; note = These nucleotides are bound via phosphorothioate linkages.
  modified_base 16: mod_base = OTHER; note = This cytosine is a 5-methyle cytosine.
gaacaccttcagaaccggaggcaac

SEQ ID NO: 784 - RNA, 25 nt, synthetic construct
  source 1..25: mol_type = other RNA
  modified_base 1: mod_base = OTHER; note = This nucleotide is modified with Y3.
  modified_base 1: mod_base = gm
  modified_base 2..3: mod_base = OTHER; note = These bases are 2-O-methyl nucleosides.
  modified_base 4: mod_base = cm
  modified_base 6..7: mod_base = cm
  modified_base 8..9: mod_base = um
  modified_base 10: mod_base = cm
  modified_base 15..16: mod_base = cm
  modified_base 22: mod_base = cm
  modified_base 23..24: mod_base = OTHER; note = These bases are 2-O-methyl nucleosides.
  modified_base 25: mod_base = cm
  modified_base 1..3: mod_base = OTHER; note = These nucleotides are bound via phosphorothioate linkages.
  modified_base 22..24: mod_base = OTHER; note = These nucleotides are bound via phosphorothioate linkages.
gaacaccttcagaaccggaggcaac

SEQ ID NO: 785 - DNA, 25 bp, synthetic construct
  misc_feature 4: note = DNA
  source 1..25: mol_type = other DNA
  misc_feature 6..10: note = DNA
  misc_feature 15..16: note = DNA
  misc_feature 22: note = DNA
  modified_base 1..3: mod_base = OTHER; note = These nucleosides are 2-4-BNA NC [N-Me] nucleosides.
  modified_base 23..25: mod_base = OTHER; note = These nucleosides are 2-4-BNA NC [N-Me] nucleosides.
  modified_base 1: mod_base = OTHER; note = This nucleotide is modified with Y4.
  modified_base 1..3: mod_base = OTHER; note = These nucleotides are bound via phosphorothioate linkages.
  modified_base 22..24: mod_base = OTHER; note = These nucleotides are bound via phosphorothioate linkages.
  modified_base 25: mod_base = OTHER; note = This cytosine is a 5-methyle cytosine.
gaacaccttcagaaccggaggcaac

SEQ ID NO: 786 - DNA, 25 bp, synthetic construct
  misc_feature 4: note = DNA
  source 1..25: mol_type = other DNA
  misc_feature 6..10: note = DNA
  misc_feature 15..16: note = DNA
  misc_feature 22: note = DNA
  modified_base 1..3: mod_base = OTHER; note = These nucleosides are 2-4-BNA NC [N-Me] nucleosides.
  modified_base 23..25: mod_base = OTHER; note = These nucleosides are 2-4-BNA NC [N-Me] nucleosides.
  modified_base 1: mod_base = OTHER; note = This nucleotide is modified with Y4.
  modified_base 25: mod_base = OTHER; note = This cytosine is a 5-methyle cytosine.
gaacaccttcagaaccggaggcaac

SEQ ID NO: 787 - RNA, 25 nt, synthetic construct
  source 1..25: mol_type = other RNA
  modified_base 1..3: mod_base = OTHER; note = These nucleosides are 2-4-BNA NC [N-Me] nucleosides.
  modified_base 23..25: mod_base = OTHER; note = These nucleosides are 2-4-BNA NC [N-Me] nucleosides.
  modified_base 1: mod_base = OTHER; note = This nucleotide is modified with Y4.
  modified_base 1..3: mod_base = OTHER; note = These nucleotides are bound via phosphorothioate linkages.
  modified_base 22..24: mod_base = OTHER; note = These nucleotides are bound via phosphorothioate linkages.
  modified_base 25: mod_base = OTHER; note = This cytosine is a 5-methyle cytosine.
gaacaccttcagaaccggaggcaac

SEQ ID NO: 788 - DNA, 21 bp, synthetic construct
  misc_feature 4..18: note = DNA
  source 1..21: mol_type = other DNA
  modified_base 1: mod_base = gm
  modified_base 2..3: mod_base = OTHER; note = These bases are 2-O-methyl nucleosides.
  modified_base 19: mod_base = OTHER; note = This base is a 2-O-methyl nucleoside.
  modified_base 20..21: mod_base = gm
  modified_base 1: mod_base = OTHER; note = This nucleotide is modified with Y3.
  modified_base 16: mod_base = OTHER; note = This cytosine is a 5-methyle cytosine.
  modified_base 1..3: mod_base = OTHER; note = These nucleotides are bound via phosphorothioate linkages.
  modified_base 18..20: mod_base = OTHER; note = These nucleotides are bound via phosphorothioate linkages.
gaacaccttcagaaccggagg

SEQ ID NO: 789 - DNA, 21 bp, synthetic construct
  misc_feature 4: note = DNA
  source 1..21: mol_type = other DNA
  misc_feature 6..10: note = DNA
  misc_feature 15..16: note = DNA
  modified_base 1: mod_base = gm
  modified_base 2..3: mod_base = OTHER; note = These bases are 2-O-methyl nucleosides.
  modified_base 19: mod_base = OTHER; note = This base is a 2-O-methyl nucleoside.
  modified_base 20..21: mod_base = gm
  modified_base 1: mod_base = OTHER; note = This nucleotide is modified with Y3.
  modified_base 1..3: mod_base = OTHER; note = These nucleotides are bound via phosphorothioate linkages.
  modified_base 18..20: mod_base = OTHER; note = These nucleotides are bound via phosphorothioate linkages.
gaacaccttcagaaccggagg

SEQ ID NO: 790 - RNA, 21 nt, synthetic construct
  source 1..21: mol_type = other RNA
  modified_base 1: mod_base = gm
  modified_base 2..3: mod_base = OTHER; note = These bases are 2-O-methyl nucleosides.
  modified_base 4: mod_base = cm
  modified_base 6..7: mod_base = cm
  modified_base 8..9: mod_base = um
  modified_base 10: mod_base = cm
  modified_base 15..16: mod_base = cm
  modified_base 19: mod_base = OTHER; note = This base is a 2-O-methyl nucleoside.
  modified_base 20..21: mod_base = gm
  modified_base 1: mod_base = OTHER; note = This nucleotide is modified with Y3.
  modified_base 1..3: mod_base = OTHER; note = These nucleotides are bound via phosphorothioate linkages.
  modified_base 18..20: mod_base = OTHER; note = These nucleotides are bound via phosphorothioate linkages.
gaacaccttcagaaccggagg

SEQ ID NO: 791 - DNA, 21 bp, synthetic construct
  misc_feature 5: note = DNA
  source 1..21: mol_type = other DNA
  misc_feature 11..14: note = DNA
  misc_feature 17..18: note = DNA
  modified_base 1: mod_base = gm
  modified_base 2..3: mod_base = OTHER; note = These bases are 2-O-methyl nucleosides.
  modified_base 4: mod_base = cm
  modified_base 6..7: mod_base = cm
  modified_base 8..9: mod_base = um
  modified_base 10: mod_base = cm
  modified_base 15..16: mod_base = cm
  modified_base 19: mod_base = OTHER; note = This base is a 2-O-methyl nucleoside.
  modified_base 20..21: mod_base = gm
  modified_base 1: mod_base = OTHER; note = This nucleotide is modified with Y3.
  modified_base 1..3: mod_base = OTHER; note = These nucleotides are bound via phosphorothioate linkages.
  modified_base 18..20: mod_base = OTHER; note = These nucleotides are bound via phosphorothioate linkages.
gaacaccttcagaaccggagg

SEQ ID NO: 792 - RNA, 21 nt, synthetic construct
  source 1..21: mol_type = other RNA
  modified_base 1..3: mod_base = OTHER; note = These nucleosides are 2-4-BNA NC [N-Me] nucleosides.
  modified_base 19..21: mod_base = OTHER; note = These nucleosides are 2-4-BNA NC [N-Me] nucleosides.
  modified_base 1..3: mod_base = OTHER; note = These nucleosides are 2-4-BNA NC [N-Me] nucleosides.
  modified_base 18..20: mod_base = OTHER; note = These nucleosides are 2-4-BNA NC [N-Me] nucleosides.
  modified_base 1: mod_base = OTHER; note = This nucleotide is modified with Y4.
gaacaccttcagaaccggagg

SEQ ID NO: 793 - DNA, 21 bp, synthetic construct
  misc_feature 4..18: note = DNA
  source 1..21: mol_type = other DNA
  modified_base 16: mod_base = OTHER; note = This cytosine is a 5-methyle cytosine.
  modified_base 1..3: mod_base = OTHER; note = These nucleosides are 2-4-BNA NC [N-Me] nucleosides.
  modified_base 19..21: mod_base = OTHER; note = These nucleosides are 2-4-BNA NC [N-Me] nucleosides.
  modified_base 1..3: mod_base = OTHER; note = These nucleotides are bound via phosphorothioate linkages.
  modified_base 18..20: mod_base = OTHER; note = These nucleotides are bound via phosphorothioate linkages.
  modified_base 1: mod_base = OTHER; note = This nucleotide is modified with Y4.
gaacaccttcagaaccggagg

SEQ ID NO: 794 - DNA, 16 bp, synthetic construct
  misc_feature 4: note = DNA
  source 1..16: mol_type = other DNA
  misc_feature 6..10: note = DNA
  modified_base 1: mod_base = gm
  modified_base 2..3: mod_base = OTHER; note = These bases are 2-O-methyl nucleosides.
  modified_base 14: mod_base = OTHER; note = This base is a 2-O-methyl nucleoside.
  modified_base 15..16: mod_base = cm
  modified_base 1..3: mod_base = OTHER; note = These nucleotides are bound via phosphorothioate linkages.
  modified_base 13..15: mod_base = OTHER; note = These nucleotides are bound via phosphorothioate linkages.
  modified_base 1: mod_base = OTHER; note = This nucleotide is modified with Y3.
gaacaccttcagaacc

SEQ ID NO: 795 - DNA, 16 bp, synthetic construct
  misc_feature 4..5: note = DNA
  source 1..16: mol_type = other DNA
  misc_feature 10..11: note = DNA
  modified_base 1..2: mod_base = cm
  modified_base 3: mod_base = um
  modified_base 14: mod_base = OTHER; note = This base is a 2-O-methyl nucleoside.
  modified_base 15..16: mod_base = gm
  modified_base 1: mod_base = OTHER; note = This nucleotide is modified with Y3.
  modified_base 1..3: mod_base = OTHER; note = These nucleotides are bound via phosphorothioate linkages.
  modified_base 13..15: mod_base = OTHER; note = These nucleotides are bound via phosphorothioate linkages.
ccttcagaaccggagg

SEQ ID NO: 796 - RNA, 16 nt, synthetic construct
  source 1..16: mol_type = other RNA
  modified_base 1: mod_base = OTHER; note = This nucleotide is modified with Y3.
  modified_base 1..3: mod_base = OTHER; note = These nucleotides are bound via phosphorothioate linkages.
  modified_base 13..15: mod_base = OTHER; note = These nucleotides are bound via phosphorothioate linkages.
  modified_base 1: mod_base = gm
  modified_base 2..3: mod_base = OTHER; note = These bases are 2-O-methyl nucleosides.
  modified_base 4: mod_base = cm
  modified_base 6..7: mod_base = cm
  modified_base 8..9: mod_base = um
  modified_base 10: mod_base = cm
  modified_base 14: mod_base = OTHER; note = This base is a 2-O-methyl nucleoside.
  modified_base 15..16: mod_base = cm
gaacaccttcagaacc

SEQ ID NO: 797 - RNA, 16 nt, synthetic construct
  source 1..16: mol_type = other RNA
  modified_base 1..2: mod_base = cm
  modified_base 3..4: mod_base = um
  modified_base 5: mod_base = cm
  modified_base 10..11: mod_base = cm
  modified_base 14: mod_base = OTHER; note = This base is a 2-O-methyl nucleoside.
  modified_base 15..16: mod_base = gm
  modified_base 1..3: mod_base = OTHER; note = These nucleotides are bound via phosphorothioate linkages.
  modified_base 13..15: mod_base = OTHER; note = These nucleotides are bound via phosphorothioate linkages.
ccttcagaaccggagg

SEQ ID NO: 798 - RNA, 16 nt, synthetic construct
  source 1..16: mol_type = other RNA
  modified_base 1: mod_base = cm
  modified_base 2: mod_base = OTHER; note = This base is a 2-O-methyl nucleoside.
  modified_base 3: mod_base = gm
  modified_base 6..7: mod_base = cm
  modified_base 13: mod_base = cm
  modified_base 14..15: mod_base = OTHER; note = These bases are 2-O-methyl nucleosides.
  modified_base 16: mod_base = cm
  modified_base 1..3: mod_base = OTHER; note = These nucleotides are bound via phosphorothioate linkages.
  modified_base 13..15: mod_base = OTHER; note = These nucleotides are bound via phosphorothioate linkages.
  modified_base 1: mod_base = OTHER; note = This nucleotide is modified with Y3.
cagaaccggaggcaac

SEQ ID NO: 799 - DNA, 16 bp, synthetic construct
  misc_feature 5: note = DNA
  source 1..16: mol_type = other DNA
  misc_feature 11..13: note = DNA
  modified_base 1: mod_base = gm
  modified_base 2..3: mod_base = OTHER; note = These bases are 2-O-methyl nucleosides.
  modified_base 4: mod_base = cm
  modified_base 6..7: mod_base = cm
  modified_base 8..9: mod_base = um
  modified_base 10: mod_base = cm
  modified_base 14: mod_base = OTHER; note = This base is a 2-O-methyl nucleoside.
  modified_base 15..16: mod_base = cm
  modified_base 1..3: mod_base = OTHER; note = These nucleotides are bound via phosphorothioate linkages.
  modified_base 13..15: mod_base = OTHER; note = These nucleotides are bound via phosphorothioate linkages.
  modified_base 1: mod_base = OTHER; note = This nucleotide is modified with Y3.
gaacaccttcagaacc

SEQ ID NO: 800 - DNA, 16 bp, synthetic construct
  misc_feature 4: note = DNA
  source 1..16: mol_type = other DNA
  misc_feature 6: note = DNA
  misc_feature 8: note = DNA
  misc_feature 10..13: note = DNA
  modified_base 1: mod_base = gm
  modified_base 2..3: mod_base = OTHER; note = These bases are 2-O-methyl nucleosides.
  modified_base 14: mod_base = OTHER; note = This base is a 2-O-methyl nucleoside.
  modified_base 15..16: mod_base = cm
  modified_base 1..3: mod_base = OTHER; note = These nucleotides are bound via phosphorothioate linkages.
  modified_base 13..15: mod_base = OTHER; note = These nucleotides are bound via phosphorothioate linkages.
  modified_base 1: mod_base = OTHER; note = This nucleotide is modified with Y3.
  modified_base 9: mod_base = OTHER; note = This t is uracil.
gaacaccttcagaacc

SEQ ID NO: 801 - DNA, 16 bp, synthetic construct
  misc_feature 4..5: note = DNA
  source 1..16: mol_type = other DNA
  misc_feature 8: note = DNA
  misc_feature 10..13: note = DNA
  modified_base 1: mod_base = gm
  modified_base 2..3: mod_base = OTHER; note = These bases are 2-O-methyl nucleosides.
  modified_base 7: mod_base = cm
  modified_base 14: mod_base = OTHER; note = This base is a 2-O-methyl nucleoside.
  modified_base 15..16: mod_base = cm
  modified_base 1..3: mod_base = OTHER; note = These nucleotides are bound via phosphorothioate linkages.
  modified_base 13..15: mod_base = OTHER; note = These nucleotides are bound via phosphorothioate linkages.
  modified_base 1: mod_base = OTHER; note = This nucleotide is modified with Y3.
  modified_base 9: mod_base = OTHER; note = This t is uracil.
gaacaccttcagaacc

SEQ ID NO: 802 - RNA, 16 nt, synthetic construct
  source 1..16: mol_type = other RNA
  modified_base 1..3: mod_base = OTHER; note = These nucleosides are 2-4-BNA NC [N-Me] nucleosides.
  modified_base 14..16: mod_base = OTHER; note = These nucleosides are 2-4-BNA NC [N-Me] nucleosides.
  modified_base 1..3: mod_base = OTHER; note = These nucleotides are bound via phosphorothioate linkages.
  modified_base 13..15: mod_base = OTHER; note = These nucleotides are bound via phosphorothioate linkages.
  modified_base 15..16: mod_base = OTHER; note = These cytosines are 5-methyle cytosines.
  modified_base 1: mod_base = OTHER; note = This nucleotide is modified with Y3.
gaacaccttcagaacc

SEQ ID NO: 803 - DNA, 16 bp, synthetic construct
  misc_feature 4: note = DNA
  source 1..16: mol_type = other DNA
  misc_feature 6..10: note = DNA
  modified_base 1..3: mod_base = OTHER; note = These nucleosides are 2-4-BNA NC [N-Me] nucleosides.
  modified_base 14..16: mod_base = OTHER; note = These nucleosides are 2-4-BNA NC [N-Me] nucleosides.
  modified_base 1..3: mod_base = OTHER; note = These nucleotides are bound via phosphorothioate linkages.
  modified_base 13..15: mod_base = OTHER; note = These nucleotides are bound via phosphorothioate linkages.
  modified_base 1: mod_base = OTHER; note = This nucleotide is modified with Y3.
  modified_base 15..16: mod_base = OTHER; note = These cytosines are 5-methyl cytosines.
gaacaccttcagaacc

SEQ ID NO: 804 - DNA, 16 bp, synthetic construct
  misc_feature 4..5: note = DNA
  source 1..16: mol_type = other DNA
  misc_feature 8: note = DNA
  misc_feature 10..13: note = DNA
  modified_base 1..3: mod_base = OTHER; note = These nucleosides are 2-4-BNA NC [N-Me] nucleosides.
  modified_base 14..16: mod_base = OTHER; note = These nucleosides are 2-4-BNA NC [N-Me] nucleosides.
  modified_base 1..3: mod_base = OTHER; note = These nucleotides are bound via phosphorothioate linkages.
  modified_base 13..15: mod_base = OTHER; note = These nucleotides are bound via phosphorothioate linkages.
  modified_base 7: mod_base = cm
  modified_base 9: mod_base = OTHER; note = This t is uracil.
  modified_base 15..16: mod_base = OTHER; note = These cytosines are 5-methyle cytosines.
  modified_base 1: mod_base = OTHER; note = This nucleotide is modified with Y3.
gaacaccttcagaacc

SEQ ID NO: 805 - DNA, 19 bp, synthetic construct
  misc_feature 9..11: note = DNA
  source 1..19: mol_type = other DNA
  modified_base 1: mod_base = gm
  modified_base 2..3: mod_base = OTHER; note = These bases are 2-O-methyl nucleosides.
  modified_base 4: mod_base = cm
  modified_base 5: mod_base = OTHER; note = This base is a 2-O-methyl nucleoside.
  modified_base 6..7: mod_base = cm
  modified_base 8: mod_base = um
  modified_base 12: mod_base = um
  modified_base 13: mod_base = cm
  modified_base 14: mod_base = OTHER; note = This base is a 2-O-methyl nucleoside.
  modified_base 15: mod_base = gm
  modified_base 16..17: mod_base = OTHER; note = These bases are 2-O-methyl nucleosides.
  modified_base 18..19: mod_base = cm
  modified_base 1..3: mod_base = OTHER; note = These nucleotides are bound via phosphorothioate linkages.
  modified_base 16..18: mod_base = OTHER; note = These nucleotides are bound via phosphorothioate linkages.
  modified_base 1: mod_base = OTHER; note = This nucleotide is modified with Y3.
gaacacctaaatcagaacc

SEQ ID NO: 806 - DNA, 25 bp, synthetic construct
  misc_feature 7..9: note = DNA
  source 1..25: mol_type = other DNA
  misc_feature 17..19: note = DNA
  modified_base 1: mod_base = gm
  modified_base 2..3: mod_base = OTHER; note = These bases are 2-O-methyl nucleosides.
  modified_base 4: mod_base = cm
  modified_base 5: mod_base = OTHER; note = This base is a 2-O-methyl nucleoside.
  modified_base 6: mod_base = cm
  modified_base 10..11: mod_base = um
  modified_base 12: mod_base = cm
  modified_base 13: mod_base = OTHER; note = This base is a 2-O-methyl nucleoside.
  modified_base 14: mod_base = gm
  modified_base 15..16: mod_base = OTHER; note = These bases are 2-O-methyl nucleosides.
  modified_base 20: mod_base = cm
  modified_base 21..22: mod_base = gm
  modified_base 23: mod_base = OTHER; note = This base is a 2-O-methyl nucleoside.
  modified_base 24..25: mod_base = gm
  modified_base 1..3: mod_base = OTHER; note = These nucleotides are bound via phosphorothioate linkages.
  modified_base 22..24: mod_base = OTHER; note = These nucleotides are bound via phosphorothioate linkages.
  modified_base 1: mod_base = OTHER; note = This nucleotide is modified with Y3.
gaacacaaattcagaaaaacggagg

SEQ ID NO: 807 - DNA, 16 bp, synthetic construct
  misc_feature 4: note = DNA
  source 1..16: mol_type = other DNA
  misc_feature 6..10: note = DNA
  modified_base 1: mod_base = gm
  modified_base 2..3: mod_base = OTHER; note = These bases are 2-O-methyl nucleosides.
  modified_base 14: mod_base = OTHER; note = This base is a 2-O-methyl nucleoside.
  modified_base 15..16: mod_base = cm
  modified_base 1..3: mod_base = OTHER; note = These nucleotides are bound via phosphorothioate linkages.
  modified_base 13..15: mod_base = OTHER; note = These nucleotides are bound via phosphorothioate linkages.
  modified_base 1: mod_base = OTHER; note = This nucleotide is modified with Y5.
  modified_base 16: mod_base = OTHER; note = This nucleotide is modified with Y3.
gaacaccttcagaacc

SEQ ID NO: 808 - DNA, 19 bp, synthetic construct
  misc_feature 1..3: note = DNA
  source 1..19: mol_type = other DNA
  misc_feature 7: note = DNA
  misc_feature 9..13: note = DNA
  modified_base 17: mod_base = OTHER; note = This base is a 2-O-methyl nucleoside.
  modified_base 18..19: mod_base = cm
  modified_base 16..18: mod_base = OTHER; note = These nucleotides are bound via phosphorothioate linkages.
  modified_base 1: mod_base = OTHER; note = This nucleotide is modified with Y3.
tcagaacaccttcagaacc

SEQ ID NO: 809 - DNA, 25 bp, synthetic construct
  misc_feature 4: note = DNA
  source 1..25: mol_type = other DNA
  misc_feature 6..10: note = DNA
  misc_feature 15..16: note = DNA
  misc_feature 22: note = DNA
  modified_base 1: mod_base = gm
  modified_base 25: mod_base = cm
  modified_base 1: mod_base = OTHER; note = This nucleotide is bound via a phosphorothioate linkage.
  modified_base 24: mod_base = OTHER; note = This nucleotide is bound via a phosphorothioate linkage.
  modified_base 1: mod_base = OTHER; note = This nucleotide is modified with Y3.
gaacaccttcagaaccggaggcaac

SEQ ID NO: 810 - DNA, 16 bp, synthetic construct
  source 1..16: mol_type = other DNA
  modified_base 1: mod_base = OTHER; note = This nucleotide is modified with Y3.
gaacaccttcagaacc

SEQ ID NO: 811 - DNA, 25 bp, synthetic construct
  source 1..25: mol_type = other DNA
  modified_base 1: mod_base = OTHER; note = This nucleotide is modified with Y3.
  modified_base 16: mod_base = OTHER; note = This cytosine is a 5-methyle cytosine.
gaacaccttcagaaccggaggcaac

SEQ ID NO: 812 - DNA, 21 bp, synthetic construct
  source 1..21: mol_type = other DNA
  modified_base 16: mod_base = OTHER; note = This cytosine is a 5-methyle cytosine.
  modified_base 1: mod_base = OTHER; note = This nucleotide is modified with Y3
gaacaccttcagaaccggagg

SEQ ID NO: 813 - RNA, 21 nt, synthetic construct
  source 1..21: mol_type = other RNA
  modified_base 1: mod_base = gm
  modified_base 2..3: mod_base = OTHER; note = These bases are 2-O-methyl nucleosides.
  modified_base 19: mod_base = OTHER; note = This base is a 2-O-methyl nucleoside.
  modified_base 20..21: mod_base = gm
  modified_base 1..3: mod_base = OTHER; note = These nucleotides are bound via phosphorothioate linkages.
  modified_base 18..20: mod_base = OTHER; note = These nucleotides are bound via phosphorothioate linkages.
  modified_base 1: mod_base = OTHER; note = This nucleotide is modified with Y6.
gaacaccttcagaaccggagg

SEQ ID NO: 814 - RNA, 25 nt, synthetic construct
  source 1..25: mol_type = other RNA
  modified_base 1: mod_base = OTHER; note = This base is a 2-O-methyl nucleoside.
  modified_base 2..3: mod_base = um
  modified_base 23: mod_base = gm
  modified_base 24..25: mod_base = cm
  modified_base 1..3: mod_base = OTHER; note = These nucleotides are bound via phosphorothioate linkages.
  modified_base 22..24: mod_base = OTHER; note = These nucleotides are bound via phosphorothioate linkages.
  modified_base 1: mod_base = OTHER; note = This nucleotide is modified with Y3.
atttcaggtaagccgaggtttggcc

SEQ ID NO: 815 - RNA, 16 nt, synthetic construct
  source 1..16: mol_type = other RNA
  modified_base 1: mod_base = OTHER; note = This base is a 2-O-methyl nucleoside.
  modified_base 2..3: mod_base = um
  modified_base 14: mod_base = cm
  modified_base 16: mod_base = OTHER; note = This base is a 2-O-methyl nucleoside.
  modified_base 15: mod_base = gm
  modified_base 1..3: mod_base = OTHER; note = These nucleotides are bound via phosphorothioate linkages.
  modified_base 13..15: mod_base = OTHER; note = These nucleotides are bound via phosphorothioate linkages.
  modified_base 1: mod_base = OTHER; note = This nucleotide is modified with Y3.
atttcaggtaagccga

SEQ ID NO: 816 - DNA, 25 bp, synthetic construct
  misc_feature 4..5: note = DNA
  source 1..25: mol_type = other DNA
  misc_feature 9: note = DNA
  misc_feature 13..14: note = DNA
  misc_feature 19..21: note = DNA
  modified_base 1: mod_base = OTHER; note = This base is a 2-O-methyl nucleoside.
  modified_base 2..3: mod_base = um
  modified_base 23: mod_base = gm
  modified_base 24..25: mod_base = cm
  modified_base 1..3: mod_base = OTHER; note = These nucleotides are bound via phosphorothioate linkages.
  modified_base 22..24: mod_base = OTHER; note = These nucleotides are bound via phosphorothioate linkages.
  modified_base 1: mod_base = OTHER; note = This nucleotide is modified with Y3.
atttcaggtaagccgaggtttggcc

SEQ ID NO: 817 - DNA, 16 bp, synthetic construct
  misc_feature 4..5: note = DNA
  source 1..16: mol_type = other DNA
  misc_feature 9: note = DNA
  misc_feature 13: note = DNA
  modified_base 1: mod_base = OTHER; note = This base is a 2-O-methyl nucleoside.
  modified_base 2..3: mod_base = um
  modified_base 14: mod_base = cm
  modified_base 15: mod_base = gm
  modified_base 16: mod_base = OTHER; note = This base is a 2-O-methyl nucleoside.
  modified_base 1..3: mod_base = OTHER; note = These nucleotides are bound via phosphorothioate linkages.
  modified_base 13..15: mod_base = OTHER; note = These nucleotides are bound via phosphorothioate linkages.
  modified_base 1: mod_base = OTHER; note = This nucleotide is modified with Y3.
atttcaggtaagccga

SEQ ID NO: 818 - DNA, 25 bp, synthetic construct
  misc_feature 7..9: note = DNA
  source 1..25: mol_type = other DNA
  misc_feature 17..18: note = DNA
  modified_base 1: mod_base = OTHER; note = This base is a 2-O-methyl nucleoside.
  modified_base 2..4: mod_base = um
  modified_base 5: mod_base = cm
  modified_base 10: mod_base = gm
  modified_base 6: mod_base = OTHER; note = This base is a 2-O-methyl nucleoside.
  modified_base 11: mod_base = um
  modified_base 12..13: mod_base = OTHER; note = These bases are 2-O-methyl nucleosides.
  modified_base 14: mod_base = gm
  modified_base 15..16: mod_base = cm
  modified_base 20: mod_base = OTHER; note = This base is a 2-O-methyl nucleoside.
  modified_base 21..22: mod_base = gm
  modified_base 23..25: mod_base = um
  modified_base 1..3: mod_base = OTHER; note = These nucleotides are bound via phosphorothioate linkages.
  modified_base 22..24: mod_base = OTHER; note = These nucleotides are bound via phosphorothioate linkages.
  modified_base 1: mod_base = OTHER; note = This nucleotide is modified with Y3.
atttcaaaagtaagccaaaaggttt

SEQ ID NO: 819 - DNA, 16 bp, synthetic construct
  misc_feature 4..5: note = DNA
  source 1..16: mol_type = other DNA
  misc_feature 9: note = DNA
  misc_feature 13: note = DNA
  modified_base 1: mod_base = OTHER; note = This base is a 2-O-methyl nucleoside.
  modified_base 2..3: mod_base = um
  modified_base 14: mod_base = cm
  modified_base 15: mod_base = gm
  modified_base 16: mod_base = OTHER; note = This base is a 2-O-methyl nucleoside.
  modified_base 1..3: mod_base = OTHER; note = These nucleotides are bound via phosphorothioate linkages.
  modified_base 13..15: mod_base = OTHER; note = These nucleotides are bound via phosphorothioate linkages.
  modified_base 1: mod_base = OTHER; note = This nucleotide is modified with Y5.
  modified_base 16: mod_base = OTHER; note = This nucleotide is modified with Y3.
atttcaggtaagccga

SEQ ID NO: 820 - DNA, 16 bp, synthetic construct
  misc_feature 4..5: note = DNA
  source 1..16: mol_type = other DNA
  misc_feature 9: note = DNA
  misc_feature 13: note = DNA
  modified_base 1..3: mod_base = OTHER; note = These nucleosides are 2-4-BNA NC [N-Me] nucleosides.
  modified_base 14..16: mod_base = OTHER; note = These nucleosides are 2-4-BNA NC [N-Me] nucleosides.
  modified_base 14: mod_base = OTHER; note = This cytosine is a 5-methyle cytosine.
  modified_base 1..3: mod_base = OTHER; note = These nucleotides are bound via phosphorothioate linkages.
  modified_base 13..15: mod_base = OTHER; note = These nucleotides are bound via phosphorothioate linkages.
  modified_base 1: mod_base = OTHER; note = This nucleotide is modified with Y3.
atttcaggtaagccga

SEQ ID NO: 821 - DNA, 25 bp, synthetic construct
  source 1..25: mol_type = other DNA
  modified_base 1: mod_base = OTHER; note = This nucleotide is modified with Y3.
  modified_base 14: mod_base = OTHER; note = This cytosine is a 5-methyle cytosine.
atttcaggtaagccgaggtttggcc

SEQ ID NO: 822 - DNA, 25 bp, synthetic construct
  misc_feature 4: note = DNA
  source 1..25: mol_type = other DNA
  misc_feature 6..10: note = DNA
  misc_feature 15..16: note = DNA
  misc_feature 22: note = DNA
  modified_base 1..3: mod_base = OTHER; note = These nucleotides are bound via phosphorothioate linkages.
  modified_base 22..24: mod_base = OTHER; note = These nucleotides are bound via phosphorothioate linkages.
  modified_base 1: mod_base = OTHER; mod_base = gm; note = This nucleotide is modified with Y6.
  modified_base 2..3: mod_base = OTHER; note = These bases are 2-O-methyl nucleosides.
  modified_base 23..24: mod_base = OTHER; note = These bases are 2-O-methyl nucleosides.
  modified_base 25: mod_base = cm
gaacaccttcagaaccggaggcaac

SEQ ID NO: 823 - RNA, 25 nt, synthetic construct
  source 1..25: mol_type = other RNA
  modified_base 1..3: mod_base = OTHER; note = These nucleotides are bound via phosphorothioate linkages.
  modified_base 23..24: mod_base = OTHER; note = These nucleotides are bound via phosphorothioate linkages.
  modified_base 1: mod_base = gm; mod_base = OTHER; note = This nucleotide is modified with Y6.
  modified_base 2..3: mod_base = OTHER; note = These bases are 2-O-methyl nucleosides.
  modified_base 22..24: mod_base = OTHER; note = These bases are 2-O-methyl nucleosides.
  modified_base 25: mod_base = cm
gaacaccttcagaaccggaggcaac

SEQ ID NO: 824 - DNA, 25 bp, synthetic construct
  source 1..25: mol_type = other DNA
  modified_base 22..24: mod_base = OTHER; note = These nucleotides are bound via phosphorothioate linkages.
  modified_base 1..3: mod_base = OTHER; note = These nucleotides are bound via phosphorothioate linkages.
  modified_base 1: mod_base = OTHER; note = This nucleotide is modified with Y6.
  modified_base 16: mod_base = OTHER; note = This cytosine is a 5-methyle cytosine.
gaacaccttcagaaccggaggcaac

SEQ ID NO: 825 - RNA, 16 nt, synthetic construct
  source 1..16: mol_type = other RNA
  modified_base 1..3: mod_base = OTHER; note = These nucleotides are bound via phosphorothioate linkages.
  modified_base 13..15: mod_base = OTHER; note = These nucleotides are bound via phosphorothioate linkages.
  modified_base 1: mod_base = gm; mod_base = OTHER; note = This nucleotide is modified with Y6.
  modified_base 2..3: mod_base = OTHER; note = These bases are 2-O-methyl nucleosides.
  modified_base 14: mod_base = OTHER; note = These bases are 2-O-methyl nucleosides.
  modified_base 15..16: mod_base = cm
gaacaccttcagaacc

SEQ ID NO: 826 - DNA, 25 bp, synthetic construct
  misc_feature 4..22: note = DNA
  source 1..25: mol_type = other DNA
  modified_base 1..3: mod_base = OTHER; note = These nucleotides are bound via phosphorothioate linkages.
  modified_base 22..24: mod_base = OTHER; note = These nucleotides are bound via phosphorothioate linkages.
  modified_base 1: mod_base = gm; mod_base = OTHER; note = This nucleotide is modified with Y6.
  modified_base 2..3: mod_base = OTHER; note = These bases are 2-O-methyl nucleosides.
  modified_base 23..24: mod_base = OTHER; note = These bases are 2-O-methyl nucleosides.
  modified_base 25: mod_base = cm
gaacaccttcagaaccggaggcaac

SEQ ID NO: 827 - RNA, 25 nt, synthetic construct
  source 1..25: mol_type = other RNA
  modified_base 1..3: mod_base = OTHER; note = These nucleotides are bound via phosphorothioate linkages.
  modified_base 22..24: mod_base = OTHER; note = These nucleotides are bound via phosphorothioate linkages.
  modified_base 1: mod_base = OTHER; mod_base = gm; note = This nucleotide is modified with Y6.
  modified_base 2..3: mod_base = OTHER; note = These bases are 2-O-methyl nucleosides.
  modified_base 4: mod_base = cm
  modified_base 6..7: mod_base = cm
  modified_base 8..9: mod_base = um
  modified_base 10: mod_base = cm
  modified_base 15..16: mod_base = cm
  modified_base 22: mod_base = cm
  modified_base 23..24: mod_base = OTHER; note = These bases are 2-O-methyl nucleosides.
  modified_base 25: mod_base = cm
gaacaccttcagaaccggaggcaac

SEQ ID NO: 828 - DNA, 25 bp, synthetic construct
  misc_feature 4: note = DNA
  source 1..25: mol_type = other DNA
  misc_feature 6..10: note = DNA
  misc_feature 15..16: note = DNA
  misc_feature 22: note = DNA
  modified_base 1..3: mod_base = OTHER; note = These nucleotides are bound via phosphorothioate linkages. These nucleosides are 2-4-BNA NC [N-Me] nucleosides.
  modified_base 22..24: mod_base = OTHER; note = These nucleotides are bound via phosphorothioate linkages.
  modified_base 23..25: mod_base = OTHER; note = These nucleosides are 2-4-BNA NC [N-Me] nucleosides.
gaacaccttcagaaccggaggcaac

SEQ ID NO: 829 - DNA, 25 bp, synthetic construct
  misc_feature 4: note = DNA
  source 1..25: mol_type = other DNA
  misc_feature 6..10: note = DNA
  misc_feature 15..16: note = DNA
  misc_feature 22: note = DNA
  modified_base 1..3: mod_base = OTHER; note = These nucleosides are 2-4-BNA NC [N-Me] nucleosides.
  modified_base 23..25: mod_base = OTHER; note = These nucleosides are 2-4-BNA NC [N-Me] nucleosides.
  modified_base 1: mod_base = OTHER; note = This nucleotide is modified with Y6.
gaacaccttcagaaccggaggcaac

SEQ ID NO: 830 - RNA, 25 nt, synthetic construct
  source 1..25: mol_type = other RNA
  modified_base 1..3: mod_base = OTHER; note = These nucleotides are bound via phosphorothioate linkages. These nucleosides are 2-4-BNA NC [N-Me] nucleosides.
  modified_base 22..24: mod_base = OTHER; note = These nucleotides are bound via phosphorothioate linkages.
  modified_base 23..25: mod_base = OTHER; note = These nucleosides are 2-4-BNA NC [N-Me] nucleosides.
  modified_base 1: mod_base = OTHER; note = This nucleotide is modified with Y1.
gaacaccttcagaaccggaggcaac

SEQ ID NO: 831 - DNA, 21 bp, synthetic construct
  misc_feature 4..18: note = DNA
  source 1..21: mol_type = other DNA
  modified_base 1..3: mod_base = OTHER; note = These nucleotides are bound via phosphorothioate linkages.
  modified_base 18..20: mod_base = OTHER; note = These nucleotides are bound via phosphorothioate linkages.
  modified_base 1: mod_base = OTHER; mod_base = gm; note = This nucleotide is modified with Y6.
  modified_base 2..3: mod_base = OTHER; note = These bases are 2-O-methyl nucleosides.
  modified_base 19: mod_base = OTHER; note = This base is a 2-O-methyl nucleoside.
  modified_base 20..21: mod_base = gm
  modified_base 16: mod_base = OTHER; note = This cytosine is a 5-methyle cytosine.
gaacaccttcagaaccggagg

SEQ ID NO: 832 - DNA, 21 bp, synthetic construct
  misc_feature 4: note = DNA
  source 1..21: mol_type = other DNA
  misc_feature 6..10: note = DNA
  misc_feature 15..16: note = DNA
  modified_base 1..3: mod_base = OTHER; note = These nucleotides are bound via phosphorothioate linkages.
  modified_base 18..20: mod_base = OTHER; note = These nucleotides are bound via phosphorothioate linkages.
  modified_base 1: mod_base = gm; mod_base = OTHER; note = This nucleotide is modified with Y6.
  modified_base 2..3: mod_base = OTHER; note = These bases are 2-O-methyl nucleosides.
  modified_base 19: mod_base = OTHER; note = These bases are 2-O-methyl nucleosides.
  modified_base 20..21: mod_base = gm
gaacaccttcagaaccggagg

SEQ ID NO: 833 - RNA, 21 nt, synthetic construct
  source 1..21: mol_type = other RNA
  modified_base 1..3: mod_base = OTHER; note = These nucleotides are bound via phosphorothioate linkages.
  modified_base 18..20: mod_base = OTHER; note = These nucleotides are bound via phosphorothioate linkages.
  modified_base 1: mod_base = gm; mod_base = OTHER; note = This nucleotide is modified with Y6.
  modified_base 2..3: mod_base = OTHER; note = These bases are 2-O-methyl nucleosides.
  modified_base 4: mod_base = cm
  modified_base 6..7: mod_base = cm
  modified_base 8..9: mod_base = um
  modified_base 10: mod_base = cm
  modified_base 15..16: mod_base = cm
  modified_base 19: mod_base = OTHER; note = This base is a 2-O-methyl nucleoside.
  modified_base 20..21: mod_base = gm
gaacaccttcagaaccggagg

SEQ ID NO: 834 - DNA, 21 bp, synthetic construct
  misc_feature 5: note = DNA
  source 1..21: mol_type = other DNA
  misc_feature 11..14: note = DNA
  misc_feature 17..18: note = DNA
  modified_base 1..3: mod_base = OTHER; note = These nucleotides are bound via phosphorothioate linkages.
  modified_base 18..20: mod_base = OTHER; note = These nucleotides are bound via phosphorothioate linkages.
  modified_base 1: mod_base = gm; mod_base = OTHER; note = This nucleotide is modified with Y6.
  modified_base 2..3: mod_base = OTHER; note = These bases are 2-O-methyl nucleosides.
  modified_base 4: mod_base = cm
  modified_base 6..7: mod_base = cm
  modified_base 8..9: mod_base = um
  modified_base 10: mod_base = cm
  modified_base 15..16: mod_base = cm
  modified_base 10: mod_base = cm
  modified_base 15..16: mod_base = cm
  modified_base 19: mod_base = OTHER; note = This base is a 2-O-methyl nucleoside.
  modified_base 20..21: mod_base = gm
gaacaccttcagaaccggagg

SEQ ID NO: 835 - RNA, 21 nt, synthetic construct
  source 1..21: mol_type = other RNA
  modified_base 1..3: mod_base = OTHER; note = These nucleotides are bound via phosphorothioate linkages. These nucleosides are 2-4-BNA NC [N-Me] nucleosides.
  modified_base 18..20: mod_base = OTHER; note = These nucleotides are bound via phosphorothioate linkages.
  modified_base 19..21: mod_base = OTHER; note = These nucleosides are 2-4-BNA NC [N-Me] nucleosides.
  modified_base 1: mod_base = OTHER; note = This nucleotide is modified with Y6.
gaacaccttcagaaccggagg

SEQ ID NO: 836 - DNA, 21 bp, synthetic construct
  misc_feature 4..18: note = DNA
  source 1..21: mol_type = other DNA
  modified_base 1..3: mod_base = OTHER; note = These nucleotides are bound via phosphorothioate linkages. These nucleosides are 2-4-BNA NC [N-Me] nucleosides.
  modified_base 18..20: mod_base = OTHER; note = These nucleotides are bound via phosphorothioate linkages.
  modified_base 19..21: mod_base = OTHER; note = These nucleosides are 2-4-BNA NC [N-Me] nucleosides.
  modified_base 16: mod_base = OTHER; note = This cytosine is a 5-methyle cytosine.
  modified_base 1: mod_base = OTHER; note = This nucleotide is modified with Y6.
gaacaccttcagaaccggagg

SEQ ID NO: 837 - DNA, 16 bp, synthetic construct
  misc_feature 4: note = DNA
  source 1..16: mol_type = other DNA
  misc_feature 6..10: note = DNA
  modified_base 1..3: mod_base = OTHER; note = These nucleotides are bound via phosphorothioate linkages.
  modified_base 13..15: mod_base = OTHER; note = These nucleotides are bound via phosphorothioate linkages.
  modified_base 1: mod_base = gm; mod_base = OTHER; note = This nucleotide is modified with Y6.
  modified_base 2..3: mod_base = OTHER; note = These bases are 2-O-methyl nucleosides.
  modified_base 14: mod_base = OTHER; note = This base is a 2-O-methyl nucleoside.
  modified_base 15..16: mod_base = cm
gaacaccttcagaacc

SEQ ID NO: 838 - DNA, 16 bp, synthetic construct
  misc_feature 4..5: note = DNA
  source 1..16: mol_type = other DNA
  misc_feature 10..11: note = DNA
  modified_base 1..3: mod_base = OTHER; note = These nucleotides are bound via phosphorothioate linkages.
  modified_base 13..15: mod_base = OTHER; note = These nucleotides are bound via phosphorothioate linkages.
  modified_base 1: mod_base = OTHER; mod_base = cm; note = This nucleotide is modified with Y6.
  modified_base 2: mod_base = cm
  modified_base 3: mod_base = um
  modified_base 14: mod_base = OTHER; note = This base is a 2-O-methyl nucleoside.
  modified_base 15..16: mod_base = gm
ccttcagaaccggagg

SEQ ID NO: 839 - RNA, 16 nt, synthetic construct
  source 1..16: mol_type = other RNA
  modified_base 1..3: mod_base = OTHER; note = These nucleotides are bound via phosphorothioate linkages.
  modified_base 13..15: mod_base = OTHER; note = These nucleotides are bound via phosphorothioate linkages.
  modified_base 1: mod_base = OTHER; mod_base = gm; note = This nucleotide is modified with Y6.
  modified_base 2..3: mod_base = OTHER; note = These bases are 2-O-methyl nucleosides.
  modified_base 4: mod_base = cm
  modified_base 6..7: mod_base = cm
  modified_base 8..9: mod_base = um
  modified_base 10: mod_base = cm
  modified_base 14: mod_base = OTHER; note = This base is a 2-O-methyl nucleoside.
  modified_base 15..16: mod_base = cm
gaacaccttcagaacc

SEQ ID NO: 840 - RNA, 16 nt, synthetic construct
  source 1..16: mol_type = other RNA
  modified_base 1..3: mod_base = OTHER; note = These nucleotides are bound via phosphorothioate linkages.
  modified_base 13..15: mod_base = OTHER; note = These nucleotides are bound via phosphorothioate linkages.
  modified_base 1: mod_base = cm; mod_base = OTHER; note = This nucleotide is modified with Y6.
  modified_base 2: mod_base = cm
  modified_base 3..4: mod_base = um
  modified_base 5: mod_base = cm
  modified_base 10..11: mod_base = cm
  modified_base 14: mod_base = OTHER; note = This base is a 2-O-methyl nucleoside.
  modified_base 15..16: mod_base = gm
ccttcagaaccggagg

SEQ ID NO: 841 - RNA, 16 nt, synthetic construct
  source 1..16: mol_type = other RNA
  modified_base 1..3: mod_base = OTHER; note = These nucleotides are bound via phosphorothioate linkages.
  modified_base 13..15: mod_base = OTHER; note = These nucleotides are bound via phosphorothioate linkages.
  modified_base 1: mod_base = OTHER; mod_base = cm; note = This nucleotide is modified with Y6.
  modified_base 2: mod_base = OTHER; note = This base is a 2-O-methyl nucleoside.
  modified_base 3: mod_base = gm
  modified_base 6..7: mod_base = cm
  modified_base 13: mod_base = cm
  modified_base 14..15: mod_base = OTHER; note = These bases are 2-O-methyl nucleosides.
  modified_base 16: mod_base = cm
cagaaccggaggcaac

SEQ ID NO: 842 - DNA, 16 bp, synthetic construct
  misc_feature 5: note = DNA
  source 1..16: mol_type = other DNA
  misc_feature 11..13: note = DNA
  modified_base 1..3: mod_base = OTHER; note = These nucleotides are bound via phosphorothioate linkages.
  modified_base 13..15: mod_base = OTHER; note = These nucleotides are bound via phosphorothioate linkages.
  modified_base 1: mod_base = OTHER; mod_base = gm; note = This nucleotide is modified with Y6.
  modified_base 2..3: mod_base = OTHER; note = These bases are 2-O-methyl nucleosides.
  modified_base 4: mod_base = cm
  modified_base 6..7: mod_base = cm
  modified_base 8..9: mod_base = um
  modified_base 10: mod_base = cm
  modified_base 14: mod_base = OTHER; note = This base is a 2-O-methyl nucleoside.
  modified_base 15..16: mod_base = cm
gaacaccttcagaacc

SEQ ID NO: 843 - DNA, 16 bp, synthetic construct
  misc_feature 4: note = DNA
  source 1..16: mol_type = other DNA
  misc_feature 6: note = DNA
  misc_feature 10..13: note = DNA
  modified_base 1..3: mod_base = OTHER; note = These nucleotides are bound via phosphorothioate linkages.
  modified_base 13..15: mod_base = OTHER; note = These nucleotides are bound via phosphorothioate linkages.
  modified_base 1: mod_base = OTHER; mod_base = gm; note = This nucleotide is modified with Y6.
  modified_base 2..3: mod_base = OTHER; note = These bases are 2-O-methyl nucleosides.
  modified_base 14: mod_base = OTHER; note = This base is a 2-O-methyl nucleoside.
  modified_base 15..16: mod_base = cm
  misc_feature 8: note = DNA
gaacaccttcagaacc

SEQ ID NO: 844 - DNA, 16 bp, synthetic construct
  misc_feature 4..5: note = DNA
  source 1..16: mol_type = other DNA
  misc_feature 8: note = DNA
  misc_feature 10..13: note = DNA
  modified_base 1..3: mod_base = OTHER; note = These nucleotides are bound via phosphorothioate linkages.
  modified_base 13..15: mod_base = OTHER; note = These nucleotides are bound via phosphorothioate linkages.
  modified_base 1: mod_base = OTHER; mod_base = gm; note = This nucleotide is modified with Y6.
  modified_base 2..3: mod_base = OTHER; note = These bases are 2-O-methyl nucleosides.
  modified_base 7: mod_base = cm
  modified_base 14: mod_base = OTHER; note = This base is a 2-O-methyl nucleoside.
  modified_base 15..16: mod_base = cm
gaacaccttcagaacc

SEQ ID NO: 845 - RNA, 16 nt, synthetic construct
  source 1..16: mol_type = other RNA
  modified_base 1..3: mod_base = OTHER; note = These nucleotides are bound via phosphorothioate linkages. These nucleosides are 2-4-BNA NC [N-Me] nucleosides.
  modified_base 13..15: mod_base = OTHER; note = These nucleotides are bound via phosphorothioate linkages.
  modified_base 14..16: mod_base = OTHER; note = These nucleosides are 2-4-BNA NC [N-Me] nucleosides.
  modified_base 1: mod_base = OTHER; note = This nucleotide is modified with Y6.
gaacaccttcagaacc

SEQ ID NO: 846 - DNA, 16 bp, synthetic construct
  misc_feature 4: note = DNA
  source 1..16: mol_type = other DNA
  misc_feature 6..10: note = 10
  modified_base 1..3: mod_base = OTHER; note = These nucleotides are bound via phosphorothioate linkages. These nucleosides are 2-4-BNA NC [N-Me] nucleosides.
  modified_base 13..15: mod_base = OTHER; note = These nucleotides are bound via phosphorothioate linkages.
  modified_base 1: mod_base = OTHER; note = This nucleotide is modified with Y6.
  modified_base 14..16: mod_base = OTHER; note = These nucleosides are 2-4-BNA NC [N-Me] nucleosides.
gaacaccttcagaacc

SEQ ID NO: 847 - DNA, 16 bp, synthetic construct
  misc_feature 4..5: note = DNA
  source 1..16: mol_type = other DNA
  misc_feature 8: note = DNA
  misc_feature 10..13: note = DNA
  modified_base 1..3: mod_base = OTHER; note = These nucleotides are bound via phosphorothioate linkages.
  modified_base 13..15: mod_base = OTHER; note = These nucleotides are bound via phosphorothioate linkages.
  modified_base 7: mod_base = cm
  modified_base 1..3: mod_base = OTHER; note = These nucleosides are 2-4-BNA NC [N-Me] nucleosides.
  modified_base 14..16: mod_base = OTHER; note = These nucleosides are 2-4-BNA NC [N-Me] nucleosides.
  modified_base 1: mod_base = OTHER; note = This nucleotide is modified with Y6.
gaacaccttcagaacc

SEQ ID NO: 848 - DNA, 19 bp, synthetic construct
  misc_feature 9..11: note = DNA
  source 1..19: mol_type = other DNA
  modified_base 1..3: mod_base = OTHER; note = These nucleotides are bound via phosphorothioate linkages.
  modified_base 16..18: mod_base = OTHER; note = These nucleotides are bound via phosphorothioate linkages.
  modified_base 1: mod_base = OTHER; mod_base = gm; note = This nucleotide is modified with Y6.
  modified_base 2..3: mod_base = OTHER; note = These bases are 2-O-methyl nucleosides.
  modified_base 4: mod_base = cm
  modified_base 5: mod_base = OTHER; note = This base is a 2-O-methyl nucleoside.
  modified_base 6..7: mod_base = cm
  modified_base 8: mod_base = um
  modified_base 12: mod_base = um
  modified_base 13: mod_base = cm
  modified_base 14: mod_base = OTHER; note = This base is a 2-O-methyl nucleoside.
  modified_base 15: mod_base = gm
  modified_base 16..17: mod_base = OTHER; note = These bases are 2-O-methyl nucleosides.
  modified_base 18..19: mod_base = cm
gaacacctaaatcagaacc

SEQ ID NO: 849 - DNA, 25 bp, synthetic construct
  misc_feature 7..9: note = DNA
  source 1..25: mol_type = other DNA
  misc_feature 17..19: note = DNA
  modified_base 1..3: mod_base = OTHER; note = These nucleotides are bound via phosphorothioate linkages.
  modified_base 22..24: mod_base = OTHER; note = These nucleotides are bound via phosphorothioate linkages.
  modified_base 1: mod_base = gm; mod_base = OTHER; note = This nucleotide is modified with Y6.
  modified_base 2..3: mod_base = OTHER; note = These bases are 2-O-methyl nucleosides.
  modified_base 4: mod_base = cm
  modified_base 5: mod_base = OTHER; note = This base is a 2-O-methyl nucleoside.
  modified_base 6: mod_base = cm
  modified_base 10..11: mod_base = um
  modified_base 12: mod_base = cm
  modified_base 13: mod_base = OTHER; note = This base is a 2-O-methyl nucleoside.
  modified_base 14: mod_base = gm
  modified_base 15..16: mod_base = OTHER; note = These bases are 2-O-methyl nucleosides.
  modified_base 20: mod_base = cm
  modified_base 21..22: mod_base = gm
  modified_base 23: mod_base = OTHER; note = This base is a 2-O-methyl nucleoside.
  modified_base 24..25: mod_base = gm
gaacacaaattcagaaaaacggagg

SEQ ID NO: 850 - DNA, 16 bp, synthetic construct
  misc_feature 4: note = DNA
  source 1..16: mol_type = other DNA
  misc_feature 6..10: note = DNA
  modified_base 1..3: mod_base = OTHER; note = These nucleotides are bound via phosphorothioate linkages.
  modified_base 13..15: mod_base = OTHER; note = These nucleotides are bound via phosphorothioate linkages.
  modified_base 1: mod_base = gm; mod_base = OTHER; note = This nucleotide is modified with Y5.
  modified_base 2..3: mod_base = OTHER; note = These bases are 2-O-methyl nucleosides.
  modified_base 14: mod_base = OTHER; note = This base is a 2-O-methyl nucleoside.
  modified_base 15..16: mod_base = cm
  modified_base 16: mod_base = OTHER; note = This nucleotide is modified with Y6.
gaacaccttcagaacc

SEQ ID NO: 851 - DNA, 19 bp, synthetic construct
  misc_feature 1..3: note = DNA
  source 1..19: mol_type = other DNA
  misc_feature 7: note = DNA
  misc_feature 9..13: note = DNA
  modified_base 17: mod_base = OTHER; note = This base is a 2-O-methyl nucleoside.
  modified_base 18..19: mod_base = cm
  modified_base 16..18: mod_base = OTHER; note = These nucleotides are bound via phosphorothioate linkages.
  modified_base 1: mod_base = OTHER; note = This nucleotide is modified with Y6.
tcagaacaccttcagaacc

SEQ ID NO: 852 - DNA, 25 bp, synthetic construct
  misc_feature 4: note = DNA
  source 1..25: mol_type = other DNA
  misc_feature 6..10: note = DNA
  misc_feature 15..16: note = DNA
  misc_feature 22: note = DNA
  modified_base 1: mod_base = gm; mod_base = OTHER; note = This nucleotide is bound via a phosphorothioate linkage. This nucleotide is modified with Y6.
  modified_base 24: mod_base = OTHER; note = This nucleotide is bound via a phosphorothioate linkage.
  modified_base 25: mod_base = cm
gaacaccttcagaaccggaggcaac

SEQ ID NO: 853 - DNA, 16 bp, synthetic construct
  source 1..16: mol_type = other DNA
  modified_base 1: mod_base = OTHER; note = This nucleotide is modified with Y6.
gaacaccttcagaacc

SEQ ID NO: 854 - DNA, 16 bp, synthetic construct
  misc_feature 4: note = DNA
  source 1..16: mol_type = other DNA
  misc_feature 6..10: note = DNA
  modified_base 1..3: mod_base = OTHER; note = These nucleotides are bound via phosphorothioate linkages.
  modified_base 13..15: mod_base = OTHER; note = These nucleotides are bound via phosphorothioate linkages.
  modified_base 1: mod_base = gm; mod_base = OTHER; note = This nucleotide is modified with Y7.
  modified_base 2..3: mod_base = OTHER; note = These bases are 2-O-methyl nucleosides.
  modified_base 14: mod_base = OTHER; note = This base is a 2-O-methyl nucleoside.
  modified_base 15..16: mod_base = cm
gaacaccttcagaacc

SEQ ID NO: 855 - DNA, 16 bp, synthetic construct
  misc_feature 4: note = DNA
  source 1..16: mol_type = other DNA
  misc_feature 6..10: note = DNA
  modified_base 1..3: mod_base = OTHER; note = These nucleotides are bound via phosphorothioate linkages.
  modified_base 13..15: mod_base = OTHER; note = These nucleotides are bound via phosphorothioate linkages.
  modified_base 1: mod_base = gm; mod_base = OTHER; note = This nucleotide is modified with Y8.
  modified_base 2..3: mod_base = OTHER; note = These bases are 2-O-methyl nucleosides.
  modified_base 14: mod_base = OTHER; note = This base is a 2-O-methyl nucleoside.
  modified_base 15..16: mod_base = cm
gaacaccttcagaacc

SEQ ID NO: 856 - DNA, 16 bp, synthetic construct
  misc_feature 4: note = DNA
  source 1..16: mol_type = other DNA
  misc_feature 6..10: note = DNA
  modified_base 1..3: mod_base = OTHER; note = These nucleotides are bound via phosphorothioate linkages.
  modified_base 13..15: mod_base = OTHER; note = These nucleotides are bound via phosphorothioate linkages.
  modified_base 1: mod_base = gm; mod_base = OTHER; note = This nucleotide is modified with Y9.
  modified_base 2..3: mod_base = OTHER; note = These bases are 2-O-methyl nucleosides.
  modified_base 14: mod_base = OTHER; note = This base is a 2-O-methyl nucleoside.
  modified_base 15..16: mod_base = cm
gaacaccttcagaacc

SEQ ID NO: 857 - DNA, 25 bp, synthetic construct
  source 1..25: mol_type = other DNA
  modified_base 1: mod_base = OTHER; note = This nucleotide is modified with Y6.
  modified_base 16: mod_base = OTHER; note = This cytosine is a 5-methyle cytosine.
gaacaccttcagaaccggaggcaac

SEQ ID NO: 858 - DNA, 21 bp, synthetic construct
  source 1..21: mol_type = other DNA
  modified_base 1: mod_base = OTHER; note = This nucleotide is modified with Y6.
  modified_base 16: mod_base = OTHER; note = This cytosine is a 5-methyle cytosine.
gaacaccttcagaaccggagg

SEQ ID NO: 859 - DNA, 25 bp, synthetic construct
  misc_feature 4: note = DNA
  source 1..25: mol_type = other DNA
  misc_feature 6..10: note = DNA
  misc_feature 15..16: note = DNA
  misc_feature 22: note = DNA
  modified_base 1..3: mod_base = OTHER; note = These nucleotides are bound via phosphorothioate linkages.
  modified_base 22..24: mod_base = OTHER; note = These nucleotides are bound via phosphorothioate linkages.
  modified_base 1: mod_base = gm; mod_base = OTHER; note = This nucleotide is modified with Y9.
  modified_base 22..24: mod_base = OTHER; note = These nucleotides are bound via phosphorothioate linkages.
  modified_base 2..3: mod_base = OTHER; note = These bases are 2-O-methyl nucleosides.
  modified_base 23..24: mod_base = OTHER; note = These bases are 2-O-methyl nucleosides.
  modified_base 25: mod_base = cm
gaacaccttcagaaccggaggcaac

SEQ ID NO: 860 - DNA, 21 bp, synthetic construct
  misc_feature 4: note = DNA
  source 1..21: mol_type = other DNA
  misc_feature 6..10: note = DNA
  misc_feature 15..16: note = DNA
  modified_base 1..3: mod_base = OTHER; note = These nucleotides are bound via phosphorothioate linkages.
  modified_base 18..20: mod_base = OTHER; note = These nucleotides are bound via phosphorothioate linkages.
  modified_base 1: mod_base = gm; mod_base = OTHER; note = This nucleotide is modified with Y9.
  modified_base 2..3: mod_base = OTHER; note = These bases are 2-O-methyl nucleosides.
  modified_base 19: mod_base = OTHER; note = This base is a 2-O-methyl nucleoside.
  modified_base 20..21: mod_base = gm
gaacaccttcagaaccggagg

SEQ ID NO: 861 - RNA, 21 nt, synthetic construct
  source 1..21: mol_type = other RNA
  modified_base 1..3: mod_base = OTHER; note = These nucleotides are bound via phosphorothioate linkages.
  modified_base 18..20: mod_base = OTHER; note = These nucleotides are bound via phosphorothioate linkages.
  modified_base 1: mod_base = gm; mod_base = OTHER; note = This nucleotide is modified with Y6.
  modified_base 2..3: mod_base = OTHER; note = These bases are 2-O-methyl nucleosides.
  modified_base 19: mod_base = OTHER; note = This base is a 2-O-methyl nucleoside.
  modified_base 20..21: mod_base = gm
gaacaccttcagaaccggagg

SEQ ID NO: 862 - RNA, 25 nt, synthetic construct
  source 1..25: mol_type = other RNA
  modified_base 1..3: mod_base = OTHER; note = These nucleotides are bound via phosphorothioate linkages.
  modified_base 22..24: mod_base = OTHER; note = These nucleotides are bound via phosphorothioate linkages.
  modified_base 1: mod_base = OTHER; note = This base is a 2-O-methyl nucleoside. This nucleotide is modified with Y6.
  modified_base 2..3: mod_base = um
  modified_base 23: mod_base = gm
  modified_base 24..25: mod_base = cm
atttcaggtaagccgaggtttggcc

SEQ ID NO: 863 - RNA, 16 nt, synthetic construct
  source 1..16: mol_type = other RNA
  modified_base 1..3: mod_base = OTHER; note = These nucleotides are bound via phosphorothioate linkages.
  modified_base 13..15: mod_base = OTHER; note = These nucleotides are bound via phosphorothioate linkages.
  modified_base 1: mod_base = OTHER; note = This base is a 2-O-methyl nucleoside. This nucleotide is modified with Y6.
  modified_base 2..3: mod_base = um
  modified_base 14: mod_base = cm
  modified_base 15: mod_base = gm
  modified_base 16: mod_base = OTHER; note = This base is a 2-O-methyl nucleoside.
atttcaggtaagccga

SEQ ID NO: 864 - DNA, 25 bp, synthetic construct
  misc_feature 9: note = DNA
  source 1..25: mol_type = other DNA
  modified_base 1: mod_base = OTHER; note = This base is a 2-O-methyl nucleoside. This nucleotide is modified with Y6.
  modified_base 2..3: mod_base = um
  modified_base 1..3: mod_base = OTHER; note = These nucleotides are bound via phosphorothioate linkages.
  modified_base 22..23: mod_base = gm
  modified_base 24..25: mod_base = cm
  modified_base 22..24: mod_base = OTHER; note = These nucleotides are bound via phosphorothioate linkages.
  misc_feature 4..5: note = DNA
  misc_feature 13..14: note = DNA
  misc_feature 19..21: note = DNA
atttcaggtaagccgaggtttggcc

SEQ ID NO: 865 - DNA, 16 bp, synthetic construct
  misc_feature 4..5: note = DNA
  source 1..16: mol_type = other DNA
  misc_feature 9: note = DNA
  misc_feature 13: note = DNA
  modified_base 1: mod_base = OTHER; note = This base is a 2-O-methyl nucleoside.This nucleotide is modified with Y6.
  modified_base 2..3: mod_base = um
  modified_base 1..3: mod_base = OTHER; note = These nucleotides are bound via phosphorothioate linkages.
  modified_base 13..15: mod_base = OTHER; note = These nucleotides are bound via phosphorothioate linkages.
  modified_base 14: mod_base = cm
  modified_base 15: mod_base = gm
  modified_base 16: mod_base = OTHER; note = This base is a 2-O-methyl nucleoside.
atttcaggtaagccga

SEQ ID NO: 866 - DNA, 25 bp, synthetic construct
  misc_feature 7..9: note = DNA
  source 1..25: mol_type = other DNA
  modified_base 1: mod_base = OTHER; note = This base is a 2-O-methyl nucleoside. This nucleotide is modified with Y6.
  modified_base 2..4: mod_base = um
  modified_base 5: mod_base = cm
  modified_base 6: mod_base = OTHER; note = This base is a 2-O-methyl nucleoside.
  modified_base 1..3: mod_base = OTHER; note = These nucleotides are bound via phosphorothioate linkages.
  modified_base 10: mod_base = gm
  modified_base 11: mod_base = um
  modified_base 12..13: mod_base = OTHER; note = These bases are 2-O-methyl nucleosides.
  modified_base 14: mod_base = gm
  modified_base 15..16: mod_base = cm
  modified_base 20: mod_base = OTHER; note = This base is a 2-O-methyl nucleoside.
  modified_base 21..22: mod_base = gm
  modified_base 23..25: mod_base = um
  modified_base 22..24: mod_base = OTHER; note = These nucleotides are bound via phosphorothioate linkages.
  misc_feature 17..19: note = DNA
atttcaaaagtaagccaaaaggttt

SEQ ID NO: 867 - DNA, 25 bp, synthetic construct
  misc_feature 4..5: note = DNA
  source 1..25: mol_type = other DNA
  modified_base 1: mod_base = OTHER; note = This base is a 2-O-methyl nucleoside. This nucleotide is modified with Y9.
  modified_base 2..3: mod_base = um
  modified_base 1..3: mod_base = OTHER; note = These nucleotides are bound via phosphorothioate linkages.
  modified_base 22: mod_base = gm
  modified_base 24..25: mod_base = cm
  modified_base 22..24: mod_base = OTHER; note = These nucleotides are bound via phosphorothioate linkages.
  misc_feature 9: note = DNA
  misc_feature 13..14: note = DNA
  misc_feature 19..21: note = DNA
atttcaggtaagccgaggtttggcc

SEQ ID NO: 868 - DNA, 16 bp, synthetic construct
  misc_feature 4..5: note = DNA
  source 1..16: mol_type = other DNA
  modified_base 1: mod_base = OTHER; note = This base is a 2-O-methyl nucleoside. This nucleotide is modified with Y5.
  modified_base 2..3: mod_base = um
  modified_base 1..3: mod_base = OTHER; note = These nucleotides are bound via phosphorothioate linkages.
  modified_base 14: mod_base = cm
  modified_base 15: mod_base = gm
  modified_base 16: mod_base = OTHER; note = This base is a 2-O-methyl nucleoside. This nucleotide is modified with Y6.
  modified_base 13..15: mod_base = OTHER; note = These nucleotides are bound via phosphorothioate linkages.
  misc_feature 9: note = DNA
  misc_feature 13: note = DNA
atttcaggtaagccga

SEQ ID NO: 869 - DNA, 16 bp, synthetic construct
  misc_feature 9: note = DNA
  source 1..16: mol_type = other DNA
  modified_base 1: mod_base = OTHER; note = This nucleotide is modified with Y6.
  modified_base 1..3: mod_base = OTHER; note = These nucleosides are 2-4-BNA NC [N-Me] nucleosides. These nucleotides are bound via phosphorothioate linkages.
  modified_base 13..15: mod_base = OTHER; note = These nucleotides are bound via phosphorothioate linkages.
  modified_base 14..16: mod_base = OTHER; note = These nucleosides are 2-4-BNA NC [N-Me] nucleosides.
  modified_base 14: mod_base = OTHER; note = This cytosine is a 5-methyle cytosine.
  misc_feature 4..5: note = DNA
  misc_feature 13: note = DNA
atttcaggtaagccga

SEQ ID NO: 870 - DNA, 25 bp, synthetic construct
  source 1..25: mol_type = other DNA
  modified_base 1: mod_base = OTHER; note = This nucleotide is modified with Y6.
  modified_base 14: mod_base = OTHER; note = This cytosine is a 5-methyle cytosine.
atttcaggtaagccgaggtttggcc

SEQ ID NO: 871 - RNA, 25 nt, synthetic construct
  source 1..25: mol_type = other RNA
  modified_base 1: mod_base = OTHER; note = This nucleotide is modified with Y1.
  modified_base 25: mod_base = OTHER; note = This nucleotide is modified with Y10.
  modified_base 1..25: mod_base = OTHER; note = These nucleotides are morpholino nucleotides.
gttgcctccggttctgaaggtgttc

SEQ ID NO: 872 - protein, 4 aa, synthetic construct
  MOD_RES 1: note = This residue is modified with BCN-AEEA.
  MOD_RES 4: note = bAla
RRRA

SEQ ID NO: 873 - RNA, 25 nt, synthetic construct
  source 1..25: mol_type = other RNA
  modified_base 1: mod_base = OTHER; note = This nucleotide is modified with Y1.
  modified_base 25: mod_base = OTHER; note = This nucleotide is modified with Y11.
  modified_base 1..25: mod_base = OTHER; note = These nucleotides are morpholino nucleotides.
gttgcctccggttctgaaggtgttc

SEQ ID NO: 874 - protein, 9 aa, synthetic construct
  MOD_RES 1: note = This residue is modified with BCN.
  MOD_RES 9: note = This cysteine is Cys (tBuS)-NH2.
GGGEEESSC

SEQ ID NO: 875 - protein, 9 aa, synthetic construct
  MOD_RES 4..6: note = These Glus are Glu (OtBu)s.
  MOD_RES 7..8: note = These Sers are Ser (tBu)s.
  MOD_RES 9: note = This Cys is Cys (tBuS).
GGGEEESSC

SEQ ID NO: 876 - protein, 9 aa, synthetic construct
  MOD_RES 9: note = This cysteine is Cys (tBus)-NH2.
GGGEEESSC

SEQ ID NO: 877 - RNA, 25 nt, synthetic construct
  source 1..25: mol_type = other RNA
  modified_base 1: mod_base = OTHER; note = This nucleotide is modified with Y1.
  modified_base 25: mod_base = OTHER; note = This nucleotide is modified with Y12.
  modified_base 1..25: mod_base = OTHER; note = These nucleotides are morpholino nucleotides.
gttgcctccggttctgaaggtgttc

SEQ ID NO: 878 - RNA, 25 nt, synthetic construct
  source 1..25: mol_type = other RNA
  modified_base 1: mod_base = OTHER; note = This nucleotide is modified with Y1.
  modified_base 25: mod_base = OTHER; note = This nucleotide is modified with Y13.
  modified_base 1..25: mod_base = OTHER; note = These nucleotides are morpholino nucleotides.
ggccaaacctcggcttacctgaaat

SEQ ID NO: 879 - protein, 4 aa, synthetic construct
  MOD_RES 1: note = This residue is modified with 4-pentynoyl-AEEA.
RRRG

SEQ ID NO: 880 - protein, 4 aa, synthetic construct
  MOD_RES 1: note = This residue is modified with 4-pentynoyl-AEEA.
  MOD_RES 1..3: note = These Args are Arg (Pbf)s.
RRRG

SEQ ID NO: 881 - RNA, 25 nt, synthetic construct
  source 1..25: mol_type = other RNA
  modified_base 25: mod_base = OTHER; note = This nucleotide is modified with Y14.
  modified_base 1: mod_base = OTHER; note = This nucleotide is modified with Y1.
  modified_base 1..25: mod_base = OTHER; note = These nucleotides are morpholino nucleotides.
ggccaaacctcggcttacctgaaat

SEQ ID NO: 882 - protein, 4 aa, synthetic construct
  MOD_RES 1: note = This residue is modified with 4-pentynoyl-AEEA.
  MOD_RES 1..3: note = These Lysines are Lys (ivDde)s.
KKKG

SEQ ID NO: 883 - RNA, 25 nt, synthetic construct
  source 1..25: mol_type = other RNA
  modified_base 1: mod_base = OTHER; note = This nucleotide is modified with Y1.
  modified_base 25: mod_base = OTHER; note = This nucleotide is modified with Y12.
  modified_base 1..25: mod_base = OTHER; note = These nucleotides are morpholino nucleotides.
ggccaaacctcggcttacctgaaat